European Patent Application EP 4 118 955 A1, published January 18, 2023. Title: METHODS AND COMPOSITIONS FOR ACCELERATED TRAIT IN INTROGRESSION. Applicant: Pioneer Hi-Bred International, Inc. Application EP, filed March 16, 2016. The sequence listing filed with the application follows.

SEQUENCE LISTING (122 sequences)

SEQ ID NO: 1 - DNA, 48 bp, Saccharomyces cerevisiae
  source 1..48: mol_type = unassigned DNA
gaagttcctattccgaagttcctattctctagaaagtataggaacttc

SEQ ID NO: 2 - DNA, 48 bp, Saccharomyces cerevisiae
  source 1..48: mol_type = unassigned DNA
gaagttcctattccgaagttcctattctccagaaagtataggaacttc

SEQ ID NO: 3 - protein, 420 aa, Zea mays
ACGLVQAQVLFQGFNWESCKQQGGWYNRLKAQVDDIAKAGVTHVWLPPPSHSVSPQGYMPGRLYDLDASKYGTAAELKSLIAAFHGRGVQCVADIVINHRCAEKKDARGVYCIFEGGTPDDRLDWGPGMICSDDTQYSDGTGHRDTGEGFAAAPDIDHLNPRVQRELSAWLNWLRSDAVGFDGWRLDFAKGYSPAVARMYVESTGPPSFVVAEIWNSLSYSGDGKPAPNQDQCRQELLDWTRAVGGPAMAFDFPTKGLLQAGVQGELWRLRDSSGNAAGLIGWAPEKAVTFVDNHDTGSTQKLWPFPSDKVMQGYAYILTHPGVPCIFYDHMFDWNLKQEISTLSAIRARNGIRAGSKLRILVADADAYVAVVDEKVMVKIGTRYGVSSVVPSDFHPAAHGKDYCVWEKASLRVPAGRHL

SEQ ID NO: 4 - DNA, 1336 bp, Zea mays
  source 1..1336: mol_type = unassigned DNA
gcctgcggcctggtccaggcacaagtcctcttccaggggtttaactgggagtcgtgcaagcagcagggaggctggtacaacaggctcaaggcccaggtcgacgacatcgccaaggccggcgtcacgcacgtctggctgcctccaccctcgcactccgtctcgccacaaggctacatgccaggccgcctatacgacctggacgcgtccaagtacggcacggcggcggagctcaagtccctgatagcggcgttccacggcaggggcgtgcagtgcgtggcggacatcgtcatcaaccaccggtgcgcggaaaagaaggacgcgcgcggcgtgtactgcatcttcgagggcgggactcccgacgaccgcctggactggggccccgggatgatctgcagcgacgacacgcagtactcggacgggacggggcaccgcgacacgggcgaggggttcgcggcggcgcccgacatcgaccacctcaacccgcgcgtgcagcgggagctctccgcctggctcaactggctcaggtccgacgccgtggggttcgacggctggcgcctcgacttcgccaagggctactcgccggccgtcgccagaatgtacgtggagagcacggggccgccgagcttcgtcgtcgcggagatatggaactcgctgagctacagcggggacggcaagccggcgcccaaccaggaccagtgccggcaggagctgctggactggacgcgggccgtcggcgggcccgccatggcgttcgacttccccaccaagggcctgctgcaggcgggcgtgcagggggagctgtggcggctgcgcgacagctccggcaacgcggccggcctgatcgggtgggcgcccgagaaggccgtcaccttcgtcgacaaccatgacaccgggtcgacgcagaagctctggccgttcccatccgacaaggtcatgcagggctacgcctacatcctcacccatccaggagtcccctgcattttctacgaccacatgttcgactggaacctgaagcaggagatatccacgctgtctgccatcagggcgcggaacggcatccgcgccgggagcaagctgcggatcctcgtggcggacgcggacgcgtacgtggccgtcgtcgacgagaaggtcatggtgaagatcgggacaaggtacggcgtgagcagcgtggtcccgtcggatttccacccggcggcgcacggcaaggactactgcgtctgggagaaagcgagcctccgcgtcccggcggggcgccacctctagcagctcagattgctcagtcttgtgctgcattgcaaacacagcagcacgacactgcataacgtcttttccttga

SEQ ID NO: 5 - protein, 264 aa, Escherichia coli
MVEQDGLHAGSPAAWVERLFGYDWAQQTIGCSDAAVFRLSAQGRPVLFVKTDLSGALNELQDEAARLSWLATTGVPCAAVLDVVTEAGRDWLLLGEVPGQDLLSSHLAPAEKVSIMADAMRRLHTLDPATCPFDHQAKHRIERARTRMEAGLVDQDDLDEEHQGLAPAELFARLKARMPDGDDLVVTHGDACLPNIMVENGRFSGFIDCGRLGVADRYQDIALATRDIAEELGGEWADRFLVLYGIAAPDSQRIAFYRLLDEFF

SEQ ID NO: 6 - DNA, 795 bp, Escherichia coli
  source 1..795: mol_type = unassigned DNA
atggttgaacaagatggattgcacgcaggttctccggccgcttgggtggagaggctattcggctatgactgggcacaacagacaatcggctgctctgatgccgccgtgttccggctgtcagcgcaggggcgcccggttctttttgtcaagaccgacctgtccggtgccctgaatgaactgcaggacgaggcagcgcggctatcgtggctggccacgacgggcgttccttgcgcagctgtgctcgacgttgtcactgaagcgggaagggactggctgctattgggcgaagtgccggggcaggatctcctgtcatctcaccttgctcctgccgagaaagtatccatcatggctgatgcaatgcggcggctgcatacgcttgatccggctacctgcccattcgaccaccaagcgaaacatcgcatcgagcgagcacgtactcggatggaagccggtcttgtcgatcaggatgatctggacgaagagcatcaggggctcgcgccagccgaactgttcgccaggctcaaggcgcgcatgcccgacggcgatgatctcgtcgtgacccatggcgatgcctgcttgccgaatatcatggtggaaaatggccgcttttctggattcatcgactgtggccggctgggtgtggcggaccgctatcaggacatagcgttggctacccgtgatattgctgaagagcttggcggcgaatgggctgaccgcttcctcgtgctttacggtatcgccgctcccgattcgcagcgcatcgccttctatcgccttcttgacgagttcttctga

SEQ ID NO: 7 - DNA, 203 bp, Cauliflower Mosaic Virus
  source 1..203: mol_type = unassigned DNA
cgctgaaatcaccagtctctctctacaaatctatctctctctataataatgtgtgagtagttcccagataagggaattagggttcttatagggtttcgctcatgtgttgagcatataagaaacccttagtatgtatttgtatttgtaaaatacttctatcaataaaatttctaattcctaaaaccaaaatccagtggcgagct

SEQ ID NO: 8 - DNA, 310 bp, Solanum tuberosum
  source 1..310: mol_type = unassigned DNA
ctagacttgtccatcttctggattggccaacttaattaatgtatgaaataaaaggatgcacacatagtgacatgctaatcactataatgtgggcatcaaagttgtgtgttatgtgtaattactagttatctgaataaaagagaaagagatcatccatatttcttatcctaaatgaatgtcacgtgtctttataattctttgatgaaccagatgcatttcattaaccaaatccatatacatataaatattaatcatatataattaatatcaattgggttagcaaaacaaatctagtctaggtgtgttttgc

SEQ ID NO: 9 - DNA, 850 bp, Zea mays
  source 1..850: mol_type = unassigned DNA
gatctcgatgtgtagtctacgagaagggttaaccgtctcttcgtgagaataaccgtggcctaaaaataagccgatgaggataaataaaatgtggtggtacagtacttcaagaggtttactcatcaagaggatgcttttccgatgagctctagtagtacatcggacctcacatacctccattgtggtgaaatattttgtgctcatttagtgatgggtaaattttgtttatgtcactctaggttttgacatttcagttttgccactcttaggttttgacaaataatttccattccgcggcaaaagcaaaacaattttattttacttttaccactcttagctttcacaatgtatcacaaatgccactctagaaattctgtttatgccacagaatgtgaaaaaaaacactcacttatttgaagccaaggtgttcatggcatggaaatgtgacataaagtaacgttcgtgtataagaaaaaattgtactcctcgtaacaagagacggaaacatcatgagacaatcgcgtttggaaggctttgcatcacctttggatgatgcgcatgaatggagtcgtctgcttgctagccttcgcctaccgcccactgagtccgggcggcaactaccatcggcgaacgacccagctgacctctaccgaccggacttgaatgcgctaccttcgtcagcgacgatggccgcgtacgctggcgacgtgcccccgcatgcatggcggcacatggcgagctcagaccgtgcgtggctggctacaaatacgtaccccgtgagtgccctagctagaaacttacacctgcaactgcgagagcgagcgtgtgagtgtagccgatagatccgccc

SEQ ID NO: 10 - protein, 233 aa, synthetic construct
  REGION 1..233: note = Sequence from Dictosoma species
MSELIKENMHMKLYMEGTVDNHHFKCTSEGEGKPYEGTQTMRIKVVEGGPLPFAFDILATSFLYGSKTFINHTQGIPDFFKQSFPEGFTWERVTTYEDGGVLTATQDTSLQDGCLIYNVKIRGVNFTSNGPVMQKKTLGWEAFTETLYPADGGLEGRNDMALKLVGGSHLIANIKTTYRSKKPAKNLKMPGVYYVDYRLERIKEANNETYVEQHEVAVARYCDLPSKLGHKLN

SEQ ID NO: 11 - DNA, 702 bp, synthetic construct
  misc_feature 1..702: note = Sequence from Dictosoma species
  source 1..702: mol_type = other DNA
atgagcgagctgattaaagagaacatgcacatgaagctgtacatggaggggaccgtcgacaaccaccacttcaagtgcacctccgagggcgagggtaagccgtatgagggcacgcagacaatgaggattaaagtggttgagggcgggccgctgcctttcgcattcgacatcctcgccaccagcttcctgtacgggtccaagaccttcatcaaccacacccagggcatccccgacttcttcaaacagtccttcccggagggtttcacgtgggagagggtgacaacctacgaagatggcggcgtgctgaccgccacgcaggatacatctctccaggacgggtgcctgatctacaacgtcaagatcaggggcgtcaacttcacgagcaacggcccggtcatgcagaagaagacgctcggctgggaagccttcacggagacactctaccccgccgacggcgggctggaaggtaggaacgacatggccctcaagctcgtgggcggcagccacctcatcgccaacatcaaaaccacctacaggagcaagaagcccgccaagaacctgaagatgcccggcgtgtactacgtcgactacaggctcgagagaattaaggaggccaacaacgagacgtacgtggagcagcacgaggttgcagttgccaggtactgcgacctgccgagcaagctcggccacaagctgaactag

SEQ ID NO: 12 - DNA, 476 bp, Zea mays
  source 1..476: mol_type = unassigned DNA
gaagaaactatgtgctgtagtatagccgctgcccgctggctagctagctagttgagtcatttagcggcgatgattgagtaataatgtgtcacgcatcaccatgcatgggtggcagtgtcagtgtgagcaatgacctgaatgaacaattgaaatgaaaagaaaaaagtattgttccaaattaaacgttttaaccttttaataggtttatacaataattgatatatgttttctgtatatgtctaatttgttatcatccatttagatatagacaaaaaaaatctaagaactaaaacaaatgctaatttgaaatgaagggagtatatattgggataatgtcgatgagatccctcgtaatatcaccgacatcacacgtgtccagttaatgtatcagtgatacgtgtattcacatttgttgcgcgtaggcgtacccaacaattttgatcgactatcagaaagtcaacggaagcgagtcgacc

SEQ ID NO: 13 - DNA, 2773 bp, Zea mays
  source 1..2773: mol_type = unassigned DNA
aagcttgcatgcctgcaggtcgactctagaggatctgcaccggacactgtctggtggcataccagacagtccggtgtgccagatcagggcacccttcggttcctttgctcctttgcttttgaaccctaactttgatcgtttattggtttgtgttgaacctttatgcacctgtggaatatataatctagaacaaactagttagtccaatcatttgtgttgggcattcaaccaccaaaattatttataggaaaaggttaaaccttatttccctttcaatctccccctttttggtgattgatgccaacacaaaccaaagaaaatatataagtgcagaattgaactagtttgcataaggtaagtgcataggttacttagaattaaatcaatttatacttttacttgatatgcatggttgctttcttttattttaacattttggaccacatttgcaccacttgttttgttttttgcaaatctttttggaaattctttttcaaagtcttttgcaaatagtcaaaggtatatgaataagattgtaagaagcattttcaagatttgaaatttctccccctgtttcaaatgcttttcctttgactaaacaaaactccccctgaataaaattctcctcttagctttcaagagggttttaaatagatatcaattggaaatatatttagatgctaattttgaaaatataccaattgaaaatcaacataccaatttgaaattaaacataccaatttaaaaaatttcaaaaagtggtggtgcggtccttttgctttgggcttaatatttctccccctttggcattaatcgccaaaaacggagactttgtgagccatttatactttctccccattggtaaatgaaatatgagtgaaagattataccaaatttggacagtgatgcggagtgacggcgaaggataaacgataccgttagagtggagtggaagccttgtcttcgccgaagactccatttccctttcaatctacgacttagcatagaaatacacttgaaaacacattagtcgtagccacgaaagagatatgatcaaaggtatacaaatgagctatgtgtgtaatgtttcaatcaaagtttcgagaatcaagaatatttagctcattcctaagtttgctaaaggttttatcatctaatggtttggtaaagatatcgactaattgttctttggtgctaacataagcaatctcgatatcacccctttgttggtgatccctcaaaaagtgataccgaatgtctatgtgcttagtgcggctgtgttcaacgggattatccgccatgcagatagcactctcattgtcacataggagagggactttgctcaatttgtagccatagtccctaaggttttgcctcatccaaagtaattgcacacaacaatgtcctgcggcaatatacttggcttcggcggtagaaagagctattgagttttgtttctttgaagtccaagacaccagggatctccctagaaactgacaagtccctgatgtgctcttcctatcaattttacaccctgcccaatcggcatctgaatatcctattaaatcaaaggtggatcccttggggtaccaaagaccaaatttaggagtgtaaactaaatatctcatgattcttttcacggccctaaggtgaacttccttaggatcggcttggaatcttgcacacatgcatatagaaagcatactatctggtcgagatgcacataaatagagtaaagatcctatcatcgaccggtataccttttggtctacggatttacctcccgtgtcgaggtcgagatgcccattagttcccatgggtgtcctgatgggcttggcatccttcattccaaacttgttgagtatgtcttgaatgtactttgtttggctgatgaaggtgccatcttggagttgcttgacttgaaatcctagaaaatatttcaacttccccatcatagacatctcgaatttcggaatcatgatcctactaaactcttcacaagtagatttgttagtagacccaaatataatatcatcaacataaatttggcatacaaacaaaacttttgaaatggttttagtaaagagagtaggatcggctttactgactctgaagccattagtgataagaaaatctcttaggcattcataccatgctgttggggcttgcttgagcccataaagcgcctttgagagtttataaacatggttagggtactcactatcttcaaagccgagaggttgctcaacatagacctattcaccccatttgatcacttttttggtccttcaggatctaatagttatgtataatttagagtctcttgtttaatggccagatatttctaattaatctaagaatttatgatattttttaattttttatcatgtctgatgagaattaacataaaggctcaattgggtcctgaattaataatagagtgaaaattaatccagaggctctattagaaccttcaattagtaataccaagatatatataagatagtagagtatagtttaaatgttggcattgttcattctttcttttgttatttaatttatgctttccacggtggttagtggttacttctgaagggtccaaataatgcatgaagagtttgaggacaagaagtctgccctaaaaatagcgatgcaaaggcatggtgtccaagccatacatatagcgcactaattttatcagcagaacaatggtatttataggtcctagtgcccaggcaacaagagacacgaataaagcatcgatcacgacacc

SEQ ID NO: 14 - protein, 75 aa, Zea mays
MAATMAVTTMVTRSKESWSSLQVPAVAFPWKPRGGKTGGLEFPRRAMFASVGLNVCPGVPAGRDPREPDPKVVRA

SEQ ID NO: 15 - DNA, 450 bp, Zea mays
  source 1..450: mol_type = unassigned DNA
atggcggcgacaatggcagtgacgacgatggtgacgaggagcaaggagagctggtcgtcattgcaggtcccggcggtggcattcccttggaagccacgaggtggcaagaccggcggcctcgagttccctcgccgggcgatgttcgccagcgtcggcctcaacgtgtgcccgggcgtcccggcggggcgcgacccgcgggagcccgatcccaaggtcgtccgggcgatggcggcgacaatggcagtgacgacgatggtgacgaggagcaaggagagctggtcgtcattgcaggtcccggcggtggcattcccttggaagccacgaggtggcaagaccggcggcctcgagttccctcgccgggcgatgttcgccagcgtcggcctcaacgtgtgcccgggcgtcccggcggggcgcgacccgcgggagcccgatcccaaggtcgtccgggcg

SEQ ID NO: 16 - DNA, 348 bp, Zea mays
  source 1..348: mol_type = unassigned DNA
gatctgacaaagcagcattagtccgttgatcggtggaagaccactcgtcagtgttgagttgaatgtttgatcaataaaatacggcaatgctgtaagggttgttttttatgccattgataatacactgtactgttcagttgttgaactctatttcttagccatgccaagtgcttttcttattttgaataacattacagcaaaaagttgaaagacaaaaaaaaaaacccccgaacagagtgctttgggtcccaagctactttagactgtgttcggcgttccccctaaatttctccccctatatctcactcacttgtcacatcagcgttctctttcccctatatctccacg

SEQ ID NO: 17 - protein, 391 aa, Bacillus amyloliquefaciens
MQKLINSVQNYAWGSKTALTELYGMENPSSQPMAELWMGAHPKSSSRVQNAAGDIVSLRDVIESDKSTLLGEAVAKRFGELPFLFKVLCAAQPLSIQVHPNKHNSEIGFAKENAAGIPMDAAERNYKDPNHKPELVFALTPFLAMNAFREFSEIVSLLQPVAGAHPAIAHFLQQPDAERLSELFASLLNMQGEEKSRALAILKSALDSQQGEPWQTIRLISEFYPEDSGLFSPLLLNVVKLNPGEAMFLFAETPHAYLQGVALEVMANSDNVLRAGLTPKYIDIPELVANVKFEAKPANQLLTQPVKQGAELDFPIPVDDFAFSLHDLSDKETTISQQSAAILFCVEGDATLWKGSQQLQLKPGESAFIAANESPVTVKGHGRLARVYNKL

SEQ ID NO: 18 - DNA, 274 bp, Bacillus amyloliquefaciens
  source 1..274: mol_type = unassigned DNA
atgaaaaaagcagtcattaacggggaacaaatcagaagtatcagcgacctccaccagacattgaaaaaggagcttgcccttccggaatactacggtgaaaacctggacgctttatgggattgtctgaccggatgggtggagtacccgctcgttttggaatggaggcagtttgaacaaagcaagcagctgactgaaaatggcgccgagagtgtgcttcaggttttccgtgaagcgaaagcggaaggctgcgacatcaccatcatactttcttaac

SEQ ID NO: 19 - DNA, 900 bp, Zea mays
  source 1..900: mol_type = unassigned DNA
ctgcagtgcagcgtgacccggtcgtgcccctctctagagataatgagcattgcatgtctaagttataaaaaattaccacatattttttttgtcacacttgtttgaagtgcagtttatctatctttatacatatatttaaactttactctacgaataatataatctatagtactacaataatatcagtgttttagagaatcatataaatgaacagttagacatggtctaaaggacaattgagtattttgacaacaggactctacagttttatctttttagtgtgcatgtgttctcctttttttttgcaaatagcttcacctatataatacttcatccattttattagtacatccatttagggtttagggttaatggtttttatagactaatttttttagtacatctattttattctattttagcctctaaattaagaaaactaaaactctattttagtttttttatttaataatttagatataaaatagaataaaataaagtgactaaaaattaaacaaataccctttaagaaattaaaaaaactaaggaaacatttttcttgtttcgagtagataatgccagcctgttaaacgccgtcgacgagtctaacggacaccaaccagcgaaccagcagcgtcgcgtcgggccaagcgaagcagacggcacggcatctctgtcgctgcctctggacccctctcgagagttccgctccaccgttggacttgctccgctgtcggcatccagaaattgcgtggcggagcggcagacgtgagccggcacggcaggcggcctcctcctcctctcacggcaccggcagctacgggggattcctttcccaccgctccttcgctttcccttcctcgcccgccgtaataaatagacaccccctccacaccctct

SEQ ID NO: 20 - DNA, 1012 bp, Zea mays
  source 1..1012: mol_type = unassigned DNA
gtacgccgctcgtcctcccccccccccctctctaccttctctagatcggcgttccggtccatgcatggttagggcccggtagttctacttctgttcatgtttgtgttagatccgtgtttgtgttagatccgtgctgctagcgttcgtacacggatgcgacctgtacgtcagacacgttctgattgctaacttgccagtgtttctctttggggaatcctgggatggctctagccgttccgcagacgggatcgatttcatgattttttttgtttcgttgcatagggtttggtttgcccttttcctttatttcaatatatgccgtgcacttgtttgtcgggtcatcttttcatgcttttttttgtcttggttgtgatgatgtggtctggttgggcggtcgttctagatcggagtagaattctgtttcaaactacctggtggatttattaattttggatctgtatgtgtgtgccatacatattcatagttacgaattgaagatgatggatggaaatatcgatctaggataggtatacatgttgatgcgggttttactgatgcatatacagagatgctttttgttcgcttggttgtgatgatgtggtgtggttgggcggtcgttcattcgttctagatcggagtagaatactgtttcaaactacctggtgtatttattaattttggaactgtatgtgtgtgtcatacatcttcatagttacgagtttaagatggatggaaatatcgatctaggataggtatacatgttgatgtgggttttactgatgcatatacatgatggcatatgcagcatctattcatatgctctaaccttgagtacctatctattataataaacaagtatgttttataattattttgatcttgatatacttggatgatggcatatgcagcagctatatgtggatttttttagccctgccttcatacgctatttatttgcttggtactgtttcttttgtcgatgctcaccctgttgtttggtgttacttctgca

SEQ ID NO: 21 - protein, 224 aa, synthetic construct
  REGION 1..224: note = Sequence from Dictosoma species
ASSENVITEFMRFKVRMEGTVNGHEFEIEGEGEGRPYEGHNTVKLKVTKGGPLPFAWDILSPQFQYGSKVYVKHPADIPDYKKLSFPEGFKWERVMNFEDGGVATVTQDSSLQDGCFIYKVKFIGVNFPSDGPVMQKKTMGWEASTERLYPRDGVLKGETHKALKLKDGGHYLVEFKSIYMAKKPVQLPGYYYVDAKLDITSHNEDYTIVEQYERTEGRHHLFL

SEQ ID NO: 22 - DNA, 678 bp, synthetic construct
  misc_feature 1..678: note = Sequence from Dictosoma species
  source 1..678: mol_type = other DNA
atggcctcctccgagaacgtcatcaccgagttcatgcgcttcaaggtgcgcatggagggcaccgtgaacggccacgagttcgagatcgagggcgagggcgagggccgcccctacgagggccacaacaccgtgaagctgaaggtgaccaagggcggccccctgcccttcgcctgggacatcctgtccccccagttccagtacggctccaaggtgtacgtgaagcaccccgccgacatccccgactacaagaagctgtccttccccgagggcttcaagtgggagcgcgtgatgaacttcgaggacggcggcgtggcgaccgtgacccaggactcctccctgcaggacggctgcttcatctacaaggtgaagttcatcggcgtgaacttcccctccgacggccccgtgatgcagaagaagaccatgggctgggaggcctccaccgagcgcctgtacccccgcgacggcgtgctgaagggcgagacccacaaggccctgaagctgaaggacggcggccactacctggtggagttcaagtccatctacatggccaagaagcccgtgcagctgcccggctactactacgtggacgccaagctggacatcacctcccacaacgaggactacaccatcgtggagcagtacgagcgcaccgagggccgccaccacctgttcctgtag

SEQ ID NO: 23 - protein, 391 aa, Escherichia coli; identical to SEQ ID NO: 17

SEQ ID NO: 24 - DNA, 1176 bp, Escherichia coli
  source 1..1176: mol_type = unassigned DNA
atgcagaagctgatcaactcggtccagaactatgcctggggctccaagaccgccctgacggaactctacggcatggagaacccgtcgtcacaaccgatggccgagctgtggatgggtgctcatccgaagtcctcttctcgcgtgcagaatgcagcaggtgacatcgtgtcgctgcgggatgtgattgagtcagacaagtccacccttctgggtgaggctgtggccaagcgcttcggcgaactcccattcctcttcaaggtgctctgcgccgcacagccgctctcaatccaagtccaccccaacaagcataactccgagatcggattcgccaaggagaatgcggctggcatcccgatggacgccgctgagagaaactacaaagacccgaatcacaagccggagcttgtcttcgcactcacgccatttctcgctatgaacgcatttcgcgagttcagcgagatcgtcagcctgctccagccggtggcgggtgctcatccagcaatcgcgcatttcttgcagcagcctgatgccgaaaggctcagcgagctgttcgcgtcccttcttaacatgcagggagaggagaagtcccgcgcacttgcaatactcaagagcgcgctggactcacagcaaggagagccgtggcaaaccatacggctcatctccgagttctatcccgaggactcaggactgttctcgccgttgctgctcaacgtggtcaagctgaaccccggagaggcgatgttcttgttcgccgaaactccgcatgcttacctccaaggagtcgctctggaagtgatggccaattcggacaacgttcttcgggcaggattgacgcccaagtacatcgacatcccggaactcgtggccaatgttaagtttgaagcgaagcctgccaaccagctgcttacgcagcctgttaagcagggagccgaactggatttccctattccggtggacgacttcgcattctccctccacgacctctcagacaaggagacgaccatctctcagcaaagcgctgcgattctgttctgcgtggaaggcgatgcgaccctgtggaagggctcacagcagcttcagctgaagcctggcgagtccgccttcatcgccgctaacgagtctcccgtcaccgtgaaagggcatgggaggctcgctcgggtctacaacaagctctag

SEQ ID NO: 25 - protein, 157 aa, Bacillus amyloliquefaciens
MMKMEGIALKKRLSWISVCLLVLVSAAGMLFSTAAKTETSSHKAHTEAQVINTFDGVADYLQTYHKLPDNYITKSEAQALGWVASKGNLADVAPGKSIGGDIFSNREGKLPGKSGRTWREADINYTSGFRNSDRILYSSDWLIYKTTDHYQTFTKIR

SEQ ID NO: 26 - DNA, 533 bp, Bacillus amyloliquefaciens
  source 1..533: mol_type = unassigned DNA
ctcatggcacaggttatcaacacgtttgacggggttgcggattatcttcagacatatcataagctacctgataattacattacaaaatcagaagcacaagccctcggctgggtggcatcaaaagggaaccttgcagacgtcgctccggggaaaagcatcggcggagacatcttctcaaacagggaaggcaaactcccgtaagtttctgcttctacctttgatatatatataataattatcattaattagtagtaatataatatttcaaatatttttttcaaaataaaagaatgtagtatatagcaattgcttttctgtagtttataagtgtgtatattttaatttataacttttctaatatatgaccaaaacatggtgatgtgcaggggcaaaagcggacgaacatggcgtgaagcggatattaactatacatcaggcttcagaaattcagaccggattctttactcaggcgactggctgatttacaaaacaacggaccattatcagacctttacaaaaatcagataactgca

SEQ ID NO: 27 - DNA, 482 bp, Cauliflower Mosaic Virus
  source 1..482: mol_type = unassigned DNA
catggagtcaaagattcaaatagaggacctaacagaactcgccgtaaagactggcgaacagttcatacagagtctcttacgactcaatgacaagaagaaaatcttcgtcaacatggtggagcacgacacgcttgtctactccaaaaatatcaaagatacagtctcagaagaccaaagggcaattgagacttttcaacaaagggtaatatccggaaacctcctcggattccattgcccagctatctgtcactttattgtgaagatagtggaaaaggaaggtggctcctacaaatgccatcattgcgataaaggaaaggccatcgttgaagatgcctctgccgacagtggtcccaaagatggacccccacccacgaggagcatcgtggaaaaagaagacgttccaaccacgtcttcaaagcaagtggattgatgtgatatctccactgacgtaagggatgacgcacaatcccactaagctgacc

SEQ ID NO: 28 - protein, 147 aa, Bacillus licheniformis
MAIEVKPINAEDTYDLRHRVLRPNQPIEVCMYETDLLRGAFHLGGFYGGKLISVASFHQAEHSELQGKKQYQLRGVATLEGYRDQKAGSSLVKHAEEILRKRGADMLWCNARTSASGYYEKLGFSEQGEVFETPPAGPHILMYKRLT

SEQ ID NO: 29 - protein, 444 aa, Bacillus licheniformis
ATGGCGATCGAGGTCAAGCCAATCAACGCCGAGGATACCTACGACCTCCGCCACAGGGTTTTGCGCCCGAACCAACCGATAGAAGTGTGCATGTACGAGACCGATCTTCTTCGCGGAGCGTTCCACCTTGGCGGCTTCTATGGCGGCAAGCTGATAAGCGTCGCGAGCTTCCACCAGGCAGAGCACAGCGAGCTCCAAGGCAAAAAGCAGTACCAACTGCGCGGCGTTGCGACCCTCGAGGGATATCGCGACCAGAAGGCTGGCAGCAGCCTTGTGAAGCACGCCGAAGAGATACTCAGGAAGAGAGGCGCCGACATGCTTTGGTGCAACGCCAGGACGAGCGCAAGCGGCTACTACGAAAAGCTTGGCTTCAGCGAGCAAGGAGAGGTCTTCGAAACGCCTCCCGCAGGCCCGCACATCCTCATGTATAAGCGCCTTACGTAG

SEQ ID NO: 30 - DNA, 1089 bp, Arabidopsis thaliana
  source 1..1089: mol_type = unassigned DNA
tttttgtgatctgatgataagtggttggttcgtgtctcatgcacttgggaggtgatctatttcacctggtgtagtttgtgtttccgtcagttggaaaaacttatccctatcgatttcgttttcattttctgcttttcttttatgtaccttcgtttgggcttgtaacgggcctttgtatttcaactctcaataataatccaagtgcatgttaaacaatttgtcatctgtttcggctttgatatactactggtgaagatgggccgtactactgcatcacaacgaaaaataataataagatgaaaaacttgaagtggaaaaaaaaaaaaacttgaatgttcactactactcattgaccataatgtttaacatacatagctcaatagtatttttgtgaatatggcaacacaaacagtccaaaacaattgtctcttactataccaaaccaagggcgccgcttgtttgccactctttgtgtgcaatagtgtgattaccacatctccacattcaatatattccctgaattatctgacgattttgatggctcactgttttcccaagtcttgaattgtcttctgtgcgccagtcaaatgcatatgtgttgagtttatcttttaaatatcaagcttttgtttttaacttttgtttgtaaccaaaaactcacagtaggagtttgatcacataattttatgtttgcctttgcaatttctagtgagtctttgattaaaagcttgaaaagaaaatgcagccaagcttaccaagtaagttatgtgtattaaccagaggaagagagaatcttgcaaaatttcaacaaacacaaaaagaagtattactacgattggtggagaaagaaaacgattccaaatcttgaactgttgttgtaaaagcatagcagaaagtgggagacaaccgaaatagaaatgactataacttaatttaatgttatcattataatttcttctagcaaatatttagaaagtaaatatcacatcaacctttaatgtaattaagctttctctttttgattcatgtgagatgaaaagaaaaaaaagaagagaaaagtgtagaaaacacatcatttctaagctgaag

SEQ ID NO: 31 - DNA, 745 bp, Zea mays
  source 1..745: mol_type = unassigned DNA
ttcttatgtgcttctagtctccaaatgtggttgatagttattttgctctaagatcaacagtaatgaagtataaatcatcgttgtggtgtgctactcggttaattgagcattaacacacacaaacatgacgaggatggtataatctccaaaaatgtgtactttgttaggtgggaccctatagccttgattaatgtgctatgttaggcatgcctggaaacgtgtgacgcatatgttttgtgaacctgttgatattatatgtgcttttatattaccatattttattaaaatactaatatttattactagtaagatataacattctatctagcttaaaaactaaccataaatattccataataactagatttaccaaactaatatactaaatatacataataaatacaaaattaacaagacaataatcaatatttatgagcttaatatatttagacattatggttggtcgacgataatcatgctaacttttcgtaattgcttgattgaaatatgcttagaataatgcctctttgttctacatggcaaatagggaccattatggtgtaacaccctgggaaccacaaacaccccgaaatgctactaaactacacaactaaccttcatatataaaatttcgacagcatctcctttgaaaatttgcatagacgtggaagcaacagagtataaacagatatcatgataagaaaacatactagacattaataatctgctagaaatgggaagaatc

SEQ ID NO: 32 - DNA, 1682 bp, Oryza sativa
  source 1..1682: mol_type = unassigned DNA
atccctcagccgcctttcactatcttttttgcccgagtcattgtcatgtgaaccttggcatgtataatcggtgaattgcgtcgattttcctcttataggtgggccaatgaatccgtgtgatcgcgtctgattggctagagatatgtttcttccttgttggatgtattttcatacataatcatatgcatacaaatatttcattacactttatagaaatggtcagtaataaaccctatcactatgtctggtgtttcattttatttgcttttaaacgaaaattgacttcctgattcaatatttaaggatcgtcaacggtgtgcagttactaaattctggtttgtaggaactatagtaaactattcaagtcttcacttattgtgcactcacctctcgccacatcaccacagatgttattcacgtcttaaatttgaactacacatcatattgacacaatattttttttaaataagcgattaaaacctagcctctatgtcaacaatggtgtacataaccagcgaagtttagggagtaaaaaacatcgccttacacaaagttcgctttaaaaaataaagagtaaattttactttggaccacccttcaaccaatgtttcactttagaacgagtaattttattattgtcactttggaccaccctcaaatcttttttccatctacatccaatttatcatgtcaaagaaatggtctacatacagctaaggagatttatcgacgaatagtagctagcatactcgaggtcattcatatgcttgagaagagagtcgggatagtccaaaataaaacaaaggtaagattacctggtcaaaagtgaaaacatcagttaaaaggtggtataaagtaaaatatcggtaataaaaggtggcccaaagtgaaatttactcttttctactattataaaaattgaggatgtttttgtcggtactttgatacgtcatttttgtatgaattggtttttaagtttattcgcttttggaaatgcatatctgtatttgagtcgggttttaagttcgtttgcttttgtaaatacagagggatttgtataagaaatatctttaaaaaaacccatatgctaatttgacataatttttgagaaaaatatatattcaggcgaattctcacaatgaacaataataagattaaaatagctttcccccgttgcagcgcatgggtattttttctagtaaaaataaaagataaacttagactcaaaacatttacaaaaacaacccctaaagttcctaaagcccaaagtgctatccacgatccatagcaagcccagcccaacccaacccaacccaacccaccccagtccagccaactggacaatagtctccacacccccccactatcaccgtgagttgtccgcacgcaccgcacgtctcgcagccaaaaaaaaaaaaagaaagaaaaaaaagaaaaagaaaaaacagcaggtgggtccgggtcgtgggggccggaaacgcgaggaggatcgcgagccagcgacgaggccggccctccctccgcttccaaagaaacgccccccatcgccactatatacatacccccccctctcctcccatccccccaaccctaccaccaccaccaccaccacctccacctcctcccccctcgctgccggacgacgagctcctcccccctccccctccgccgccgccgcgccg

SEQ ID NO: 33 - DNA, 462 bp, Oryza sativa
  source 1..462: mol_type = unassigned DNA
gtaaccaccccgcccctctcctctttctttctccgttttttttttccgtctcggtctcgatctttggccttggtagtttgggtgggcgagaggcggcttcgtgcgcgcccagatcggtgcgcgggaggggcgggatctcgcggctggggctctcgccggcgtggatcaggcccggatctcgcggggaatggggctctcggatgtagatctgcgatccgccgttgttgggggagatgatggggggtttaaaatttccgccatgctaaacaagatcaggaagaggggaaaagggcactatggtttatatttttatatatttctgctgcttcgtcaggcttagatgtgctagatctttctttcttctttttgtgggtagaatttgaatccctcagcattgttcatcggtagtttttcttttcatgatttgtgacaaatgcagcctcgtgcggagcttttttgtag

SEQ ID NO: 34 - protein, 183 aa, Streptomyces viridochromogenes
MSPERRPVEIRPATAADMAAVCDIVNHYIETSTVNFRTEPQTPQEWIDDLERLQDRYPWLVAEVEGVVAGIAYAGPWKARNAYDWTVESTVYVSHRHQRLGLGSTLYTHLLKSMEAQGFKSVVAVIGLPNDPSVRLHEALGYTARGTLRAAGYKHGGWHDVGFWQRDFELPAPPRPVRPVTQI

SEQ ID NO: 35 - DNA, 552 bp, Streptomyces viridochromogenes
  source 1..552: mol_type = unassigned DNA
atgtcccccgagcgccgccccgtcgagatccgcccggccaccgccgccgacatggccgccgtgtgcgacatcgtgaaccactacatcgagacctccaccgtgaacttccgcaccgagccgcagaccccgcaggagtggatcgacgacctggagcgcctccaggaccgctacccgtggctcgtggccgaggtggagggcgtggtggccggcatcgcctacgccggcccgtggaaggcccgcaacgcctacgactggaccgtggagtccaccgtgtacgtgtcccaccgccaccagcgcctcggcctcggctccaccctctacacccacctcctcaagagcatggaggcccagggcttcaagtccgtggtggccgtgatcggcctcccgaacgacccgtccgtgcgcctccacgaggccctcggctacaccgcccgcggcaccctgcgcgccgccggctacaagcacggcggctggcacgacgtcggcttctggcagcgcgacttcgagctgccggccccgccgcgcccggtgcgcccggtgacgcagatctga

SEQ ID NO: 36 - protein, 231 aa, synthetic construct
  REGION 1..231: note = Sequence from Zoanthus species
MAHSKHGLKEEMTMKYHMEGCVNGHKFVITGEGIGYPFKGKQTINLCVIEGGPLPFSEDILSAGFKYGDRIFTEYPQDIVDYFKNSCPAGYTWGRSFLFEDGAVCICNVDITVSVKENCIYHKSIFNGVNFPADGPVMKKMTTNWEASCEKIMPVPKQGILKGDVSMYLLLKDGGRYRCQFDTVYKAKSVPSKMPEWHFIQHKLLREDRSDAKNQKWQLTEHAIAFPSALA

SEQ ID NO: 37 - DNA, 696 bp, synthetic construct
  misc_feature 1..696: note = Sequence from Zoanthus species
  source 1..696: mol_type = other DNA
atggcccacagcaagcacggcctgaaggaggagatgaccatgaagtaccacatggagggctgcgtgaacggccacaagttcgtgatcaccggcgagggcatcggctaccccttcaagggcaagcagaccatcaacctgtgcgtgatcgagggcggccccctgcccttcagcgaggacatcctgagcgccggcttcaagtacggcgaccggatcttcaccgagtacccccaggacatcgtggactacttcaagaacagctgccccgccggctacacctggggccggagcttcctgttcgaggacggcgccgtgtgcatctgtaacgtggacatcaccgtgagcgtgaaggagaactgcatctaccacaagagcatcttcaacggcgtgaacttccccgccgacggccccgtgatgaagaagatgaccaccaactgggaggccagctgcgagaagatcatgcccgtgcctaagcagggcatcctgaagggcgacgtgagcatgtacctgctgctgaaggacggcggccggtaccggtgccagttcgacaccgtgtacaaggccaagagcgtgcccagcaagatgcccgagtggcacttcatccagcacaagctgctgcgggaggaccggagcgacgccaagaaccagaagtggcagctgaccgagcacgccatcgccttccccagcgccctggcctga

SEQ ID NO: 38 - protein, 207 aa, Escherichia coli
MARLDKSKVINSALELLNEVGIEGLTTRKLAQKLGVEQPTLYWHVKNKRALLDALAIEMLDRHHTHFCPLEGESWQDFLRNNAKSFRCALLSHRDGAKVHLGTRPTEKQYETLENQLAFLCQQGFSLENALYALSAVGHFTLGCVLEDQEHQVAKEERETPTTDSMPPLLRQAIELFDHQGAEPAFLFGLELIICGLEKQLKCESGS

SEQ ID NO: 39 - DNA, 624 bp, Escherichia coli
  source 1..624: mol_type = unassigned DNA
atggccagactcgacaagagcaaggtgatcaacagcgcactggagctgctgaacgaggtcggaatcgaaggcctcacaacccgtaaactcgcccagaagctcggggtagagcagcctacattgtattggcacgtcaagaacaagcgggctttgctagacgccctcgccattgagatgctcgataggcaccatacccacttctgccctttggaaggggaaagctggcaagacttcttgaggaacaacgctaagagcttcagatgtgctttgctcagtcaccgtgatggagccaaggtccacctaggtacacggcctacggagaagcagtatgaaactctcgagaaccagctcgccttcctgtgccaacaaggtttctcccttgagaatgccctctacgcactctccgctgtagggcacttcactctgggttgcgtattggaagatcaagagcaccaagtcgctaaggaggagagggaaacacctactactgatagtatgccgccactgctccgacaagctatcgagctcttcgatcaccaaggtgcagagccagccttcctgttcggccttgaattgatcatatgcggattggagaagcagctgaagtgtgaaagtgggtcttaa

SEQ ID NO: 40 - DNA, 19 bp, Escherichia coli
  source 1..19: mol_type = unassigned DNA
actctatcagtgatagagt

SEQ ID NO: 41 - DNA, 34 bp, synthetic construct
  misc_feature 1..34: note = LOX-FAS
  source 1..34: mol_type = other DNA
acaacttcgtatatacctttctatacgaagttgt

SEQ ID NO: 42 - DNA, 34 bp, synthetic construct
  misc_feature 1..34: note = LOX-2272
  source 1..34: mol_type = other DNA
ataacttcgtataggataccttatacgaagttat

SEQ ID NO: 43 - DNA, 9810 bp, synthetic construct
  misc_feature 1..9810: note = PHP70154
  source 1..9810: mol_type = other DNA
agcgtcagaccccgtagaaaagatcaaaggatcttcttgagatcctttttttctgcgcgtaatctgctgcttgcaaacaaaaaaaccaccgctaccagcggtggtttgtttgccggatcaagagctaccaactctttttccgaaggtaactggcttcagcagagcgcagataccaaatactgtccttctagtgtagccgtagttaggccaccacttcaagaactctgtagcaccgcctacatacctcgctctgctaatcctgttaccagtggctgctgccagtggcgataagtcgtgtcttaccgggttggactcaagacgatagttaccggataaggcgcagcggtcgggctgaacggggggttcgtgcacacagcccagcttggagcgaacgacctacaccgaactgagatacctacagcgtgagctatgagaaagcgccacgcttcccgaagggagaaaggcggacaggtatccggtaagcggcagggtcggaacaggagagcgcacgagggagcttccagggggaaacgcctggtatctttatagtcctgtcgggtttcgccacctctgacttgagcgtcgatttttgtgatgctcgtcaggggggcggagcctatggaaaaacgccagcaacgcggcctttttacggttcctggccttttgctggccttttgctcacatgttctttcctgcgttatcccctgattctgtggataaccgtattaccgcctttgagtgagctgataccgagcggataacaatttcacacaggaaacagctatgaccatgattacgccaagctatcaactttgtatagaaaagttgaagcttcgctgaaatcaccagtctctctctacaaatctatctctctctataataatgtgtgagtagttcccagataagggaattagggttcttatagggtttcgctcatgtgttgagcatataagaaacccttagtatgtatttgtatttgtaaaatacttctatcaataaaatttctaattcctaaaaccaaaatccagtggcgagctgctagcgaagttcctattccgaagttcctattctctagaaagtataggaacttcagatccaccggctagaggatccaccatggttgaacaagatggattgcacgcaggttctccggccgcttgggtggagaggctattcggctatgactgggcacaacagacaatcggctgctctgatgccgccgtgttccggctgtcagcgcaggggcgcccggttctttttgtcaagaccgacctgtccggtgccctgaatgaactgcaggacgaggcagcgcggctatcgtggctggccacgacgggcgttccttgcgcagctgtgctcgacgttgtcactgaagcgggaagggactggctgctattgggcgaagtgccggggcaggatctcctgtcatctcaccttgctcctgccgagaaagtatccatcatggctgatgcaatgcggcggctgcatacgcttgatccggctacctgcccattcgaccaccaagcgaaacatcgcatcgagcgagcacgtactcggatggaagccggtcttgtcgatcaggatgatctggacgaagagcatcaggggctcgcgccagccgaactgttcgccaggctcaaggcgcgcatgcccgacggcgatgatctcgtcgtgacccatggcgatgcctgcttgccgaatatcatggtggaaaatggccgcttttctggattcatcgactgtggccggctgggtgtggcggaccgctatcaggacatagcgttggctacccgtgatattgctgaagagcttggcggcgaatgggctgaccgcttcctcgtgctttacggtatcgccgctcccgattcgcagcgcatcgccttctatcgccttcttgacgagttcttctgaggatccaccatggttaacctagacttgtccatcttctggattggccaacttaattaatgtatgaaataaaaggatgcacacatagtgacatgctaatcactataatgtgggcatcaaagttgtgtgttatgtgtaattactagttatctgaataaaagagaaagagatcatccatatttcttatcctaaatgaatgtcacgtgtctttataattctttgatgaaccagatgcatttcattaaccaaatccatatacatataaatattaatcatatataattaatatcaattgggttagcaaaacaaatctagtctaggtgtgttttgcgaatgcggccgggtaccgagctcgaattcggcccaagtttgtacaaaaaagcaggctccggccagaatggcccggaccgaagctggccgctctagaactagtggatctcgatgtgtagtctacgagaagggttaaccgtctcttcgtgagaataaccgtggcctaaaaataagccgatgaggataaataaaatgtggtggtacagtacttcaagaggtttactcatcaagaggatgcttttccgatgagctctagtagtacatcggacctcacatacctccattgtggtgaaatattttgtgctcatttagtgatgggtaaattttgtttatgtcactctaggttttgacatttcagttttgccactcttaggttttgacaaataatttccattccgcggcaaaagcaaaacaattttattttacttttaccactcttagctttcacaatgtatcacaaatgccactctagaaattctgtttatgccacagaatgtgaaaaaaaacactcacttatttgaagccaaggtgttcatggcatggaaatgtgacataaagtaacgttcgtgtataagaaaaaattgtactcctcgtaacaagagacggaaacatcatgagacaatcgcgtttggaaggctttgcatcacctttggatgatgcgcatgaatggagtcgtctgcttgctagccttcgcctaccgcccactgagtccgggcggcaactaccatcggcgaacgacccagctgacctctaccgaccggacttgaatgcgctaccttcgtcagcgacgatggccgcgtacgctggcgacgtgcccccgcatgcatggcggcacatggcgagctcagaccgtgcgtggctggctacaaatacgtaccccgtgagtgccctagctagaaacttacacctgcaactgcgagagcgagcgtgtgagtgtagccgatagatccgcccatgagcgagctgattaaagagaacatgcacatgaagctgtacatggaggggaccgtcgacaaccaccacttcaagtgcacctccgagggcgagggtaagccgtatgagggcacgcagacaatgaggattaaagtggttgagggcgggccgctgcctttcgcattcgacatcctcgccaccagcttcctgtacgggtccaagaccttcatcaaccacacccagggcatccccgacttcttcaaacagtccttcccggagggtttcacgtgggagagggtgacaacctacgaagatggcggcgtgctgaccgccacgcaggatacatctctccaggacgggtgcctgatctacaacgtcaagatcaggggcgtcaacttcacgagcaacggcccggtcatgcagaagaagacgctcggctgggaagccttcacggagacactctaccccgccgacggcgggctggaaggtaggaacgacatggccctcaagctcgtgggcggcagccacctcatcgccaacatcaaaaccacctacaggagcaagaagcccgccaagaacctgaagatgcccggcgtgtactacgtcgactacaggctcgagagaattaaggaggccaacaacgagacgtacgtggagcagcacgaggttgcagttgccaggtactgcgacctgccgagcaagctcggccacaagctgaactagggatctcgatagggatctgttaacgatccccggcggtgtcccccactgaagaaactatgtgctgtagtatagccgctgcccgctggctagctagctagttgagtcatttagcggcgatgattgagtaataatgtgtcacgcatcaccatgcatgggtggcagtgtcagtgtgagcaatgacctgaatgaacaattgaaatgaaaagaaaaaagtattgttccaaattaaacgttttaaccttttaataggtttatacaataattgatatatgttttctgtatatgtctaatttgttatcatccatttagatatagacaaaaaaaatctaagaactaaaacaaatgctaatttgaaatgaagggagtatatattgggataatgtcgatgagatccctcgtaatatcaccgacatcacacgtgtccagttaatgtatcagtgatacgtgtattcacatttgttgcgcgtaggcgtacccaacaattttgatcgactatcagaaagtcaacggaagcgagtcgacctcgagggggggccccggccgaagcttgcatgcctgcaggtcgactctagaggatctgcaccggacactgtctggtggcataccagacagtccggtgtgccagatcagggcacccttcggttcctttgctcctttgcttttgaaccctaactttgatcgtttattggtttgtgttgaacctttatgcacctgtggaatatataatctagaacaaactagttagtccaatcatttgtgttgggcattcaaccaccaaaattatttataggaaaaggttaaaccttatttccctttcaatctccccctttttggtgattgatgccaacacaaaccaaagaaaatatataagtgcagaattgaactagtttgcataaggtaagtgcataggttacttagaattaaatcaatttatacttttacttgatatgcatggttgctttcttttattttaacattttggaccacatttgcaccacttgttttgttttttgcaaatctttttggaaattctttttcaaagtcttttgcaaatagtcaaaggtatatgaataagattgtaagaagcattttcaagatttgaaatttctccccctgtttcaaatgcttttcctttgactaaacaaaactccccctgaataaaattctcctcttagctttcaagagggttttaaatagatatcaattggaaatatatttagatgctaattttgaaaatataccaattgaaaatcaacataccaatttgaaattaaacataccaatttaaaaaatttcaaaaagtggtggtgcggtccttttgctttgggcttaatatttctccccctttggcattaatcgccaaaaacggagactttgtgagccatttatactttctccccattggtaaatgaaatatgagtgaaagattataccaaatttggacagtgatgcggagtgacggcgaaggataaacgataccgttagagtggagtggaagccttgtcttcgccgaagactccatttccctttcaatctacgacttagcatagaaatacacttgaaaacacattagtcgtagccacgaaagagatatgatcaaaggtatacaaatgagctatgtgtgtaatgtttcaatcaaagtttcgagaatcaagaatatttagctcattcctaagtttgctaaaggttttatcatctaatggtttggtaaagatatcgactaattgttctttggtgctaacataagcaatctcgatatcacccctttgttggtgatccctcaaaaagtgataccgaatgtctatgtgcttagtgcggctgtgttcaacgggattatccgccatgcagatagcactctcattgtcacataggagagggactttgctcaatttgtagccatagtccctaaggttttgcctcatccaaagtaattgcacacaacaatgtcctgcggcaatatacttggcttcggcggtagaaagagctattgagttttgtttctttgaagtccaagacaccagggatctccctagaaactgacaagtccctgatgtgctcttcctatcaattttacaccctgcccaatcggcatctgaatatcctattaaatcaaaggtggatcccttggggtaccaaatttaaggagtgtaaactaaatatctcatgattcttttcacggccctaaggtgaacttccttaggatcggcttggaatcttgcacacatgcatatagaaagcatagctatctggtcgagatgcacataaatagagtaaagatcctatcatcgaccggtataccttttggtcgtacggatttacctcccgtgtcgaggtcgagatgcccattagttcccatgggtgtacctgatgggcttggcatccttcattccaaacttgttgagtatgtcttgaatgtactttgtttggctgatgaaggtgccatcttggagttgcttgacttgaaatcctagaaaatatttcaacttccccatcatagacatctcgaatttcggaatcatgatcctactaaactcttcacaagtagatttgttagtagacccaaatataatatcatcaacataaatttggcatacaaacaaaacttttgaaatggttttagtaaagagagtaggatcggctttactgactctgaagccattagtgataagaaaatctcttaggcattcataccatgctgttggggcttgcttgagcccataaagcgcctttgagagtttataaacatggttagggtactcactatcttcaaagccgagaggttgctcaacatagacctattcaccccatttgatcacttttttggtccttcaggatctaatagttatgtataatttagagtctcttgtttaatggccagatatttctaattaatctaagaatttatgatattttttaattttttatcatgtctgatgagaattaacataaaggctcaattgggtcctgaattaataatagagtgaaaattaatccagaggctctattagaaccttcaattagtaataccaagatatatataagatagtagagtatagtttaaatgttggcattgttcattctttcttttgttatttaatttatgctttccacggtggttagtggttacttctgaagggtccaaataatgcatgaagagtttgaggacaagaagtctgccctaaaaatagcgatgcaaaggcatggtgtccaagccatacatatagcgcactaattttatcagcagaacaatggtatttataggtcctagtgcccaggcaacaagagacacgaataaagcatcgatcacgacaccagatctcatggcacaggttatcaacacgtttgacggggttgcggattatcttcagacatatcataagctacctgataattacattacaaaatcagaagcacaagccctcggctgggtggcatcaaaagggaaccttgcagacgtcgctccggggaaaagcatcggcggagacatcttctcaaacagggaaggcaaactcccgtaagtttctgcttctacctttgatatatatataataattatcattaattagtagtaatataatatttcaaatatttttttcaaaataaaagaatgtagtatatagcaattgcttttctgtagtttataagtgtgtatattttaatttataacttttctaatatatgaccaaaacatggtgatgtgcaggggcaaaagcggacgaacatggcgtgaagcggatattaactatacatcaggcttcagaaattcagaccggattctttactcaggcgactggctgatttacaaaacaacggaccattatcagacctttacaaaaatcagataactgcagctagacttgtccatcttctggattggccaacttaattaatgtatgaaataaaaggatgcacacatagtgacatgctaatcactataatgtgggcatcaaagttgtgtgttatgtgtaattactagttatctgaataaaagagaaagagatcatccatatttcttatcctaaatgaatgtcacgtgtctttataattctttgatgaaccagatgcatttcattaaccaaatccatatacatataaatattaatcatatataattaatatcaattgggttagcaaaacaaatctagggtcacccggtccgggcctagaaggccgatctcccgggcacccagctttcttgtacaaagtggccgttaacggatcccggtgaagttcctattccgaagttcctattctccagaaagtataggaacttcactagagcttgcggccgccccgggcaactttattatacatagttgataattcactggccgtcgttttacaacgtcgtgactgggaaaaccctggcgttacccaacttaatcgccttgcagcacatccccctttcgccagctggcgtaatagcgaagaggcccgcaccgatcgcccttcccaacagttgcgcagcctgaatggcgaatggcgcctgatgcggtattttctccttacgcatctgtgcggtatttcacaccgcatatggtgcactctcagtacaatctgctctgatgccgcatagttaagccagccccgacacccgccaacacccgctgacgcgccctgacgggcttgtctgctcccggcatccgcttacagacaagctgtgaccgtctccgggagctgcatgtgtcagaggttttcaccgtcatcaccgaaacgcgcgagacgaaagggcctcgtgatacgcctatttttataggttaatgtcatgataataatggtttcttagacgtcaggtggcacttttcggggaaatgtgcgcggaacccctatttgtttatttttctaaatacattcaaatatgtatccgctcatgagacaataaccctgataaatgcttcaataatattgaaaaaggaagagtatgagtattcaacatttccgtgtcgcccttattcccttttttgcggcattttgccttcctgtttttgctcacccagaaacgctggtgaaagtaaaagatgctgaagatcagttgggtgcacgagtgggttacatcgaactggatctcaacagcggtaagatccttgagagttttcgccccgaagaacgttttccaatgatgagcacttttaaagttctgctatgtggcgcggtattatcccgtattgacgccgggcaagagcaactcggtcgccgcatacactattctcagaatgacttggttgagtactcaccagtcacagaaaagcatcttacggatggcatgacagtaagagaattatgcagtgctgccataaccatgagtgataacactgcggccaacttacttctgacaacgatcggaggaccgaaggagctaaccgcttttttgcacaacatgggggatcatgtaactcgccttgatcgttgggaaccggagctgaatgaagccataccaaacgacgagcgtgacaccacgatgcctgtagcaatggcaacaacgttgcgcaaactattaactggcgaactacttactctagcttcccggcaacaattaatagactggatggaggcggataaagttgcaggaccacttctgcgctcggcccttccggctggctggtttattgctgataaatctggagccggtgagcgtgggtctcgcggtatcattgcagcactggggccagatggtaagccctcccgtatcgtagttatctacacgacggggagtcaggcaactatggatgaacgaaatagacagatcgctgagataggtgcctcactgattaagcattggtaactgtcagaccaagtttactcatatatactttagattgatttaaaacttcatttttaatttaaaaggatctaggtgaagatcctttttgataatctcatgaccaaaatcccttaacgtgagttttcgttccactg

SEQ ID NO: 44 - DNA, 8485 bp, synthetic construct
  misc_feature 1..8485: note = FRT1-FRT87 from PHP69519
  source 1..8485: mol_type = other DNA
gaagttcctattccgaagttcctattctctagaaagtataggaacttcagatccaccggctagaggatccaccatggttgaacaagatggattgcacgcaggttctccggccgcttgggtggagaggctattcggctatgactgggcacaacagacaatcggctgctctgatgccgccgtgttccggctgtcagcgcaggggcgcccggttctttttgtcaagaccgacctgtccggtgccctgaatgaactgcaggacgaggcagcgcggctatcgtggctggccacgacgggcgttccttgcgcagctgtgctcgacgttgtcactgaagcgggaagggactggctgctattgggcgaagtgccggggcaggatctcctgtcatctcaccttgctcctgccgagaaagtatccatcatggctgatgcaatgcggcggctgcatacgcttgatccggctacctgcccattcgaccaccaagcgaaacatcgcatcgagcgagcacgtactcggatggaagccggtcttgtcgatcaggatgatctggacgaagagcatcaggggctcgcgccagccgaactgttcgccaggctcaaggcgcgcatgcccgacggcgatgatctcgtcgtgacccatggcgatgcctgcttgccgaatatcatggtggaaaatggccgcttttctggattcatcgactgtggccggctgggtgtggcggaccgctatcaggacatagcgttggctacccgtgatattgctgaagagcttggcggcgaatgggctgaccgcttcctcgtgctttacggtatcgccgctcccgattcgcagcgcatcgccttctatcgccttcttgacgagttcttctgaggatccaccatggttaacctagacttgtccatcttctggattggccaacttaattaatgtatgaaataaaaggatgcacacatagtgacatgctaatcactataatgtgggcatcaaagttgtgtgttatgtgtaattactagttatctgaataaaagagaaagagatcatccatatttcttatcctaaatgaatgtcacgtgtctttataattctttgatgaaccagatgcatttcattaaccaaatccatatacatataaatattaatcatatataattaatatcaattgggttagcaaaacaaatctagtctaggtgtgttttgcgaattgcggccgggtaccgagctcgaattcggcccaagtttgtacaaaaaagcaggctccggccagaatggcccggaccgaagctggccgctctagaactaggtaagtgactagggtcacatcgaattgggatctaggagcttgtaggagcttgctaggagcttgcatgcgcggccgcgaggtcatcacatcaatccacttgctttgaagacgtggttggaacgtcttctttttccacgatgctcctcgtgggtgggggtccatctttgggaccactgtcggcagaggcatcttcaacgatggcctttcctttatcgcaatgatggcatttgtaggagccaccttccttttccactatcttcacaataaagtgacagatagctgggcaatggaatccgaggaggtttccggatattaccctttgttgaaaagtctcaattgccctttggtcttctgagactgtatctttgatatttttggagtagacaagcgtgtcgtgctccaccatgttgacgaagattttcttcttgtcattgagtcgtaagagactctgtatgaactgttcgccagtctttacggcgagttctgttaggtcctctatttgaatctttgactccatggacggtatcgataagctagcttgatatcacatcaatccacttgctttgaagacgtggttggaacgtcttctttttccacgatgctcctcgtgggtgggggtccatctttgggaccactgtcggcagaggcatcttcaacgatggcctttcctttatcgcaatgatggcatttgtaggagccaccttccttttccactatcttcacaataaagtgacagatagctgggcaatggaatccgaggaggtttccggatattaccctttgttgaaaagtctcaattgccctttggtcttctgagactgtatctttgatatttttggagtagacaagcgtgtcgtgctccaccatgttgacgaagattttcttcttgtcattgagtcgtaagagactctgtatgaactgttcgccagtctttacggcgagttctgttaggtcctctatttgaatctttgactccatgatcgaattatcacatcaatccacttgctttgaagacgtggttggaacgtcttctttttccacgatgctcctcgtgggtgggggtccatctttgggaccactgtcggcagaggcatcttcaacgatggcctttcctttatcgcaatgatggcatttgtaggagccaccttccttttccactatcttcacaataaagtgacagatagctgggcaatggaatccgaggaggtttccggatattaccctttgttgaaaagtctcaattgccctttggtcttctgagactgtatctttgatatttttggagtagacaagcgtgtcgtgctccaccatgttgacgaagattttcttcttgtcattgagtcgtaagagactctgtatgaactgttcgccagtctttacggcgagttctgttaggtcctctatttgaatctttgactccatgggaattcctgcagccgcagtgcagcgtgacccggtcgtgcccctctctagagataatgagcattgcatgtctaagttataaaaaattaccacatattttttttgtcacacttgtttgaagtgcagtttatctatctttatacatatatttaaactttactctacgaataatataatctatagtactacaataatatcagtgttttagagaatcatataaatgaacagttagacatggtctaaaggacaattgagtattttgacaacaggactctacagttttatctttttagtgtgcatgtgttctcctttttttttgcaaatagcttcacctatataatacttcatccattttattagtacatccatttagggtttagggttaatggtttttatagactaatttttttagtacatctattttattctattttagcctctaaattaagaaaactaaaactctattttagtttttttatttaataatttagatataaaatagaataaaataaagtgactaaaaattaaacaaataccctttaagaaattaaaaaaactaaggaaacatttttcttgtttcgagtagataatgccagcctgttaaacgccgtcgacgagtctaacggacaccaaccagcgaaccagcagcgtcgcgtcgggccaagcgaagcagacggcacggcatctctgtcgctgcctctggacccctctcgagagttccgctccaccgttggacttgctccgctgtcggcatccagaaattgcgtggcggagcggcagacgtgagccggcacggcaggcggcctcctcctcctctcacggcaccggcagctacgggggattcctttcccaccgctccttcgctttcccttcctcgcccgccgtaataaatagacaccccctccacaccctctttccccaacctcgtgttgttcggagcgcacacacacacaaccagatctcccccaaatccacccgtcggcacctccgcttcaaggtacgccgctcgtcctcccccccccccctctctaccttctctagatcggcgttccggtccatggttagggcccggtagttctacttctgttcatgtttgtgttagatccgtgtttgtgttagatccgtgctgctagcgttcgtacacggatgcgacctgtacgtcagacacgttctgattgctaacttgccagtgtttctctttggggaatcctgggatggctctagccgttccgcagacgggatcgatttcatgattttttttgtttcgttgcatagggtttggtttgcccttttcctttatttcaatatatgccgtgcacttgtttgtcgggtcatcttttcatgcttttttttgtcttggttgtgatgatgtggtctggttgggcggtcgttctagatcggagtagaattctgtttcaaactacctggtggatttattaattttggatctgtatgtgtgtgccatacatattcatagttacgaattgaagatgatggatggaaatatcgatctaggataggtatacatgttgatgcgggttttactgatgcatatacagagatgctttttgttcgcttggttgtgatgatgtggtgtggttgggcggtcgttcattcgttctagatcggagtagaatactgtttcaaactacctggtgtatttattaattttggaactgtatgtgtgtgtcatacatcttcatagttacgagtttaagatggatggaaatatcgatctaggataggtatacatgttgatgtgggttttactgatgcatatacatgatggcatatgcagcatctattcatatgctctaaccttgagtacctatctattataataaacaagtatgttttataattattttgatcttgatatacttggatgatggcatatgcagcagctatatgtggatttttttagccctgccttcatacgctatttatttgcttggtactgtttcttttgtcgatgctcaccctgttgtttggtgttacttctgcagactagtatggcgatcgaggtcaagccaatcaacgccgaggatacctacgacctccgccacagggttttgcgcccgaaccaaccgatagaagtgtgcatgtacgagaccgatcttcttcgcggagcgttccaccttggcggcttctatggcggcaagctgataagcgtcgcgagcttccaccaggcagagcacagcgagctccaaggcaaaaagcagtaccaactgcgcggcgttgcgaccctcgagggatatcgcgaccagaaggctggcagcagccttgtgaagcacgccgaagagatactcaggaagagaggcgccgacatgctttggtgcaacgccaggacgagcgcaagcggctactacgaaaagcttggcttcagcgagcaaggagaggtcttcgaaacgcctcccgcaggcccgcacatcctcatgtataagcgccttacgtagggatccgtttttgtgatctgatgataagtggttggttcgtgtctcatgcacttgggaggtgatctatttcacctggtgtagtttgtgtttccgtcagttggaaaaacttatccctatcgatttcgttttcattttctgcttttcttttatgtaccttcgtttgggcttgtaacgggcctttgtatttcaactctcaataataatccaagtgcatgttaaacaatttgtcatctgtttcggctttgatatactactggtgaagatgggccgtactactgcatcacaacgaaaaataataataagatgaaaaacttgaagtggaaaaaaaaaaaaacttgaatgttcactactactcattgaccataatgtttaacatacatagctcaatagtatttttgtgaatatggcaacacaaacagtccaaaacaattgtctcttactataccaaaccaagggcgccgcttgtttgccactctttgtgtgcaatagtgtgattaccacatctccacattcaatatattccctgaattatctgacgattttgatggctcactgttttcccaagtcttgaattgtcttctgtgcgccagtcaaatgcatatgtgttgagtttatcttttaaatatcaagcttttgtttttaacttttgtttgtaaccaaaaactcacagtaggagtttgatcacataattttatgtttgcctttgcaatttctagtgagtctttgattaaaagcttgaaaagaaaatgcagccaagcttaccaagtaagttatgtgtattaaccagaggaagagagaatcttgcaaaatttcaacaaacacaaaaagaagtattactacgattggtggagaaagaaaacgattccaaatcttgaactgttgttgtaaaagcatagcagaaagtgggagacaaccgaaatagaaatgactataacttaatttaatgttatcattataatttcttctagcaaatatttagaaagtaaatatcacatcaacctttaatgtaattaagctttctctttttgattcatgtgagatgaaaagaaaaaaaagaagagaaaagtgtagaaaacacatcatttctaagctgaagcctagtggatctcgatgtgtagtctacgagaagggttaaccgtctcttcgtgagaataaccgtggcctaaaaataagccgatgaggataaataaaatgtggtggtacagtacttcaagaggtttactcatcaagaggatgcttttccgatgagctctagtagtacatcggacctcacatacctccattgtggtgaaatattttgtgctcatttagtgatgggtaaattttgtttatgtcactctaggttttgacatttcagttttgccactcttaggttttgacaaataatttccattccgcggcaaaagcaaaacaattttattttacttttaccactcttagctttcacaatgtatcacaaatgccactctagaaattctgtttatgccacagaatgtgaaaaaaaacactcacttatttgaagccaaggtgttcatggcatggaaatgtgacataaagtaacgttcgtgtataagaaaaaattgtactcctcgtaacaagagacggaaacatcatgagacaatcgcgtttggaaggctttgcatcacctttggatgatgcgcatgaatggagtcgtctgcttgctagccttcgcctaccgcccactgagtccgggcggcaactaccatcggcgaacgacccagctgacctctaccgaccggacttgaatgcgctaccttcgtcagcgacgatggccgcgtacgctggcgacgtgcccccgcatgcatggcggcacatggcgagctcagaccgtgcgtggctggctacaaatacgtaccccgtgagtgccctagctagaaacttacacctgcaactgcgagagcgagcgtgtgagtgtagccgatagatccgcccatggcctcctccgagaacgtcatcaccgagttcatgcgcttcaaggtgcgcatggagggcaccgtgaacggccacgagttcgagatcgagggcgagggcgagggccgcccctacgagggccacaacaccgtgaagctgaaggtgaccaagggcggccccctgcccttcgcctgggacatcctgtccccccagttccagtacggctccaaggtgtacgtgaagcaccccgccgacatccccgactacaagaagctgtccttccccgagggcttcaagtgggagcgcgtgatgaacttcgaggacggcggcgtggcgaccgtgacccaggactcctccctgcaggacggctgcttcatctacaaggtgaagttcatcggcgtgaacttcccctccgacggccccgtgatgcagaagaagaccatgggctgggaggcctccaccgagcgcctgtacccccgcgacggcgtgctgaagggcgagacccacaaggccctgaagctgaaggacggcggccactacctggtggagttcaagtccatctacatggccaagaagcccgtgcagctgcccggctactactacgtggacgccaagctggacatcacctcccacaacgaggactacaccatcgtggagcagtacgagcgcaccgagggccgccaccacctgttcctgtagggatctcgatagggatctgttaacgatccccggcggtgtcccccactgaagaaactatgtgctgtagtatagccgctgcccgctggctagctagctagttgagtcatttagcggcgatgattgagtaataatgtgtcacgcatcaccatgcatgggtggcagtgtcagtgtgagcaatgacctgaatgaacaattgaaatgaaaagaaaaaagtattgttccaaattaaacgttttaaccttttaataggtttatacaataattgatatatgttttctgtatatgtctaatttgttatcatccatttagatatagacaaaaaaaatctaagaactaaaacaaatgctaatttgaaatgaagggagtatatattgggataatgtcgatgagatccctcgtaatatcaccgacatcacacgtgtccagttaatgtatcagtgatacgtgtattcacatttgttgcgcgtaggcgtacccaacaattttgatcgactatcagaaagtcaacggaagcgagtcgacctcgagggggggccccggccgaagcttggtcacccggtccgggcctagaaggccgatctcccgggcacccagctttcttgtacaaagtggccgttaacggatcccggtgaagttcctattccgaagttcctattctccagaaagtataggaacttc

SEQ ID NO: 45 - DNA, 3602 bp, synthetic construct
  misc_feature 1..3602: note = UBI PRO-FLPm-pinII
  source 1..3602: mol_type = other DNA
ctgcagtgcagcgtgacccggtcgtgcccctctctagagataatgagcattgcatgtctaagttataaaaaattaccacatattttttttgtcacacttgtttgaagtgcagtttatctatctttatacatatatttaaactttactctacgaataatataatctatagtactacaataatatcagtgttttagagaatcatataaatgaacagttagacatggtctaaaggacaattgagtattttgacaacaggactctacagttttatctttttagtgtgcatgtgttctcctttttttttgcaaatagcttcacctatataatacttcatccattttattagtacatccatttagggtttagggttaatggtttttatagactaatttttttagtacatctattttattctattttagcctctaaattaagaaaactaaaactctattttagtttttttatttaataatttagatataaaatagaataaaataaagtgactaaaaattaaacaaataccctttaagaaattaaaaaaactaaggaaacatttttcttgtttcgagtagataatgccagcctgttaaacgccgtcgacgagtctaacggacaccaaccagcgaaccagcagcgtcgcgtcgggccaagcgaagcagacggcacggcatctctgtcgctgcctctggacccctctcgagagttccgctccaccgttggacttgctccgctgtcggcatccagaaattgcgtggcggagcggcagacgtgagccggcacggcaggcggcctcctcctcctctcacggcacggcagctacgggggattcctttcccaccgctccttcgctttcccttcctcgcccgccgtaataaatagacaccccctccacaccctctttccccaacctcgtgttgttcggagcgcacacacacacaaccagatctcccccaaatccacccgtcggcacctccgcttcaaggtacgccgctcgtcctccccccccccccctctctaccttctctagatcggcgttccggtccatggttagggcccggtagttctacttctgttcatgtttgtgttagatccgtgtttgtgttagatccgtgctgctagcgttcgtacacggatgcgacctgtacgtcagacacgttctgattgctaacttgccagtgtttctctttggggaatcctgggatggctctagccgttccgcagacgggatcgatttcatgattttttttgtttcgttgcatagggtttggtttgcccttttcctttatttcaatatatgccgtgcacttgtttgtcgggtcatcttttcatgcttttttttgtcttggttgtgatgatgtggtctggttgggcggtcgttctagatcggagtagaattctgtttcaaactacctggtggatttattaattttggatctgtatgtgtgtgccatacatattcatagttacgaattgaagatgatggatggaaatatcgatctaggataggtatacatgttgatgcgggttttactgatgcatatacagagatgctttttgttcgcttggttgtgatgatgtggtgtggttgggcggtcgttcattcgttctagatcggagtagaatactgtttcaaactacctggtgtatttattaattttggaactgtatgtgtgtgtcatacatcttcatagttacgagtttaagatggatggaaatatcgatctaggataggtatacatgttgatgtgggttttactgatgcatatacatgatggcatatgcagcatctattcatatgctctaaccttgagtacctatctattataataaacaagtatgttttataattattttgatcttgatatacttggatgatggcatatgcagcagctatatgtggatttttttagccctgccttcatacgctatttatttgcttggtactgtttcttttgtcgatgctcaccctgttgtttggtgttacttctgcaggtcgactctagaggatccaacaatgccccagttcgacatcctctgcaagaccccccccaaggtgctcgtgaggcagttcgtggagaggttcgagaggccctccggcgagaagatcgccctctgcgccgccgagctcacctacctctgctggatgatcacccacaacggcaccgccattaagagggccaccttcatgtcatacaacaccatcatctccaactccctctccttcgacatcgtgaacaagtccctccagttcaaatacaagacccagaaggccaccatcctcgaggcctccctcaagaagctcatccccgcctgggagttcaccatcatcccctactacggccagaagcaccagtccgacatcaccgacatcgtgtcatccctccagcttcagttcgagtcctccgaggaggctgacaagggcaactcccactccaagaagatgctgaaggccctcctctccgagggcgagtccatctgggagatcaccgagaagatcctcaactccttcgagtacacctccaggttcactaagaccaagaccctctaccagttcctcttcctcgccaccttcatcaactgcggcaggttctcagacatcaagaacgtggaccccaagtccttcaagctcgtgcagaacaagtacctcggcgtgatcatccagtgcctcgtgaccgagaccaagacctccgtgtccaggcacatctacttcttctccgctcgcggcaggatcgaccccctcgtgtacctcgacgagttcctcaggaactcagagcccgtgctcaagagggtgaacaggaccggcaactcctcctccaacaagcaggagtaccagctcctcaaggacaacctcgtgaggtcctacaacaaggccctcaagaagaacgccccctactccatcttcgccatcaagaacggccccaagtcccacatcggtaggcacctcatgacctccttcctctcaatgaagggcctcaccgagctcaccaacgtggtgggcaactggtccgacaagagggcctccgccgtggccaggaccacctacacccaccagatcaccgccatccccgaccactacttcgccctcgtgtcaaggtactacgcctacgaccccatctccaaggagatgatcgccctcaaggacgagactaaccccatcgaggagtggcagcacatcgagcagctcaagggctccgccgagggctccatcaggtaccccgcctggaacggcatcatctcccaggaggtgctcgactacctctcctcctacatcaacaggaggatctgagttaacctagacttgtccatcttctggattggccaacttaattaatgtatgaaataaaaggatgcacacatagtgacatgctaatcactataatgtgggcatcaaagttgtgtgttatgtgtaattactagttatctgaataaaagagaaagagatcatccatatttcttatcctaaatgaatgtcacgtgtctttataattctttgatgaaccagatgcatttcattaaccaaatccatatacatataaatattaatcatatataattaatatcaattgggttagcaaaacaaatctagtctaggtgtgttttgc

SEQ ID NO: 46 - DNA, 9305 bp, synthetic construct
  misc_feature 1..9305: note = FRT1-FRT87 fragment from PHP68884
  source 1..9305: mol_type = other DNA
gaagttcctattccgaagttcctattctctagaaagtataggaacttcagatccaccggctagaggatccaccatggttgaacaagatggattgcacgcaggttctccggccgcttgggtggagaggctattcggctatgactgggcacaacagacaatcggctgctctgatgccgccgtgttccggctgtcagcgcaggggcgcccggttctttttgtcaagaccgacctgtccggtgccctgaatgaactgcaggacgaggcagcgcggctatcgtggctggccacgacgggcgttccttgcgcagctgtgctcgacgttgtcactgaagcgggaagggactggctgctattgggcgaagtgccggggcaggatctcctgtcatctcaccttgctcctgccgagaaagtatccatcatggctgatgcaatgcggcggctgcatacgcttgatccggctacctgcccattcgaccaccaagcgaaacatcgcatcgagcgagcacgtactcggatggaagccggtcttgtcgatcaggatgatctggacgaagagcatcaggggctcgcgccagccgaactgttcgccaggctcaaggcgcgcatgcccgacggcgatgatctcgtcgtgacccatggcgatgcctgcttgccgaatatcatggtggaaaatggccgcttttctggattcatcgactgtggccggctgggtgtggcggaccgctatcaggacatagcgttggctacccgtgatattgctgaagagcttggcggcgaatgggctgaccgcttcctcgtgctttacggtatcgccgctcccgattcgcagcgcatcgccttctatcgccttcttgacgagttcttctgaggatccaccatggttaacctagacttgtccatcttctggattggccaacttaattaatgtatgaaataaaaggatgcacacatagtgacatgctaatcactataatgtgggcatcaaagttgtgtgttatgtgtaattactagttatctgaataaaagagaaagagatcatccatatttcttatcctaaatgaatgtcacgtgtctttataattctttgatgaaccagatgcatttcattaaccaaatccatatacatataaatattaatcatatataattaatatcaattgggttagcaaaacaaatctagtctaggtgtgttttgcgaatgcggccgggtaccgagctcgaattcggcccaagtttgtacaaaaaagcaggctccggccagaatggcccggaccgaagctggccgctctagaactaggcatggagtcaaagattcaaatagaggacctaacagaactcgccgtaaagactggcgaacagttcatacagagtctcttacgactcaatgacaagaagaaaatcttcgtcaacatggtggagcacgacacgcttgtctactccaaaaatatcaaagatacagtctcagaagaccaaagggcaattgagacttttcaacaaagggtaatatccggaaacctcctcggattccattgcccagctatctgtcactttattgtgaagatagtggaaaaggaaggtggctcctacaaatgccatcattgcgataaaggaaaggccatcgttgaagatgcctctgccgacagtggtcccaaagatggacccccacccacgaggagcatcgtggaaaaagaagacgttccaaccacgtcttcaaagcaagtggattgatgtgatatctccactgacgtaagggatgacgcacaatcccactaagctgacctagtggatctcgatgtgtagtctacgagaagggttaaccgtctcttcgtgagaataaccgtggcctaaaaataagccgatgaggataaataaaatgtggtggtacagtacttcaagaggtttactcatcaagaggatgcttttccgatgagctctagtagtacatcggacctcacatacctccattgtggtgaaatattttgtgctcatttagtgatgggtaaattttgtttatgtcactctaggttttgacatttcagttttgccactcttaggttttgacaaataatttccattccgcggcaaaagcaaaacaattttattttacttttaccactcttagctttcacaatgtatcacaaatgccactctagaaattctgtttatgccacagaatgtgaaaaaaaacactcacttatttgaagccaaggtgttcatggcatggaaatgtgacataaagtaacgttcgtgtataagaaaaaattgtactcctcgtaacaagagacggaaacatcatgagacaatcgcgtttggaaggctttgcatcacctttggatgatgcgcatgaatggagtcgtctgcttgctagccttcgcctaccgcccactgagtccgggcggcaactaccatcggcgaacgacccagctgacctctaccgaccggacttgaatgcgctaccttcgtcagcgacgatggccgcgtacgctggcgacgtgcccccgcatgcatggcggcacatggcgagctcagaccgtgcgtggctggctacaaatacgtaccccgtgagtgccctagctagaaacttacacctgcaactgcgagagcgagcgtgtgagtgtagccgatagatccgcccatgagcgagctgattaaagagaacatgcacatgaagctgtacatggaggggaccgtcgacaaccaccacttcaagtgcacctccgagggcgagggtaagccgtatgagggcacgcagacaatgaggattaaagtggttgagggcgggccgctgcctttcgcattcgacatcctcgccaccagcttcctgtacgggtccaagaccttcatcaaccacacccagggcatccccgacttcttcaaacagtccttcccggagggtttcacgtgggagagggtgacaacctacgaagatggcggcgtgctgaccgccacgcaggatacatctctccaggacgggtgcctgatctacaacgtcaagatcaggggcgtcaacttcacgagcaacggcccggtcatgcagaagaagacgctcggctgggaagccttcacggagacactctaccccgccgacggcgggctggaaggtaggaacgacatggccctcaagctcgtgggcggcagccacctcatcgccaacatcaaaaccacctacaggagcaagaagcccgccaagaacctgaagatgcccggcgtgtactacgtcgactacaggctcgagagaattaaggaggccaacaacgagacgtacgtggagcagcacgaggttgcagttgccaggtactgcgacctgccgagcaagctcggccacaagctgaactagggatctcgatagggatctgttaacgatccccggcggtgtcccccactgaagaaactatgtgctgtagtatagccgctgcccgctggctagctagctagttgagtcatttagcggcgatgattgagtaataatgtgtcacgcatcaccatgcatgggtggcagtgtcagtgtgagcaatgacctgaatgaacaattgaaatgaaaagaaaaaagtattgttccaaattaaacgttttaaccttttaataggtttatacaataattgatatatgttttctgtatatgtctaatttgttatcatccatttagatatagacaaaaaaaatctaagaactaaaacaaatgctaatttgaaatgaagggagtatatattgggataatgtcgatgagatccctcgtaatatcaccgacatcacacgtgtccagttaatgtatcagtgatacgtgtattcacatttgttgcgcgtaggcgtacccaacaattttgatcgactatcagaaagtcaacggaagcgagtcgacctcgaggcatggagtcaaagattcaaatagaggacctaacagaactcgccgtaaagactggcgaacagttcatacagagtctcttacgactcaatgacaagaagaaaatcttcgtcaacatggtggagcacgacacgcttgtctactccaaaaatatcaaagatacagtctcagaagaccaaagggcaattgagacttttcaacaaagggtaatatccggaaacctcctcggattccattgcccagctatctgtcactttattgtgaagatagtggaaaaggaaggtggctcctacaaatgccatcattgcgataaaggaaaggccatcgttgaagatgcctctgccgacagtggtcccaaagatggacccccacccacgaggagcatcgtggaaaaagaagacgttccaaccacgtcttcaaagcaagtggattgatgtgatatctccactgacgtaagggatgacgcacaatcccactaagctgaccgggcccggccgaagcttgcatgcctgcaggtcgactctagaggatctgcaccggacactgtctggtggcataccagacagtccggtgtgccagatcagggcacccttcggttcctttgctcctttgcttttgaaccctaactttgatcgtttattggtttgtgttgaacctttatgcacctgtggaatatataatctagaacaaactagttagtccaatcatttgtgttgggcattcaaccaccaaaattatttataggaaaaggttaaaccttatttccctttcaatctccccctttttggtgattgatgccaacacaaaccaaagaaaatatataagtgcagaattgaactagtttgcataaggtaagtgcataggttacttagaattaaatcaatttatacttttacttgatatgcatggttgctttcttttattttaacattttggaccacatttgcaccacttgttttgttttttgcaaatctttttggaaattctttttcaaagtcttttgcaaatagtcaaaggtatatgaataagattgtaagaagcattttcaagatttgaaatttctccccctgtttcaaatgcttttcctttgactaaacaaaactccccctgaataaaattctcctcttagctttcaagagggttttaaatagatatcaattggaaatatatttagatgctaattttgaaaatataccaattgaaaatcaacataccaatttgaaattaaacataccaatttaaaaaatttcaaaaagtggtggtgcggtccttttgctttgggcttaatatttctccccctttggcattaatcgccaaaaacggagactttgtgagccatttatactttctccccattggtaaatgaaatatgagtgaaagattataccaaatttggacagtgatgcggagtgacggcgaaggataaacgataccgttagagtggagtggaagccttgtcttcgccgaagactccatttccctttcaatctacgacttagcatagaaatacacttgaaaacacattagtcgtagccacgaaagagatatgatcaaaggtatacaaatgagctatgtgtgtaatgtttcaatcaaagtttcgagaatcaagaatatttagctcattcctaagtttgctaaaggttttatcatctaatggtttggtaaagatatcgactaattgttctttggtgctaacataagcaatctcgatatcacccctttgttggtgatccctcaaaaagtgataccgaatgtctatgtgcttagtgcggctgtgttcaacgggattatccgccatgcagatagcactctcattgtcacataggagagggactttgctcaatttgtagccatagtccctaaggttttgcctcatccaaagtaattgcacacaacaatgtcctgcggcaatatacttggcttcggcggtagaaagagctattgagttttgtttctttgaagtccaagacaccagggatctccctagaaactgacaagtccctgatgtgctcttcctatcaattttacaccctgcccaatcggcatctgaatatcctattaaatcaaaggtggatcccttggggtaccaaagaccaaatttaggagtgtaaactaaatatctcatgattcttttcacggccctaaggtgaacttccttaggatcggcttggaatcttgcacacatgcatatagaaagcatactatctggtcgagatgcacataaatagagtaaagatcctatcatcgaccggtataccttttggtctacggatttacctcccgtgtcgaggtcgagatgcccattagttcccatgggtgtcctgatgggcttggcatccttcattccaaacttgttgagtatgtcttgaatgtactttgtttggctgatgaaggtgccatcttggagttgcttgacttgaaatcctagaaaatatttcaacttccccatcatagacatctcgaatttcggaatcatgatcctactaaactcttcacaagtagatttgttagtagacccaaatataatatcatcaacataaatttggcatacaaacaaaacttttgaaatggttttagtaaagagagtaggatcggctttactgactctgaagccattagtgataagaaaatctcttaggcattcataccatgctgttggggcttgcttgagcccataaagcgcctttgagagtttataaacatggttagggtactcactatcttcaaagccgagaggttgctcaacatagacctattcaccccatttgatcacttttttggtccttcaggatctaatagttatgtataatttagagtctcttgtttaatggccagatatttctaattaatctaagaatttatgatattttttaattttttatcatgtctgatgagaattaacataaaggctcaattgggtcctgaattaataatagagtgaaaattaatccagaggctctattagaaccttcaattagtaataccaagatatatataagatagtagagtatagtttaaatgttggcattgttcattctttcttttgttatttaatttatgctttccacggtggttagtggttacttctgaagggtccaaataatgcatgaagagtttgaggacaagaagtctgccctaaaaatagcgatgcaaaggcatggtgtccaagccatacatatagcgcactaattttatcagcagaacaatggtatttataggtcctagtgcccaggcaacaagagacacgaataaagcatcgatcacgacaccatggcggcgacaatggcagtgacgacgatggtgacgaggagcaaggagagctggtcgtcattgcaggtcccggcggtggcattcccttggaagccacgaggtggcaagaccggcggcctcgagttccctcgccgggcgatgttcgccagcgtcggcctcaacgtgtgcccgggcgtcccggcggggcgcgacccgcgggagcccgatcccaaggtcgtccgggcggcctgcggcctggtccaggcacaagtcctcttccaggggtttaactgggagtcgtgcaagcagcagggaggctggtacaacaggctcaaggcccaggtcgacgacatcgccaaggccggcgtcacgcacgtctggctgcctccaccctcgcactccgtctcgccacaaggctacatgccaggccgcctatacgacctggacgcgtccaagtacggcacggcggcggagctcaagtccctgatagcggcgttccacggcaggggcgtgcagtgcgtggcggacatcgtcatcaaccaccggtgcgcggaaaagaaggacgcgcgcggcgtgtactgcatcttcgagggcgggactcccgacgaccgcctggactggggccccgggatgatctgcagcgacgacacgcagtactcggacgggacggggcaccgcgacacgggcgaggggttcgcggcggcgcccgacatcgaccacctcaacccgcgcgtgcagcgggagctctccgcctggctcaactggctcaggtccgacgccgtggggttcgacggctggcgcctcgacttcgccaagggctactcgccggccgtcgccagaatgtacgtggagagcacggggccgccgagcttcgtcgtcgcggagatatggaactcgctgagctacagcggggacggcaagccggcgcccaaccaggaccagtgccggcaggagctgctggactggacgcgggccgtcggcgggcccgccatggcgttcgacttccccaccaagggcctgctgcaggcgggcgtgcagggggagctgtggcggctgcgcgacagctccggcaacgcggccggcctgatcgggtgggcgcccgagaaggccgtcaccttcgtcgacaaccatgacaccgggtcgacgcagaagctctggccgttcccatccgacaaggtcatgcagggctacgcctacatcctcacccatccaggagtcccctgcattttctacgaccacatgttcgactggaacctgaagcaggagatatccacgctgtctgccatcagggcgcggaacggcatccgcgccgggagcaagctgcggatcctcgtggcggacgcggacgcgtacgtggccgtcgtcgacgagaaggtcatggtgaagatcgggacaaggtacggcgtgagcagcgtggtcccgtcggatttccacccggcggcgcacggcaaggactactgcgtctgggagaaagcgagcctccgcgtcccggcggggcgccacctctagcagctcagattgctcagtcttgtgctgcattgcaaacacagcagcacgacactgcataacgtcttttccttgagatctgacaaagcagcattagtccgttgatcggtggaagaccactcgtcagtgttgagttgaatgtttgatcaataaaatacggcaatgctgtaagggttgttttttatgccattgataatacactgtactgttcagttgttgaactctatttcttagccatgccaagtgcttttcttattttgaataacattacagcaaaaagttgaaagacaaaaaaaaaaacccccgaacagagtgctttgggtcccaagctactttagactgtgttcggcgttccccctaaatttctccccctatatctcactcacttgtcacatcagcgttctctttcccctatatctccacgtcgacgcggccgctctagaactagtggatcccccgggctgcaggaattcctcgagaccgtacgtgcgcgcgaatgcatccagatcttccctctagtcaaggccttaagcgcgcgttcgaacgcgcggttaagcttggtcacccggtccgggcctagaaggccgatctcccgggcacccagctttcttgtacaaagtggccgttaacggatcccggtgaagttcctattccgaagttcctattctccagaaagtataggaacttc

SEQ ID NO: 47 - DNA, 8962 bp, synthetic construct
  misc_feature 1..8962: note = T-DNA from PHP66566
  source 1..8962: mol_type = other DNA
gtttacccgccaatatatcctgtcaaacactgatagtttaaactgaaggcgggaaacgacaatctgatcatgagcggagaattaagggagtcacgttatgacccccgccgatgacgcgggacaagccgttttacgtttggaactgacagaaccgcaacgttgaaggagccactcagcaagctggtacgattgtaatacgactcactatagggcgaattgagcgctgtttaaacgctcttcaactggaagagcggttacgctgtttaaacgctcttcaactggaagagcggttactaccggttcactagctagctgctaaggttaccagagctggtcacctttgtccaccaacttattaagtatctagttgaagacacgttcttcttcacgtaagaagacactcagtagtcttcggccagaatggcctcttgattcagcgggcctagaaggccggatcactgactagctaatttaaatcctgataaggacccggcggaccgaagctggccgctctagaactaggctgcagtgcagcgtgacccggtcgtgcccctctctagagataatgagcattgcatgtctaagttataaaaaattaccacatattttttttgtcacacttgtttgaagtgcagtttatctatctttatacatatatttaaactttactctacgaataatataatctatagtactacaataatatcagtgttttagagaatcatataaatgaacagttagacatggtctaaaggacaattgagtattttgacaacaggactctacagttttatctttttagtgtgcatgtgttctcctttttttttgcaaatagcttcacctatataatacttcatccattttattagtacatccatttagggtttagggttaatggtttttatagactaatttttttagtacatctattttattctattttagcctctaaattaagaaaactaaaactctattttagtttttttatttaataatttagatataaaatagaataaaataaagtgactaaaaattaaacaaataccctttaagaaattaaaaaaactaaggaaacatttttcttgtttcgagtagataatgccagcctgttaaacgccgtcgacgagtctaacggacaccaaccagcgaaccagcagcgtcgcgtcgggccaagcgaagcagacggcacggcatctctgtcgctgcctctggacccctctcgagagttccgctccaccgttggacttgctccgctgtcggcatccagaaattgcgtggcggagcggcagacgtgagccggcacggcaggcggcctcctcctcctctcacggcaccggcagctacgggggattcctttcccaccgctccttcgctttcccttcctcgcccgccgtaataaatagacaccccctccacaccctctttccccaacctcgtgttgttcggagcgcacacacacacaaccagatctcccccaaatccacccgtcggcacctccgcttcaaggtacgccgctcgtcctcccccccccccctctctaccttctctagatcggcgttccggtccatgcatggttagggcccggtagttctacttctgttcatgtttgtgttagatccgtgtttgtgttagatccgtgctgctagcgttcgtacacggatgcgacctgtacgtcagacacgttctgattgctaacttgccagtgtttctctttggggaatcctgggatggctctagccgttccgcagacgggatcgatttcatgattttttttgtttcgttgcatagggtttggtttgcccttttcctttatttcaatatatgccgtgcacttgtttgtcgggtcatcttttcatgcttttttttgtcttggttgtgatgatgtggtctggttgggcggtcgttctagatcggagtagaattctgtttcaaactacctggtggatttattaattttggatctgtatgtgtgtgccatacatattcatagttacgaattgaagatgatggatggaaatatcgatctaggataggtatacatgttgatgcgggttttactgatgcatatacagagatgctttttgttcgcttggttgtgatgatgtggtgtggttgggcggtcgttcattcgttctagatcggagtagaatactgtttcaaactacctggtgtatttattaattttggaactgtatgtgtgtgtcatacatcttcatagttacgagtttaagatggatggaaatatcgatctaggataggtatacatgttgatgtgggttttactgatgcatatacatgatggcatatgcagcatctattcatatgctctaaccttgagtacctatctattataataaacaagtatgttttataattattttgatcttgatatacttggatgatggcatatgcagcagctatatgtggatttttttagccctgccttcatacgctatttatttgcttggtactgtttcttttgtcgatgctcaccctgttgtttggtgttacttctgcaggtcgactctagaggatccagcgagagcccaggatgaaaaaagcagtcattaacggggaacaaatcagaagtatcagcgacctccaccagacattgaaaaaggagcttgcccttccggaatactacggtgaaaacctggacgctttatgggattgtctgaccggatgggtggagtacccgctcgttttggaatggaggcagtttgaacaaagcaagcagctgactgaaaatggcgccgagagtgtgcttcaggttttccgtgaagcgaaagcggaaggctgcgacatcaccatcatactttcttaactgcagctagacttgtccatcttctggattggccaacttaattaatgtatgaaataaaaggatgcacacatagtgacatgctaatcactataatgtgggcatcaaagttgtgtgttatgtgtaattactagttatctgaataaaagagaaagagatcatccatatttcttatcctaaatgaatgtcacgtgtctttataattctttgatgaaccagatgcatttcattaaccaaatccatatacatataaatattaatcatatataattaatatcaattgggttagcaaaacaaatccctagtggatctcgatgtgtagtctacgagaagggttaaccgtctcttcgtgagaataaccgtggcctaaaaataagccgatgaggataaataaaatgtggtggtacagtacttcaagaggtttactcatcaagaggatgcttttccgatgagctctagtagtacatcggacctcacatacctccattgtggtgaaatattttgtgctcatttagtgatgggtaaattttgtttatgtcactctaggttttgacatttcagttttgccactcttaggttttgacaaataatttccattccgcggcaaaagcaaaacaattttattttacttttaccactcttagctttcacaatgtatcacaaatgccactctagaaattctgtttatgccacagaatgtgaaaaaaaacactcacttatttgaagccaaggtgttcatggcatggaaatgtgacataaagtaacgttcgtgtataagaaaaaattgtactcctcgtaacaagagacggaaacatcatgagacaatcgcgtttggaaggctttgcatcacctttggatgatgcgcatgaatggagtcgtctgcttgctagccttcgcctaccgcccactgagtccgggcggcaactaccatcggcgaacgacccagctgacctctaccgaccggacttgaatgcgctaccttcgtcagcgacgatggccgcgtacgctggcgacgtgcccccgcatgcatggcggcacatggcgagctcagaccgtgcgtggctggctacaaatacgtaccccgtgagtgccctagctagaaacttacacctgcaactgcgagagcgagcgtgtgagtgtagccgatagatccgcccatggcctcctccgagaacgtcatcaccgagttcatgcgcttcaaggtgcgcatggagggcaccgtgaacggccacgagttcgagatcgagggcgagggcgagggccgcccctacgagggccacaacaccgtgaagctgaaggtgaccaagggcggccccctgcccttcgcctgggacatcctgtccccccagttccagtacggctccaaggtgtacgtgaagcaccccgccgacatccccgactacaagaagctgtccttccccgagggcttcaagtgggagcgcgtgatgaacttcgaggacggcggcgtggcgaccgtgacccaggactcctccctgcaggacggctgcttcatctacaaggtgaagttcatcggcgtgaacttcccctccgacggccccgtgatgcagaagaagaccatgggctgggaggcctccaccgagcgcctgtacccccgcgacggcgtgctgaagggcgagacccacaaggccctgaagctgaaggacggcggccactacctggtggagttcaagtccatctacatggccaagaagcccgtgcagctgcccggctactactacgtggacgccaagctggacatcacctcccacaacgaggactacaccatcgtggagcagtacgagcgcaccgagggccgccaccacctgttcctgtagggatctcgatagggatctgttaacgatccccggcggtgtcccccactgaagaaactatgtgctgtagtatagccgctgcccgctggctagctagctagttgagtcatttagcggcgatgattgagtaataatgtgtcacgcatcaccatgcatgggtggcagtgtcagtgtgagcaatgacctgaatgaacaattgaaatgaaaagaaaaaagtattgttccaaattaaacgttttaaccttttaataggtttatacaataattgatatatgttttctgtatatgtctaatttgttatcatccatttagatatagacaaaaaaaatctaagaactaaaacaaatgctaatttgaaatgaagggagtatatattgggataatgtcgatgagatccctcgtaatatcaccgacatcacacgtgtccagttaatgtatcagtgatacgtgtattcacatttgttgcgcgtaggcgtacccaacaattttgatcgactatcagaaagtcaacggaagcgagtcgacctcgagggggggccccggccgaagcttgcatgcctgcagtgcagcgtgacccggtcgtgcccctctctagagataatgagcattgcatgtctaagttataaaaaattaccacatattttttttgtcacacttgtttgaagtgcagtttatctatctttatacatatatttaaactttactctacgaataatataatctatagtactacaataatatcagtgttttagagaatcatataaatgaacagttagacatggtctaaaggacaattgagtattttgacaacaggactctacagttttatctttttagtgtgcatgtgttctcctttttttttgcaaatagcttcacctatataatacttcatccattttattagtacatccatttagggtttagggttaatggtttttatagactaatttttttagtacatctattttattctattttagcctctaaattaagaaaactaaaactctattttagtttttttatttaataatttagatataaaatagaataaaataaagtgactaaaaattaaacaaataccctttaagaaattaaaaaaactaaggaaacatttttcttgtttcgagtagataatgccagcctgttaaacgccgtcgacgagtctaacggacaccaaccagcgaaccagcagcgtcgcgtcgggccaagcgaagcagacggcacggcatctctgtcgctgcctctggacccctctcgagagttccgctccaccgttggacttgctccgctgtcggcatccagaaattgcgtggcggagcggcagacgtgagccggcacggcaggcggcctcctcctcctctcacggcaccggcagctacgggggattcctttcccaccgctccttcgctttcccttcctcgcccgccgtaataaatagacaccccctccacaccctctttccccaacctcgtgttgttcggagcgcacacacacacaaccagatctcccccaaatccacccgtcggcacctccgcttcaaggtacgccgctcgtcctcccccccccccctctctaccttctctagatcggcgttccggtccatgcatggttagggcccggtagttctacttctgttcatgtttgtgttagatccgtgtttgtgttagatccgtgctgctagcgttcgtacacggatgcgacctgtacgtcagacacgttctgattgctaacttgccagtgtttctctttggggaatcctgggatggctctagccgttccgcagacgggatcgatttcatgattttttttgtttcgttgcatagggtttggtttgcccttttcctttatttcaatatatgccgtgcacttgtttgtcgggtcatcttttcatgcttttttttgtcttggttgtgatgatgtggtctggttgggcggtcgttctagatcggagtagaattctgtttcaaactacctggtggatttattaattttggatctgtatgtgtgtgccatacatattcatagttacgaattgaagatgatggatggaaatatcgatctaggataggtatacatgttgatgcgggttttactgatgcatatacagagatgctttttgttcgcttggttgtgatgatgtggtgtggttgggcggtcgttcattcgttctagatcggagtagaatactgtttcaaactacctggtgtatttattaattttggaactgtatgtgtgtgtcatacatcttcatagttacgagtttaagatggatggaaatatcgatctaggataggtatacatgttgatgtgggttttactgatgcatatacatgatggcatatgcagcatctattcatatgctctaaccttgagtacctatctattataataaacaagtatgttttataattattttgatcttgatatacttggatgatggcatatgcagcagctatatgtggatttttttagccctgccttcatacgctatttatttgcttggtactgtttcttttgtcgatgctcaccctgttgtttggtgttacttctgcaggtcgactctagaggatccatgcagaagctgatcaactcggtccagaactatgcctggggctccaagaccgccctgacggaactctacggcatggagaacccgtcgtcacaaccgatggccgagctgtggatgggtgctcatccgaagtcctcttctcgcgtgcagaatgcagcaggtgacatcgtgtcgctgcgggatgtgattgagtcagacaagtccacccttctgggtgaggctgtggccaagcgcttcggcgaactcccattcctcttcaaggtgctctgcgccgcacagccgctctcaatccaagtccaccccaacaagcataactccgagatcggattcgccaaggagaatgcggctggcatcccgatggacgccgctgagagaaactacaaagacccgaatcacaagccggagcttgtcttcgcactcacgccatttctcgctatgaacgcatttcgcgagttcagcgagatcgtcagcctgctccagccggtggcgggtgctcatccagcaatcgcgcatttcttgcagcagcctgatgccgaaaggctcagcgagctgttcgcgtcccttcttaacatgcagggagaggagaagtcccgcgcacttgcaatactcaagagcgcgctggactcacagcaaggagagccgtggcaaaccatacggctcatctccgagttctatcccgaggactcaggactgttctcgccgttgctgctcaacgtggtcaagctgaaccccggagaggcgatgttcttgttcgccgaaactccgcatgcttacctccaaggagtcgctctggaagtgatggccaattcggacaacgttcttcgggcaggattgacgcccaagtacatcgacatcccggaactcgtggccaatgttaagtttgaagcgaagcctgccaaccagctgcttacgcagcctgttaagcagggagccgaactggatttccctattccggtggacgacttcgcattctccctccacgacctctcagacaaggagacgaccatctctcagcaaagcgctgcgattctgttctgcgtggaaggcgatgcgaccctgtggaagggctcacagcagcttcagctgaagcctggcgagtccgccttcatcgccgctaacgagtctcccgtcaccgtgaaagggcatgggaggctcgctcgggtctacaacaagctctaggagcttactgaaaaaattaacatctcttgctaagatccatggatattcgaacgcgtaggtaccacatggttaacctagacttgtccatcttctggattggccaacttaattaatgtatgaaataaaaggatgcacacatagtgacatgctaatcactataatgtgggcatcaaagttgtgtgttatgtgtaattactagttatctgaataaaagagaaagagatcatccatatttcttatcctaaatgaatgtcacgtgtctttataattctttgatgaaccagatgcatttcattaaccaaatccatatacatataaatattaatcatatataattaatatcaattgggttagcaaaacaaatctagtctaggtgtgttttgcgaatgcggcctgtaccgagctcgaattcattccgattaatcgtggcctcttgctcttcaggatgaagagctatgtttaaacgtgcaagcgctactagacaattcagtacattaaaaacgtccgcaatgtgttattaagttgtctaagcgtcaatttgtttacaccacaatatatcct

SEQ ID NO: 48 - DNA, 9807 bp, synthetic construct
  misc_feature 1..9807: note = PHP71464
  source 1..9807: mol_type = other DNA
agcgtcagaccccgtagaaaagatcaaaggatcttcttgagatcctttttttctgcgcgtaatctgctgcttgcaaacaaaaaaaccaccgctaccagcggtggtttgtttgccggatcaagagctaccaactctttttccgaaggtaactggcttcagcagagcgcagataccaaatactgtccttctagtgtagccgtagttaggccaccacttcaagaactctgtagcaccgcctacatacctcgctctgctaatcctgttaccagtggctgctgccagtggcgataagtcgtgtcttaccgggttggactcaagacgatagttaccggataaggcgcagcggtcgggctgaacggggggttcgtgcacacagcccagcttggagcgaacgacctacaccgaactgagatacctacagcgtgagctatgagaaagcgccacgcttcccgaagggagaaaggcggacaggtatccggtaagcggcagggtcggaacaggagagcgcacgagggagcttccagggggaaacgcctggtatctttatagtcctgtcgggtttcgccacctctgacttgagcgtcgatttttgtgatgctcgtcaggggggcggagcctatggaaaaacgccagcaacgcggcctttttacggttcctggccttttgctggccttttgctcacatgttctttcctgcgttatcccctgattctgtggataaccgtattaccgcctttgagtgagctgataccgagcggataacaatttcacacaggaaacagctatgaccatgattacgccaagctatcaactttgtatagaaaagttgaagcttcgctgaaatcaccagtctctctctacaaatctatctctctctataataatgtgtgagtagttcccagataagggaattagggttcttatagggtttcgctcatgtgttgagcatataagaaacccttagtatgtatttgtatttgtaaaatacttctatcaataaaatttctaattcctaaaaccaaaatccagtggcgagctgctagcgaagttcctattccgaagttcctattctctagaaagtataggaacttcagatccaccggctagaggatccaccatggttgaacaagatggattgcacgcaggttctccggccgcttgggtggagaggctattcggctatgactgggcacaacagacaatcggctgctctgatgccgccgtgttccggctgtcagcgcaggggcgcccggttctttttgtcaagaccgacctgtccggtgccctgaatgaactgcaggacgaggcagcgcggctatcgtggctggccacgacgggcgttccttgcgcagctgtgctcgacgttgtcactgaagcgggaagggactggctgctattgggcgaagtgccggggcaggatctcctgtcatctcaccttgctcctgccgagaaagtatccatcatggctgatgcaatgcggcggctgcatacgcttgatccggctacctgcccattcgaccaccaagcgaaacatcgcatcgagcgagcacgtactcggatggaagccggtcttgtcgatcaggatgatctggacgaagagcatcaggggctcgcgccagccgaactgttcgccaggctcaaggcgcgcatgcccgacggcgatgatctcgtcgtgacccatggcgatgcctgcttgccgaatatcatggtggaaaatggccgcttttctggattcatcgactgtggccggctgggtgtggcggaccgctatcaggacatagcgttggctacccgtgatattgctgaagagcttggcggcgaatgggctgaccgcttcctcgtgctttacggtatcgccgctcccgattcgcagcgcatcgccttctatcgccttcttgacgagttcttctgaggatccaccatggttaacctagacttgtccatcttctggattggccaacttaattaatgtatgaaataaaaggatgcacacatagtgacatgctaatcactataatgtgggcatcaaagttgtgtgttatgtgtaattactagttatctgaataaaagagaaagagatcatccatatttcttatcctaaatgaatgtcacgtgtctttataattctttgatgaaccagatgcatttcattaaccaaatccatatacatataaatattaatcatatataattaatatcaattgggttagcaaaacaaatctagtctaggtgtgttttgcgaatgcggccgggtaccgagctcgaattcggcccaagtttgtacaaaaaagcaggctccggccagaatggcccggaccgaagctggccgctctagaactagtggatctcgatgtgtagtctacgagaagggttaaccgtctcttcgtgagaataaccgtggcctaaaaataagccgatgaggataaataaaatgtggtggtacagtacttcaagaggtttactcatcaagaggatgcttttccgatgagctctagtagtacatcggacctcacatacctccattgtggtgaaatattttgtgctcatttagtgatgggtaaattttgtttatgtcactctaggttttgacatttcagttttgccactcttaggttttgacaaataatttccattccgcggcaaaagcaaaacaattttattttacttttaccactcttagctttcacaatgtatcacaaatgccactctagaaattctgtttatgccacagaatgtgaaaaaaaacactcacttatttgaagccaaggtgttcatggcatggaaatgtgacataaagtaacgttcgtgtataagaaaaaattgtactcctcgtaacaagagacggaaacatcatgagacaatcgcgtttggaaggctttgcatcacctttggatgatgcgcatgaatggagtcgtctgcttgctagccttcgcctaccgcccactgagtccgggcggcaactaccatcggcgaacgacccagctgacctctaccgaccggacttgaatgcgctaccttcgtcagcgacgatggccgcgtacgctggcgacgtgcccccgcatgcatggcggcacatggcgagctcagaccgtgcgtggctggctacaaatacgtaccccgtgagtgccctagctagaaacttacacctgcaactgcgagagcgagcgtgtgagtgtagccgatagatccgcccatggcccacagcaagcacggcctgaaggaggagatgaccatgaagtaccacatggagggctgcgtgaacggccacaagttcgtgatcaccggcgagggcatcggctaccccttcaagggcaagcagaccatcaacctgtgcgtgatcgagggcggccccctgcccttcagcgaggacatcctgagcgccggcttcaagtacggcgaccggatcttcaccgagtacccccaggacatcgtggactacttcaagaacagctgccccgccggctacacctggggccggagcttcctgttcgaggacggcgccgtgtgcatctgtaacgtggacatcaccgtgagcgtgaaggagaactgcatctaccacaagagcatcttcaacggcgtgaacttccccgccgacggccccgtgatgaagaagatgaccaccaactgggaggccagctgcgagaagatcatgcccgtgcctaagcagggcatcctgaagggcgacgtgagcatgtacctgctgctgaaggacggcggccggtaccggtgccagttcgacaccgtgtacaaggccaagagcgtgcccagcaagatgcccgagtggcacttcatccagcacaagctgctgcgggaggaccggagcgacgccaagaaccagaagtggcagctgaccgagcacgccatcgccttccccagcgccctggcctgaggatctcgatagggatctgttaacgatccccggcggtgtcccccactgaagaaactatgtgctgtagtatagccgctgcccgctggctagctagctagttgagtcatttagcggcgatgattgagtaataatgtgtcacgcatcaccatgcatgggtggcagtgtcagtgtgagcaatgacctgaatgaacaattgaaatgaaaagaaaaaagtattgttccaaattaaacgttttaaccttttaataggtttatacaataattgatatatgttttctgtatatgtctaatttgttatcatccatttagatatagacaaaaaaaatctaagaactaaaacaaatgctaatttgaaatgaagggagtatatattgggataatgtcgatgagatccctcgtaatatcaccgacatcacacgtgtccagttaatgtatcagtgatacgtgtattcacatttgttgcgcgtaggcgtacccaacaattttgatcgactatcagaaagtcaacggaagcgagtcgacctcgagggggggccccggccgaagcttgcatgcctgcaggtcgactctagaggatctgcaccggacactgtctggtggcataccagacagtccggtgtgccagatcagggcacccttcggttcctttgctcctttgcttttgaaccctaactttgatcgtttattggtttgtgttgaacctttatgcacctgtggaatatataatctagaacaaactagttagtccaatcatttgtgttgggcattcaaccaccaaaattatttataggaaaaggttaaaccttatttccctttcaatctccccctttttggtgattgatgccaacacaaaccaaagaaaatatataagtgcagaattgaactagtttgcataaggtaagtgcataggttacttagaattaaatcaatttatacttttacttgatatgcatggttgctttcttttattttaacattttggaccacatttgcaccacttgttttgttttttgcaaatctttttggaaattctttttcaaagtcttttgcaaatagtcaaaggtatatgaataagattgtaagaagcattttcaagatttgaaatttctccccctgtttcaaatgcttttcctttgactaaacaaaactccccctgaataaaattctcctcttagctttcaagagggttttaaatagatatcaattggaaatatatttagatgctaattttgaaaatataccaattgaaaatcaacataccaatttgaaattaaacataccaatttaaaaaatttcaaaaagtggtggtgcggtccttttgctttgggcttaatatttctccccctttggcattaatcgccaaaaacggagactttgtgagccatttatactttctccccattggtaaatgaaatatgagtgaaagattataccaaatttggacagtgatgcggagtgacggcgaaggataaacgataccgttagagtggagtggaagccttgtcttcgccgaagactccatttccctttcaatctacgacttagcatagaaatacacttgaaaacacattagtcgtagccacgaaagagatatgatcaaaggtatacaaatgagctatgtgtgtaatgtttcaatcaaagtttcgagaatcaagaatatttagctcattcctaagtttgctaaaggttttatcatctaatggtttggtaaagatatcgactaattgttctttggtgctaacataagcaatctcgatatcacccctttgttggtgatccctcaaaaagtgataccgaatgtctatgtgcttagtgcggctgtgttcaacgggattatccgccatgcagatagcactctcattgtcacataggagagggactttgctcaatttgtagccatagtccctaaggttttgcctcatccaaagtaattgcacacaacaatgtcctgcggcaatatacttggcttcggcggtagaaagagctattgagttttgtttctttgaagtccaagacaccagggatctccctagaaactgacaagtccctgatgtgctcttcctatcaattttacaccctgcccaatcggcatctgaatatcctattaaatcaaaggtggatcccttggggtaccaaagaccaaatttaggagtgtaaactaaatatctcatgattcttttcacggccctaaggtgaacttccttaggatcggcttggaatcttgcacacatgcatatagaaagcatactatctggtcgagatgcacataaatagagtaaagatcctatcatcgaccggtataccttttggtctacggatttacctcccgtgtcgaggtcgagatgcccattagttcccatgggtgtcctgatgggcttggcatccttcattccaaacttgttgagtatgtcttgaatgtactttgtttggctgatgaaggtgccatcttggagttgcttgacttgaaatcctagaaaatatttcaacttccccatcatagacatctcgaatttcggaatcatgatcctactaaactcttcacaagtagatttgttagtagacccaaatataatatcatcaacataaatttggcatacaaacaaaacttttgaaatggttttagtaaagagagtaggatcggctttactgactctgaagccattagtgataagaaaatctcttaggcattcataccatgctgttggggcttgcttgagcccataaagcgcctttgagagtttataaacatggttagggtactcactatcttcaaagccgagaggttgctcaacatagacctattcaccccatttgatcacttttttggtccttcaggatctaatagttatgtataatttagagtctcttgtttaatggccagatatttctaattaatctaagaatttatgatattttttaattttttatcatgtctgatgagaattaacataaaggctcaattgggtcctgaattaataatagagtgaaaattaatccagaggctctattagaaccttcaattagtaataccaagatatatataagatagtagagtatagtttaaatgttggcattgttcattctttcttttgttatttaatttatgctttccacggtggttagtggttacttctgaagggtccaaataatgcatgaagagtttgaggacaagaagtctgccctaaaaatagcgatgcaaaggcatggtgtccaagccatacatatagcgcactaattttatcagcagaacaatggtatttataggtcctagtgcccaggcaacaagagacacgaataaagcatcgatcacgacaccagatctcatggcacaggttatcaacacgtttgacggggttgcggattatcttcagacatatcataagctacctgataattacattacaaaatcagaagcacaagccctcggctgggtggcatcaaaagggaaccttgcagacgtcgctccggggaaaagcatcggcggagacatcttctcaaacagggaaggcaaactcccgtaagtttctgcttctacctttgatatatatataataattatcattaattagtagtaatataatatttcaaatatttttttcaaaataaaagaatgtagtatatagcaattgcttttctgtagtttataagtgtgtatattttaatttataacttttctaatatatgaccaaaacatggtgatgtgcaggggcaaaagcggacgaacatggcgtgaagcggatattaactatacatcaggcttcagaaattcagaccggattctttactcaggcgactggctgatttacaaaacaacggaccattatcagacctttacaaaaatcagataactgcagctagacttgtccatcttctggattggccaacttaattaatgtatgaaataaaaggatgcacacatagtgacatgctaatcactataatgtgggcatcaaagttgtgtgttatgtgtaattactagttatctgaataaaagagaaagagatcatccatatttcttatcctaaatgaatgtcacgtgtctttataattctttgatgaaccagatgcatttcattaaccaaatccatatacatataaatattaatcatatataattaatatcaattgggttagcaaaacaaatctagggtcacccggtccgggcctagaaggccgatctcccgggcacccagctttcttgtacaaagtggccgttaacggatcccggtgaagttcctattccgaagttcctattctccagaaagtataggaacttcactagagcttgcggccgccccgggcaactttattatacatagttgataattcactggccgtcgttttacaacgtcgtgactgggaaaaccctggcgttacccaacttaatcgccttgcagcacatccccctttcgccagctggcgtaatagcgaagaggcccgcaccgatcgcccttcccaacagttgcgcagcctgaatggcgaatggcgcctgatgcggtattttctccttacgcatctgtgcggtatttcacaccgcatatggtgcactctcagtacaatctgctctgatgccgcatagttaagccagccccgacacccgccaacacccgctgacgcgccctgacgggcttgtctgctcccggcatccgcttacagacaagctgtgaccgtctccgggagctgcatgtgtcagaggttttcaccgtcatcaccgaaacgcgcgagacgaaagggcctcgtgatacgcctatttttataggttaatgtcatgataataatggtttcttagacgtcaggtggcacttttcggggaaatgtgcgcggaacccctatttgtttatttttctaaatacattcaaatatgtatccgctcatgagacaataaccctgataaatgcttcaataatattgaaaaaggaagagtatgagtattcaacatttccgtgtcgcccttattcccttttttgcggcattttgccttcctgtttttgctcacccagaaacgctggtgaaagtaaaagatgctgaagatcagttgggtgcacgagtgggttacatcgaactggatctcaacagcggtaagatccttgagagttttcgccccgaagaacgttttccaatgatgagcacttttaaagttctgctatgtggcgcggtattatcccgtattgacgccgggcaagagcaactcggtcgccgcatacactattctcagaatgacttggttgagtactcaccagtcacagaaaagcatcttacggatggcatgacagtaagagaattatgcagtgctgccataaccatgagtgataacactgcggccaacttacttctgacaacgatcggaggaccgaaggagctaaccgcttttttgcacaacatgggggatcatgtaactcgccttgatcgttgggaaccggagctgaatgaagccataccaaacgacgagcgtgacaccacgatgcctgtagcaatggcaacaacgttgcgcaaactattaactggcgaactacttactctagcttcccggcaacaattaatagactggatggaggcggataaagttgcaggaccacttctgcgctcggcccttccggctggctggtttattgctgataaatctggagccggtgagcgtgggtctcgcggtatcattgcagcactggggccagatggtaagccctcccgtatcgtagttatctacacgacggggagtcaggcaactatggatgaacgaaatagacagatcgctgagataggtgcctcactgattaagcattggtaactgtcagaccaagtttactcatatatactttagattgatttaaaacttcatttttaatttaaaaggatctaggtgaagatcctttttgataatctcatgaccaaaatcccttaacgtgagttttcgttccactg

SEQ ID NO: 49 - DNA, 2085 bp, synthetic construct
  misc_feature 1..2085: note = dpzm03g014880.1.1_Promoter glycosyltransferase
  source 1..2085: mol_type = other DNA
agatgacaggggtgttgtgttgaagggatggcgatcgacgactgttaatcgtgttttctgctttttggctagggtttgtgattcctctgagtttgaacatcatatgttgtgttgctgtcatctcgagtttgtgttcgtggtgatactatcaaactggaaattgtaccacgcggctgaaagcacctaccgctgacaggcagaagccatgcacgaatagattccaacatggaaaatgtaaaagtcgatgtttagagatgcacataatgtgagacttctaaactaattttatactccctccagtcttcagatactcgatattttgaacatgatcttatatagaaaacgtaatacattgatctgttcactattcactaatttatacatgtgttaagcattaaagtgctcgcagttcacacaatattatgctattgttaattttattttggtttccatttatttcttaaaaggatttttcttactactataacatgtaaaactattgtatctatcctgcaccatgggaggtgatttttgttatttacgttattttctactccctgtgttcctggtcactttggcttttctatagtataatattccaaacttgtgagtatttcgagtatttattggggtagtgtaaagtttatatgcatacttcctgtatatagaggttgatgctatttatctaatgatagtggtaaggcttagctaatagtatgatttgtgtacggtgagttgcatccgttcacaattctctttctcacatgcttctcttcctttgattttggatatgccattaagtacaagaacaaacaccatttactgctcaaatagaaaacatcatctaactatcaaatttctgcttcaataaaattcacctacaacgtatatgtgttcactcgactgattatccagaagtcatgatgtttcggcgattttgaatttttgtgagaattgtacaccagaatttttgacgccttacctggatggaatcgtgaataaattacttgttcttcttcaggcacgcaattacttgtgttgaattaggtttcaggttgcttcaaatatatttgttatcatgtttagtaaacaatgctaattgctcatgttcatattctagaatggcaagcaaatggtgcacggagagcattgacagctctagcgtcagtagcagattcatcacaggcgttgttcacttgggagttttatgcatagtgaatctctgttattgtgcatcatggcctcatggggttgtcgtattgttattgcgctttctaacttactcataataacaactttatatatcatttacattgttttttgtttgtctatctgatcataagtttgtagcaataacttttttgtttgtccatttacatggggcagcaggctgctgcgctcttgggagagcagcccgtctaccacgccgtacaacgttccattggctgcggggccaccatgcccctagtggcgctgcccgacaaggaggctgggtatttgggggattatcagcgaagcatcatgactcccgacgaagcaggggctgcgaccagcgcgctggacgttgctggggccgcctgatggtggcgacggctgctgtctgggggcagcagcagagctcatgatcgtcgagacctttgataccagattggtaggagccacgttccttataatgacgatatgtttccgttgcaacgcacgggcatccacctagtaacctatatgtgtggggttttctcctcctaggtttagctctccaaactagcctgaaaaaaagaaaaacacacccggagaaaaaaaaaagcacccaaatttgactcgcgaaatgcatgccgtttaatttgatccgagcccacagtctctcctcgggcccaccgcgtccgaccggcgcgcacgggcatccacctagtaacctatatgtgtggggttttctcctcctaggtttagctctccaaactagcctgaaaaaaagaaaaacacacccggagaaaaaaaaaagcacccaaatttgactcgcgaaatgcatgccgtttaatttgatccgagcccacagtctctcctcgggcccaccgcgtccgaccggcg

SEQ ID NO: 50 - DNA, 6270 bp, synthetic construct
  misc_feature 1..6270: note = PHP5096
  source 1..6270: mol_type = other DNA
tcgcgcgtttcggtgatgacggtgaaaacctctgacacatgcagctcccggagacggtcacagcttgtctgtaagcggatgccgggagcagacaagcccgtcagggcgcgtcagcgggtgttggcgggtgtcggggctggcttaactatgcggcatcagagcagattgtactgagagtgcaccatatgcggtgtgaaataccgcacagatgcgtaaggagaaaataccgcatcaggcgccattcgccattcaggctgcgcaactgttgggaagggcgatcggtgcgggcctcttcgctattacgccagctggcgaaagggggatgtgctgcaaggcgattaagttgggtaacgccagggttttcccagtcacgacgttgtaaaacgacggccagtgccaagcttgcatgcctgcagtgcagcgtgacccggtcgtgcccctctctagagataatgagcattgcatgtctaagttataaaaaattaccacatattttttttgtcacacttgtttgaagtgcagtttatctatctttatacatatatttaaactttactctacgaataatataatctatagtactacaataatatcagtgttttagagaatcatataaatgaacagttagacatggtctaaaggacaattgagtattttgacaacaggactctacagttttatctttttagtgtgcatgtgttctcctttttttttgcaaatagcttcacctatataatacttcatccattttattagtacatccatttagggtttagggttaatggtttttatagactaatttttttagtacatctattttattctattttagcctctaaattaagaaaactaaaactctattttagtttttttatttaataatttagatataaaatagaataaaataaagtgactaaaaattaaacaaataccctttaagaaattaaaaaaactaaggaaacatttttcttgtttcgagtagataatgccagcctgttaaacgccgtcgacgagtctaacggacaccaaccagcgaaccagcagcgtcgcgtcgggccaagcgaagcagacggcacggcatctctgtcgctgcctctggacccctctcgagagttccgctccaccgttggacttgctccgctgtcggcatccagaaattgcgtggcggagcggcagacgtgagccggcacggcaggcggcctcctcctcctctcacggcacggcagctacgggggattcctttcccaccgctccttcgctttcccttcctcgcccgccgtaataaatagacaccccctccacaccctctttccccaacctcgtgttgttcggagcgcacacacacacaaccagatctcccccaaatccacccgtcggcacctccgcttcaaggtacgccgctcgtcctccccccccccccctctctaccttctctagatcggcgttccggtccatggttagggcccggtagttctacttctgttcatgtttgtgttagatccgtgtttgtgttagatccgtgctgctagcgttcgtacacggatgcgacctgtacgtcagacacgttctgattgctaacttgccagtgtttctctttggggaatcctgggatggctctagccgttccgcagacgggatcgatttcatgattttttttgtttcgttgcatagggtttggtttgcccttttcctttatttcaatatatgccgtgcacttgtttgtcgggtcatcttttcatgcttttttttgtcttggttgtgatgatgtggtctggttgggcggtcgttctagatcggagtagaattctgtttcaaactacctggtggatttattaattttggatctgtatgtgtgtgccatacatattcatagttacgaattgaagatgatggatggaaatatcgatctaggataggtatacatgttgatgcgggttttactgatgcatatacagagatgctttttgttcgcttggttgtgatgatgtggtgtggttgggcggtcgttcattcgttctagatcggagtagaatactgtttcaaactacctggtgtatttattaattttggaactgtatgtgtgtgtcatacatcttcatagttacgagtttaagatggatggaaatatcgatctaggataggtatacatgttgatgtgggttttactgatgcatatacatgatggcatatgcagcatctattcatatgctctaaccttgagtacctatctattataataaacaagtatgttttataattattttgatcttgatatacttggatgatggcatatgcagcagctatatgtggatttttttagccctgccttcatacgctatttatttgcttggtactgtttcttttgtcgatgctcaccctgttgtttggtgttacttctgcaggtcgactctagaggatccaacaatgccccagttcgacatcctctgcaagaccccccccaaggtgctcgtgaggcagttcgtggagaggttcgagaggccctccggcgagaagatcgccctctgcgccgccgagctcacctacctctgctggatgatcacccacaacggcaccgccattaagagggccaccttcatgtcatacaacaccatcatctccaactccctctccttcgacatcgtgaacaagtccctccagttcaaatacaagacccagaaggccaccatcctcgaggcctccctcaagaagctcatccccgcctgggagttcaccatcatcccctactacggccagaagcaccagtccgacatcaccgacatcgtgtcatccctccagcttcagttcgagtcctccgaggaggctgacaagggcaactcccactccaagaagatgctgaaggccctcctctccgagggcgagtccatctgggagatcaccgagaagatcctcaactccttcgagtacacctccaggttcactaagaccaagaccctctaccagttcctcttcctcgccaccttcatcaactgcggcaggttctcagacatcaagaacgtggaccccaagtccttcaagctcgtgcagaacaagtacctcggcgtgatcatccagtgcctcgtgaccgagaccaagacctccgtgtccaggcacatctacttcttctccgctcgcggcaggatcgaccccctcgtgtacctcgacgagttcctcaggaactcagagcccgtgctcaagagggtgaacaggaccggcaactcctcctccaacaagcaggagtaccagctcctcaaggacaacctcgtgaggtcctacaacaaggccctcaagaagaacgccccctactccatcttcgccatcaagaacggccccaagtcccacatcggtaggcacctcatgacctccttcctctcaatgaagggcctcaccgagctcaccaacgtggtgggcaactggtccgacaagagggcctccgccgtggccaggaccacctacacccaccagatcaccgccatccccgaccactacttcgccctcgtgtcaaggtactacgcctacgaccccatctccaaggagatgatcgccctcaaggacgagactaaccccatcgaggagtggcagcacatcgagcagctcaagggctccgccgagggctccatcaggtaccccgcctggaacggcatcatctcccaggaggtgctcgactacctctcctcctacatcaacaggaggatctgagttaacctagacttgtccatcttctggattggccaacttaattaatgtatgaaataaaaggatgcacacatagtgacatgctaatcactataatgtgggcatcaaagttgtgtgttatgtgtaattactagttatctgaataaaagagaaagagatcatccatatttcttatcctaaatgaatgtcacgtgtctttataattctttgatgaaccagatgcatttcattaaccaaatccatatacatataaatattaatcatatataattaatatcaattgggttagcaaaacaaatctagtctaggtgtgttttgcgaattgcggccgcgatctggggaattcgtaatcatggtcatagctgtttcctgtgtgaaattgttatccgctcacaattccacacaacatacgagccggaagcataaagtgtaaagcctggggtgcctaatgagtgagctaactcacattaattgcgttgcgctcactgcccgctttccagtcgggaaacctgtcgtgccagctgcattaatgaatcggccaacgcgcggggagaggcggtttgcgtattgggcgctcttccgcttcctcgctcactgactcgctgcgctcggtcgttcggctgcggcgagcggtatcagctcactcaaaggcggtaatacggttatccacagaatcaggggataacgcaggaaagaacatgtgagcaaaaggccagcaaaaggccaggaaccgtaaaaaggccgcgttgctggcgtttttccataggctccgcccccctgacgagcatcacaaaaatcgacgctcaagtcagaggtggcgaaacccgacaggactataaagataccaggcgtttccccctggaagctccctcgtgcgctctcctgttccgaccctgccgcttaccggatacctgtccgcctttctcccttcgggaagcgtggcgctttctcatagctcacgctgtaggtatctcagttcggtgtaggtcgttcgctccaagctgggctgtgtgcacgaaccccccgttcagcccgaccgctgcgccttatccggtaactatcgtcttgagtccaacccggtaagacacgacttatcgccactggcagcagccactggtaacaggattagcagagcgaggtatgtaggcggtgctacagagttcttgaagtggtggcctaactacggctacactagaaggacagtatttggtatctgcgctctgctgaagccagttaccttcggaaaaagagttggtagctcttgatccggcaaacaaaccaccgctggtagcggtggtttttttgtttgcaagcagcagattacgcgcagaaaaaaaggatctcaagaagatcctttgatcttttctacggggtctgacgctcagtggaacgaaaactcacgttaagggattttggtcatgagattatcaaaaaggatcttcacctagatccttttaaattaaaaatgaagttttaaatcaatctaaagtatatatgagtaaacttggtctgacagttaccaatgcttaatcagtgaggcacctatctcagcgatctgtctatttcgttcatccatagttgcctgactccccgtcgtgtagataactacgatacgggagggcttaccatctggccccagtgctgcaatgataccgcgagacccacgctcaccggctccagatttatcagcaataaaccagccagccggaagggccgagcgcagaagtggtcctgcaactttatccgcctccatccagtctattaattgttgccgggaagctagagtaagtagttcgccagttaatagtttgcgcaacgttgttgccattgctacaggcatcgtggtgtcacgctcgtcgtttggtatggcttcattcagctccggttcccaacgatcaaggcgagttacatgatcccccatgttgtgcaaaaaagcggttagctccttcggtcctccgatcgttgtcagaagtaagttggccgcagtgttatcactcatggttatggcagcactgcataattctcttactgtcatgccatccgtaagatgcttttctgtgactggtgagtactcaaccaagtcattctgagaatagtgtatgcggcgaccgagttgctcttgcccggcgtcaatacgggataataccgcgccacatagcagaactttaaaagtgctcatcattggaaaacgttcttcggggcgaaaactctcaaggatcttaccgctgttgagatccagttcgatgtaacccactcgtgcacccaactgatcttcagcatcttttactttcaccagcgtttctgggtgagcaaaaacaggaaggcaaaatgccgcaaaaaagggaataagggcgacacggaaatgttgaatactcatactcttcctttttcaatattattgaagcatttatcagggttattgtctcatgagcggatacatatttgaatgtatttagaaaaataaacaaataggggttccgcgcacatttccccgaaaagtgccacctgacgtctaagaaaccattattatcatgacattaacctataaaaataggcgtatcacgaggccctttcgtc

SEQ ID NO: 51 - DNA, 8986 bp, synthetic construct
  misc_feature 1..8986: note = PHP01
  source 1..8986: mol_type = other DNA
gtttacccgccaatatatcctgtcaaacactgatagtttaaactgaaggcgggaaacgacaatctgatcatgagcggagaattaagggagtcacgttatgacccccgccgatgacgcgggacaagccgttttacgtttggaactgacagaaccgcaacgttgaaggagccactcagcaagctggtacgattgtaatacgactcactatagggcgaattgagcgctgtttaaacgctcttcaactggaagagcggttactaccggttaagtgactagggtcacgtgaccctagtcacttaggttatgatatcacatcaatccacttgctttgaagacgtggttggaacgtcttctttttccacgatgctcctcgtgggtgggggtccatctttgggaccactgtcggcagaggcatcttcaacgatggcctttcctttatcgcaatgatggcatttgtaggagccaccttccttttccactatcttcacaataaagtgacagatagctgggcaatggaatccgaggaggtttccggatattaccctttgttgaaaagtctcaattgccctttggtcttctgagactgtatctttgatatttttggagtagacaagcgtgtcgtgctccaccatgttgacgaagattttcttcttgtcattgagtcgtaagagactctgtatgaactgttcgccagtctttacggcgagttctgttaggtcctctatttgaatctttgactccatgatcgaaccagaaagcttgcatgcctgcaggtcgactctagaggatctgcaccggacactgtctggtggcataccagacagtccggtgtgccagatcagggcacccttcggttcctttgctcctttgcttttgaaccctaactttgatcgtttattggtttgtgttgaacctttatgcacctgtggaatatataatctagaacaaactagttagtccaatcatttgtgttgggcattcaaccaccaaaattatttataggaaaaggttaaaccttatttccctttcaatctccccctttttggtgattgatgccaacacaaaccaaagaaaatatataagtgcagaattgaactagtttgcataaggtaagtgcataggttacttagaattaaatcaatttatacttttacttgatatgcatggttgctttcttttattttaacattttggaccacatttgcaccacttgttttgttttttgcaaatctttttggaaattctttttcaaagtcttttgcaaatagtcaaaggtatatgaataagattgtaagaagcattttcaagatttgaaatttctccccctgtttcaaatgcttttcctttgactaaacaaaactccccctgaataaaattctcctcttagctttcaagagggttttaaatagatatcaattggaaatatatttagatgctaattttgaaaatataccaattgaaaatcaacataccaatttgaaattaaacataccaatttaaaaaatttcaaaaagtggtggtgcggtccttttgctttgggcttaatatttctccccctttggcattaatcgccaaaaacggagactttgtgagccatttatactttctccccattggtaaatgaaatatgagtgaaagattataccaaatttggacagtgatgcggagtgacggcgaaggataaacgataccgttagagtggagtggaagccttgtcttcgccgaagactccatttccctttcaatctacgacttagcatagaaatacacttgaaaacacattagtcgtagccacgaaagagatatgatcaaaggtatacaaatgagctatgtgtgtaatgtttcaatcaaagtttcgagaatcaagaatatttagctcattcctaagtttgctaaaggttttatcatctaatggtttggtaaagatatcgactaattgttctttggtgctaacataagcaatctcgatatcacccctttgttggtgatccctcaaaaagtgataccgaatgtctatgtgcttagtgcggctgtgttcaacgggattatccgccatgcagatagcactctcattgtcacataggagagggactttgctcaatttgtagccatagtccctaaggttttgcctcatccaaagtaattgcacacaacaatgtcctgcggcaatatacttggcttcggcggtagaaagagctattgagttttgtttctttgaagtccaagacaccagggatctccctagaaactgacaagtccctgatgtgctcttcctatcaattttacaccctgcccaatcggcatctgaatatcctattaaatcaaaggtggatcccttggggtaccaaagaccaaatttaggagtgtaaactaaatatctcatgattcttttcacggccctaaggtgaacttccttaggatcggcttggaatcttgcacacatgcatatagaaagcatactatctggtcgagatgcacataaatagagtaaagatcctatcatcgaccggtataccttttggtctacggatttacctcccgtgtcgaggtcgagatgcccattagttcccatgggtgtcctgatgggcttggcatccttcattccaaacttgttgagtatgtcttgaatgtactttgtttggctgatgaaggtgccatcttggagttgcttgacttgaaatcctagaaaatatttcaacttccccatcatagacatctcgaatttcggaatcatgatcctactaaactcttcacaagtagatttgttagtagacccaaatataatatcatcaacataaatttggcatacaaacaaaacttttgaaatggttttagtaaagagagtaggatcggctttactgactctgaagccattagtgataagaaaatctcttaggcattcataccatgctgttggggcttgcttgagcccataaagcgcctttgagagtttataaacatggttagggtactcactatcttcaaagccgagaggttgctcaacatagacctattcaccccatttgatcacttttttggtccttcaggatctaatagttatgtataatttagagtctcttgtttaatggccagatatttctaattaatctaagaatttatgatattttttaattttttatcatgtctgatgagaattaacataaaggctcaattgggtcctgaattaataatagagtgaaaattaatccagaggctctattagaaccttcaattagtaataccaagatatatataagatagtagagtatagtttaaatgttggcattgttcattctttcttttgttatttaatttatgctttccacggtggttagtggttacttctgaagggtccaaataatgcatgaagagtttgaggacaagaagtctgccctaaaaatagcgatgcaaaggcatggtgtccaagccatacatatagcgcactaattttatcagcagaacaatggtatttataggtcctagtgcccaggcaacaagagacacgaataaagcatcgatcacgacaccatggccagactcgacaagagcaaggtgatcaacagcgcactggagctgctgaacgaggtcggaatcgaaggcctcacaacccgtaaactcgcccagaagctcggggtagagcagcctacattgtattggcacgtcaagaacaagcgggctttgctagacgccctcgccattgagatgctcgataggcaccatacccacttctgccctttggaaggggaaagctggcaagacttcttgaggaacaacgctaagagcttcagatgtgctttgctcagtcaccgtgatggagccaaggtccacctaggtacacggcctacggagaagcagtatgaaactctcgagaaccagctcgccttcctgtgccaacaaggtttctcccttgagaatgccctctacgcactctccgctgtagggcacttcactctgggttgcgtattggaagatcaagagcaccaagtcgctaaggaggagagggaaacacctactactgatagtatgccgccactgctccgacaagctatcgagctcttcgatcaccaaggtgcagagccagccttcctgttcggccttgaattgatcatatgcggattggagaagcagctgaagtgtgaaagtgggtcttaacacatcgttctgaaggccgaaagtgggtcttaatgatagctgcagaaggtacctcagccgtcaacagccagggtgattagagccccagcatgcaaaatgatcacctggtcgctcatccttgactaaagcatggctcggcggtcgctgtttacctatatccctatagtaggtactcctgtacataaagcctgaaaaaatgggttcagttgtttatcgaactctgccaaatttgcttttgcatataatgtaaaattcagctagctctgctaagctcctcgcttcagttcgacagaactgcaattgatattgatgttatggaaattgatattggaacaatcagcaatattatgcttatattcatttcttgggcgtgctctactctgtgccgatgatatcatccgatgggttttgtacttcttacttatgaagtgaacgataataggttgcctggtcccagttctcagcttgatgttatgataatcatatgtgatttcagttctttgtctggcattggtctgtttttgtgtctgtgtctgtgggctgtggctctgtgtgttgataactcgagcttgattgcatcagtgaactgcgacttacaacagcagacagagtgttagcagcagggaaggagaatagagaaattagggagtaaagagaacatagttgcctttcagaggacagcttagcaagataacaaaattatgttctctccttttaaggattacagaggcatagcctcagcgacgcgcgtgctagcggatccagttatcatcatcgtgttgggcttcctgggcctggcctgcctagcaggcctgtcgacagcttcagaaggggaactcgttggcggattgtccacagtagcacgtactatatgcagaaaaagtccttatgtctctcttatcattagcctattaatcatattaattcagtccacataggaccgaatttataacttaacaatcttttagtttcctgagcaatatcgttaaatcaaaacatattcttgtaccaaattttgctatcaacggttcaacgctggtgcagcgtgacccggtcgtgcccctctctagagataatgagcattgcatgtctaagttataaaaaattaccacatattttttttgtcacacttgtttgaagtgcagtttatctatctttatacatatatttaaactttactctacgaataatataatctatagtactacaataatatcagtgttttagagaatcatataaatgaacagttagacatggtctaaaggacaattgagtattttgacaacaggactctacagttttatctttttagtgtgcatgtgttctcctttttttttgcaaatagcttcacctatataatacttcatccattttattagtacatccatttagggtttagggttaatggtttttatagactaatttttttagtacatctattttattctattttagcctctaaattaagaaaactaaaactctattttagtttttttatttaataatttagatataaaatagaataaaataaagtgactaaaaattaaacaaataccctttaagaaattaaaaaaactaaggaaacatttttcttgtttcgagtagataatgccagcctgttaaacgccgtcgacgagtctaacggacaccaaccagcgaaccagcagcgtcgcgtcgggccaagcgaagcagacggcacggcatctctgtcgctgcctctggacccctctcgagagttccgctccaccgttggacttgctccgctgtcggcatccagaaattgcgtggcggagcggcagacgtgagccggcacggcaggcggcctcctcctcctctcacggcaccggcagctacgggggattcctttcccaccgctccttcgctttcccttcctcgcccgccgtaataaatagacaccccctccacaccctctttccccaacctcgtgttgttcggagcgcacacacacacaaccagatctcccccaaatccacccgtcggcacctccgcttcaaggtacgccgctcgtcctcccccccccccctctctaccttctctagatcggcgttccggtccatgcatggttagggcccggtagttctacttctgttcatgtttgtgttagatccgtgtttgtgttagatccgtgctgctagcgttcgtacacggatgcgacctgtacgtcagacacgttctgattgctaacttgccagtgtttctctttggggaatcctgggatggctctagccgttccgcagacgggatcgatttcatgattttttttgtttcgttgcatagggtttggtttgcccttttcctttatttcaatatatgccgtgcacttgtttgtcgggtcatcttttcatgcttttttttgtcttggttgtgatgatgtggtctggttgggcggtcgttctagatcggagtagaattctgtttcaaactacctggtggatttattaattttggatctgtatgtgtgtgccatacatattcatagttacgaattgaagatgatggatggaaatatcgatctaggataggtatacatgttgatgcgggttttactgatgcatatacagagatgctttttgttcgcttggttgtgatgatgtggtgtggttgggcggtcgttcattcgttctagatcggagtagaatactgtttcaaactacctggtgtatttattaattttggaactgtatgtgtgtgtcatacatcttcatagttacgagtttaagatggatggaaatatcgatctaggataggtatacatgttgatgtgggttttactgatgcatatacatgatggcatatgcagcatctattcatatgctctaaccttgagtacctatctattataataaacaagtatgttttataattattttgatcttgatatacttggatgatggcatatgcagcagctatatgtggatttttttagccctgccttcatacgctatttatttgcttggtactgtttcttttgtcgatgctcaccctgttgtttggtgttacttctgcaggtcgactttaacttagcctaggatccatgcaaaaactcattaactcagtgcaaaactatgcctggggcagcaaaacggcgttgactgaactttatggtatggaaaatccgtccagccagccgatggccgagctgtggatgggcgcacatccgaaaagcagttcacgagtgcagaatgccgccggagatatcgtttcactgcgtgatgtgattgagagtgataaatcgactctgctcggagaggccgttgccaaacgctttggcgaactgcctttcctgttcaaagtattatgcgcagcacagccactctccattcaggttcatccaaacaaacacaattctgaaatcggttttgccaaagaaaatgccgcaggtatcccgatggatgccgccgagcgtaactataaagatcctaaccacaagccggagctggtttttgcgctgacgcctttccttgcgatgaacgcgtttcgtgaattttccgagattgtctccctactccagccggtcgcaggtgcacatccggcgattgctcactttttacaacagcctgatgccgaacgtttaagcgaactgttcgccagcctgttgaatatgcagggtgaagaaaaatcccgcgcgctggcgattttaaaatcggccctcgatagccagcagggtgaaccgtggcaaacgattcgtttaatttctgaattttacccggaagacagcggtctgttctccccgctattgctgaatgtggtgaaattgaaccctggcgaagcgatgttcctgttcgctgaaacaccgcacgcttacctgcaaggcgtggcgctggaagtgatggcaaactccgataacgtgctgcgtgcgggtctgacgcctaaatacattgatattccggaactggttgccaatgtgaaattcgaagccaaaccggctaaccagttgttgacccagccggtgaaacaaggtgcagaactggacttcccgattccagtggatgattttgccttctcgctgcatgaccttagtgataaagaaaccaccattagccagcagagtgccgccattttgttctgcgtcgaaggcgatgcaacgttgtggaaaggttctcagcagttacagcttaaaccgggtgaatcagcgtttattgccgccaacgaatcaccggtgactgtcaaaggccacggccgtttagcgcgcgtttacaacaagctgtaaatcactagcgaacgcgtaggtaccacatggttaacctagacttgtccatcttctggattggccaacttaattaatgtatgaaataaaaggatgcacacatagtgacatgctaatcactataatgtgggcatcaaagttgtgtgttatgtgtaattactagttatctgaataaaagagaaagagatcatccatatttcttatcctaaatgaatgtcacgtgtctttataattctttgatgaaccagatgcatttcattaaccaaatccatatacatataaatattaatcatatataattaatatcaattgggttagcaaaacaaatctagtctaggtgtgttttgcgaatgcggccgccaccgcggtggagctcgaattccggtccgaagctggccgataagtgactagggtcacgtgaccctagtcacttaggtaccgagctcgaattcattccgattaatcgtggcctcttgctcttcaggatgaagagctatgtttaaacgtgcaagcgctactagacaattcagtacattaaaaacgtccgcaatgtgttattaagttgtctaagcgtcaatttgtttacaccacaatatatcctgccac

SEQ ID NO: 52 - DNA, 9304 bp, synthetic construct
  misc_feature 1..9304: note = PHP02
  source 1..9304: mol_type = other DNA
agaagttcctattccgaagttcctattctctagaaagtataggaacttcagatccaccggctagaggatccaccatggttgaacaagatggattgcacgcaggttctccggccgcttgggtggagaggctattcggctatgactgggcacaacagacaatcggctgctctgatgccgccgtgttccggctgtcagcgcaggggcgcccggttctttttgtcaagaccgacctgtccggtgccctgaatgaactgcaggacgaggcagcgcggctatcgtggctggccacgacgggcgttccttgcgcagctgtgctcgacgttgtcactgaagcgggaagggactggctgctattgggcgaagtgccggggcaggatctcctgtcatctcaccttgctcctgccgagaaagtatccatcatggctgatgcaatgcggcggctgcatacgcttgatccggctacctgcccattcgaccaccaagcgaaacatcgcatcgagcgagcacgtactcggatggaagccggtcttgtcgatcaggatgatctggacgaagagcatcaggggctcgcgccagccgaactgttcgccaggctcaaggcgcgcatgcccgacggcgatgatctcgtcgtgacccatggcgatgcctgcttgccgaatatcatggtggaaaatggccgcttttctggattcatcgactgtggccggctgggtgtggcggaccgctatcaggacatagcgttggctacccgtgatattgctgaagagcttggcggcgaatgggctgaccgcttcctcgtgctttacggtatcgccgctcccgattcgcagcgcatcgccttctatcgccttcttgacgagttcttctgaggatccaccatggttaacctagacttgtccatcttctggattggccaacttaattaatgtatgaaataaaaggatgcacacatagtgacatgctaatcactataatgtgggcatcaaagttgtgtgttatgtgtaattactagttatctgaataaaagagaaagagatcatccatatttcttatcctaaatgaatgtcacgtgtctttataattctttgatgaaccagatgcatttcattaaccaaatccatatacatataaatattaatcatatataattaatatcaattgggttagcaaaacaaatctagtctaggtgtgttttgcgaatgcggccgggtaccgagctcgaattcggcccaagtttgtacaaaaaagcaggctccggccagaatggcccggaccgaagctggccgctctagaactaggcatggagtcaaagattcaaatagaggacctaacagaactcgccgtaaagactggcgaacagttcatacagagtctcttacgactcaatgacaagaagaaaatcttcgtcaacatggtggagcacgacacgcttgtctactccaaaaatatcaaagatacagtctcagaagaccaaagggcaattgagacttttcaacaaagggtaatatccggaaacctcctcggattccattgcccagctatctgtcactttattgtgaagatagtggaaaaggaaggtggctcctacaaatgccatcattgcgataaaggaaaggccatcgttgaagatgcctctgccgacagtggtcccaaagatggacccccacccacgaggagcatcgtggaaaaagaagacgttccaaccacgtcttcaaagcaagtggattgatgtgatatctccactgacgtaagggatgacgcacaatcccactaagctgacctagtggatctcgatgtgtagtctacgagaagggttaaccgtctcttcgtgagaataaccgtggcctaaaaataagccgatgaggataaataaaatgtggtggtacagtacttcaagaggtttactcatcaagaggatgcttttccgatgagctctagtagtacatcggacctcacatacctccattgtggtgaaatattttgtgctcatttagtgatgggtaaattttgtttatgtcactctaggttttgacatttcagttttgccactcttaggttttgacaaataatttccattccgcggcaaaagcaaaacaattttattttacttttaccactcttagctttcacaatgtatcacaaatgccactctagaaattctgtttatgccacagaatgtgaaaaaaaacactcacttatttgaagccaaggtgttcatggcatggaaatgtgacataaagtaacgttcgtgtataagaaaaaattgtactcctcgtaacaagagacggaaacatcatgagacaatcgcgtttggaaggctttgcatcacctttggatgatgcgcatgaatggagtcgtctgcttgctagccttcgcctaccgcccactgagtccgggcggcaactaccatcggcgaacgacccagctgacctctaccgaccggacttgaatgcgctaccttcgtcagcgacgatggccgcgtacgctggcgacgtgcccccgcatgcatggcggcacatggcgagctcagaccgtgcgtggctggctacaaatacgtaccccgtgagtgccctagctagaaacttacacctgcaactgcgagagcgagcgtgtgagtgtagccgatagatccgcccgcctcctccgagaacgtcatcaccgagttcatgcgcttcaaggtgcgcatggagggcaccgtgaacggccacgagttcgagatcgagggcgagggcgagggccgcccctacgagggccacaacaccgtgaagctgaaggtgaccaagggcggccccctgcccttcgcctgggacatcctgtccccccagttccagtacggctccaaggtgtacgtgaagcaccccgccgacatccccgactacaagaagctgtccttccccgagggcttcaagtgggagcgcgtgatgaacttcgaggacggcggcgtggcgaccgtgacccaggactcctccctgcaggacggctgcttcatctacaaggtgaagttcatcggcgtgaacttcccctccgacggccccgtgatgcagaagaagaccatgggctgggaggcctccaccgagcgcctgtacccccgcgacggcgtgctgaagggcgagacccacaaggccctgaagctgaaggacggcggccactacctggtggagttcaagtccatctacatggccaagaagcccgtgcagctgcccggctactactacgtggacgccaagctggacatcacctcccacaacgaggactacaccatcgtggagcagtacgagcgcaccgagggccgccaccacctgttcctgtagtgaagaaactatgtgctgtagtatagccgctgcccgctggctagctagctagttgagtcatttagcggcgatgattgagtaataatgtgtcacgcatcaccatgcatgggtggcagtgtcagtgtgagcaatgacctgaatgaacaattgaaatgaaaagaaaaaagtattgttccaaattaaacgttttaaccttttaataggtttatacaataattgatatatgttttctgtatatgtctaatttgttatcatccatttagatatagacaaaaaaaatctaagaactaaaacaaatgctaatttgaaatgaagggagtatatattgggataatgtcgatgagatccctcgtaatatcaccgacatcacacgtgtccagttaatgtatcagtgatacgtgtattcacatttgttgcgcgtaggcgtacccaacaattttgatcgactatcagaaagtcaacggaagcgagtcgacctcgaggcatggagtcaaagattcaaatagaggacctaacagaactcgccgtaaagactggcgaacagttcatacagagtctcttacgactcaatgacaagaagaaaatcttcgtcaacatggtggagcacgacacgcttgtctactccaaaaatatcaaagatacagtctcagaagaccaaagggcaattgagacttttcaacaaagggtaatatccggaaacctcctcggattccattgcccagctatctgtcactttattgtgaagatagtggaaaaggaaggtggctcctacaaatgccatcattgcgataaaggaaaggccatcgttgaagatgcctctgccgacagtggtcccaaagatggacccccacccacgaggagcatcgtggaaaaagaagacgttccaaccacgtcttcaaagcaagtggattgatgtgatatctccactgacgtaagggatgacgcacaatcccactaagctgaccttcggagaagcttgcatgcctgcaggtcgactctagaggatctgcaccggacactgtctggtggcataccagacagtccggtgtgccagatcagggcacccttcggttcctttgctcctttgcttttgaaccctaactttgatcgtttattggtttgtgttgaacctttatgcacctgtggaatatataatctagaacaaactagttagtccaatcatttgtgttgggcattcaaccaccaaaattatttataggaaaaggttaaaccttatttccctttcaatctccccctttttggtgattgatgccaacacaaaccaaagaaaatatataagtgcagaattgaactagtttgcataaggtaagtgcataggttacttagaattaaatcaatttatacttttacttgatatgcatggttgctttcttttattttaacattttggaccacatttgcaccacttgttttgttttttgcaaatctttttggaaattctttttcaaagtcttttgcaaatagtcaaaggtatatgaataagattgtaagaagcattttcaagatttgaaatttctccccctgtttcaaatgcttttcctttgactaaacaaaactccccctgaataaaattctcctcttagctttcaagagggttttaaatagatatcaattggaaatatatttagatgctaattttgaaaatataccaattgaaaatcaacataccaatttgaaattaaacataccaatttaaaaaatttcaaaaagtggtggtgcggtccttttgctttgggcttaatatttctccccctttggcattaatcgccaaaaacggagactttgtgagccatttatactttctccccattggtaaatgaaatatgagtgaaagattataccaaatttggacagtgatgcggagtgacggcgaaggataaacgataccgttagagtggagtggaagccttgtcttcgccgaagactccatttccctttcaatctacgacttagcatagaaatacacttgaaaacacattagtcgtagccacgaaagagatatgatcaaaggtatacaaatgagctatgtgtgtaatgtttcaatcaaagtttcgagaatcaagaatatttagctcattcctaagtttgctaaaggttttatcatctaatggtttggtaaagatatcgactaattgttctttggtgctaacataagcaatctcgatatcacccctttgttggtgatccctcaaaaagtgataccgaatgtctatgtgcttagtgcggctgtgttcaacgggattatccgccatgcagatagcactctcattgtcacataggagagggactttgctcaatttgtagccatagtccctaaggttttgcctcatccaaagtaattgcacacaacaatgtcctgcggcaatatacttggcttcggcggtagaaagagctattgagttttgtttctttgaagtccaagacaccagggatctccctagaaactgacaagtccctgatgtgctcttcctatcaattttacaccctgcccaatcggcatctgaatatcctattaaatcaaaggtggatcccttggggtaccaaagaccaaatttaggagtgtaaactaaatatctcatgattcttttcacggccctaaggtgaacttccttaggatcggcttggaatcttgcacacatgcatatagaaagcatactatctggtcgagatgcacataaatagagtaaagatcctatcatcgaccggtataccttttggtctacggatttacctcccgtgtcgaggtcgagatgcccattagttcccatgggtgtcctgatgggcttggcatccttcattccaaacttgttgagtatgtcttgaatgtactttgtttggctgatgaaggtgccatcttggagttgcttgacttgaaatcctagaaaatatttcaacttccccatcatagacatctcgaatttcggaatcatgatcctactaaactcttcacaagtagatttgttagtagacccaaatataatatcatcaacataaatttggcatacaaacaaaacttttgaaatggttttagtaaagagagtaggatcggctttactgactctgaagccattagtgataagaaaatctcttaggcattcataccatgctgttggggcttgcttgagcccataaagcgcctttgagagtttataaacatggttagggtactcactatcttcaaagccgagaggttgctcaacatagacctattcaccccatttgatcacttttttggtccttcaggatctaatagttatgtataatttagagtctcttgtttaatggccagatatttctaattaatctaagaatttatgatattttttaattttttatcatgtctgatgagaattaacataaaggctcaattgggtcctgaattaataatagagtgaaaattaatccagaggctctattagaaccttcaattagtaataccaagatatatataagatagtagagtatagtttaaatgttggcattgttcattctttcttttgttatttaatttatgctttccacggtggttagtggttacttctgaagggtccaaataatgcatgaagagtttgaggacaagaagtctgccctaaaaatagcgatgcaaaggcatggtgtccaagccatacatatagcgcactaattttatcagcagaacaatggtatttataggtcctagtgcccaggcaacaagagacacgaataaagcatcgatcacgacaccgagactctatcagtgatagagtgtatataagactctatcagtgatagagtgaactctatcagtgatagagttatggcggcgacaatggcagtgacgacgatggtgacgaggagcaaggagagctggtcgtcattgcaggtcccggcggtggcattcccttggaagccacgaggtggcaagaccggcggcctcgagttccctcgccgggcgatgttcgccagcgtcggcctcaacgtgtgcccgggcgtcccggcggggcgcgacccgcgggagcccgatcccaaggtcgtccgggcggcctgcggcctggtccaggcacaagtcctcttccaggggtttaactgggagtcgtgcaagcagcagggaggctggtacaacaggctcaaggcccaggtcgacgacatcgccaaggccggcgtcacgcacgtctggctgcctccaccctcgcactccgtctcgccacaaggctacatgccaggccgcctatacgacctggacgcgtccaagtacggcacggcggcggagctcaagtccctgatagcggcgttccacggcaggggcgtgcagtgcgtggcggacatcgtcatcaaccaccggtgcgcggaaaagaaggacgcgcgcggcgtgtactgcatcttcgagggcgggactcccgacgaccgcctggactggggccccgggatgatctgcagcgacgacacgcagtactcggacgggacggggcaccgcgacacgggcgaggggttcgcggcggcgcccgacatcgaccacctcaacccgcgcgtgcagcgggagctctccgcctggctcaactggctcaggtccgacgccgtggggttcgacggctggcgcctcgacttcgccaagggctactcgccggccgtcgccagaatgtacgtggagagcacggggccgccgagcttcgtcgtcgcggagatatggaactcgctgagctacagcggggacggcaagccggcgcccaaccaggaccagtgccggcaggagctgctggactggacgcgggccgtcggcgggcccgccatggcgttcgacttccccaccaagggcctgctgcaggcgggcgtgcagggggagctgtggcggctgcgcgacagctccggcaacgcggccggcctgatcgggtgggcgcccgagaaggccgtcaccttcgtcgacaaccatgacaccgggtcgacgcagaagctctggccgttcccatccgacaaggtcatgcagggctacgcctacatcctcacccatccaggagtcccctgcattttctacgaccacatgttcgactggaacctgaagcaggagatatccacgctgtctgccatcagggcgcggaacggcatccgcgccgggagcaagctgcggatcctcgtggcggacgcggacgcgtacgtggccgtcgtcgacgagaaggtcatggtgaagatcgggacaaggtacggcgtgagcagcgtggtcccgtcggatttccacccggcggcgcacggcaaggactactgcgtctgggagaaagcgagcctccgcgtcccggcggggcgccacctctagcagctcagattgctcagtcttgtgctgcattgcaaacacagcagcacgacactgcataacgtcttttccttgagatctgacaaagcagcattagtccgttgatcggtggaagaccactcgtcagtgttgagttgaatgtttgatcaataaaatacggcaatgctgtaagggttgttttttatgccattgataatacactgtactgttcagttgttgaactctatttcttagccatgccaagtgcttttcttattttgaataacattacagcaaaaagttgaaagacaaaaaaaaaaacccccgaacagagtgctttgggtcccaagctactttagactgtgttcggcgttccccctaaatttctccccctatatctcactcacttgtcacatcagcgttctctttcccctatatctccacgtcgacgcggccgctctagaactagtggatcccccgggctgcaggaattcctcgagaccgtacgtgcgcgcgaatgcatccagatcttccctctagtcaaggccttaagcgcgcgttcgaacgcgcggttaagcttggtcacccggtccgggcctagaaggccgatctcccgggcacccagctttcttgtacaaagtggccgttaacggatcccggtgaagttcctattccgaagttcctattctccagaaagtataggaacttcgat

SEQ ID NO: 53 - DNA, 9325 bp, synthetic construct
  misc_feature 1..9325: note = PHP03
  source 1..9325: mol_type = other DNA
agaagttcctattccgaagttcctattctctagaaagtataggaacttcagatccaccggctagaggatccaccatggttgaacaagatggattgcacgcaggttctccggccgcttgggtggagaggctattcggctatgactgggcacaacagacaatcggctgctctgatgccgccgtgttccggctgtcagcgcaggggcgcccggttctttttgtcaagaccgacctgtccggtgccctgaatgaactgcaggacgaggcagcgcggctatcgtggctggccacgacgggcgttccttgcgcagctgtgctcgacgttgtcactgaagcgggaagggactggctgctattgggcgaagtgccggggcaggatctcctgtcatctcaccttgctcctgccgagaaagtatccatcatggctgatgcaatgcggcggctgcatacgcttgatccggctacctgcccattcgaccaccaagcgaaacatcgcatcgagcgagcacgtactcggatggaagccggtcttgtcgatcaggatgatctggacgaagagcatcaggggctcgcgccagccgaactgttcgccaggctcaaggcgcgcatgcccgacggcgatgatctcgtcgtgacccatggcgatgcctgcttgccgaatatcatggtggaaaatggccgcttttctggattcatcgactgtggccggctgggtgtggcggaccgctatcaggacatagcgttggctacccgtgatattgctgaagagcttggcggcgaatgggctgaccgcttcctcgtgctttacggtatcgccgctcccgattcgcagcgcatcgccttctatcgccttcttgacgagttcttctgaggatccaccatggttaacctagacttgtccatcttctggattggccaacttaattaatgtatgaaataaaaggatgcacacatagtgacatgctaatcactataatgtgggcatcaaagttgtgtgttatgtgtaattactagttatctgaataaaagagaaagagatcatccatatttcttatcctaaatgaatgtcacgtgtctttataattctttgatgaaccagatgcatttcattaaccaaatccatatacatataaatattaatcatatataattaatatcaattgggttagcaaaacaaatctagtctaggtgtgttttgcgaatgcggccgggtaccgagctcgaattcggcccaagtttgtacaaaaaagcaggctccggccagaatggcccggaccgaagctggccgctctagaactaggcatggagtcaaagattcaaatagaggacctaacagaactcgccgtaaagactggcgaacagttcatacagagtctcttacgactcaatgacaagaagaaaatcttcgtcaacatggtggagcacgacacgcttgtctactccaaaaatatcaaagatacagtctcagaagaccaaagggcaattgagacttttcaacaaagggtaatatccggaaacctcctcggattccattgcccagctatctgtcactttattgtgaagatagtggaaaaggaaggtggctcctacaaatgccatcattgcgataaaggaaaggccatcgttgaagatgcctctgccgacagtggtcccaaagatggacccccacccacgaggagcatcgtggaaaaagaagacgttccaaccacgtcttcaaagcaagtggattgatgtgatatctccactgacgtaagggatgacgcacaatcccactaagctgacctagtggatctcgatgtgtagtctacgagaagggttaaccgtctcttcgtgagaataaccgtggcctaaaaataagccgatgaggataaataaaatgtggtggtacagtacttcaagaggtttactcatcaagaggatgcttttccgatgagctctagtagtacatcggacctcacatacctccattgtggtgaaatattttgtgctcatttagtgatgggtaaattttgtttatgtcactctaggttttgacatttcagttttgccactcttaggttttgacaaataatttccattccgcggcaaaagcaaaacaattttattttacttttaccactcttagctttcacaatgtatcacaaatgccactctagaaattctgtttatgccacagaatgtgaaaaaaaacactcacttatttgaagccaaggtgttcatggcatggaaatgtgacataaagtaacgttcgtgtataagaaaaaattgtactcctcgtaacaagagacggaaacatcatgagacaatcgcgtttggaaggctttgcatcacctttggatgatgcgcatgaatggagtcgtctgcttgctagccttcgcctaccgcccactgagtccgggcggcaactaccatcggcgaacgacccagctgacctctaccgaccggacttgaatgcgctaccttcgtcagcgacgatggccgcgtacgctggcgacgtgcccccgcatgcatggcggcacatggcgagctcagaccgtgcgtggctggctacaaatacgtaccccgtgagtgccctagctagaaacttacacctgcaactgcgagagcgagcgtgtgagtgtagccgatagatccgcccatggcccacagcaagcacggcctgaaggaggagatgaccatgaagtaccacatggagggctgcgtgaacggccacaagttcgtgatcaccggcgagggcatcggctaccccttcaagggcaagcagaccatcaacctgtgcgtgatcgagggcggccccctgcccttcagcgaggacatcctgagcgccggcttcaagtacggcgaccggatcttcaccgagtacccccaggacatcgtggactacttcaagaacagctgccccgccggctacacctggggccggagcttcctgttcgaggacggcgccgtgtgcatctgtaacgtggacatcaccgtgagcgtgaaggagaactgcatctaccacaagagcatcttcaacggcgtgaacttccccgccgacggccccgtgatgaagaagatgaccaccaactgggaggccagctgcgagaagatcatgcccgtgcctaagcagggcatcctgaagggcgacgtgagcatgtacctgctgctgaaggacggcggccggtaccggtgccagttcgacaccgtgtacaaggccaagagcgtgcccagcaagatgcccgagtggcacttcatccagcacaagctgctgcgggaggaccggagcgacgccaagaaccagaagtggcagctgaccgagcacgccatcgccttccccagcgccctggcctgatgaagaaactatgtgctgtagtatagccgctgcccgctggctagctagctagttgagtcatttagcggcgatgattgagtaataatgtgtcacgcatcaccatgcatgggtggcagtgtcagtgtgagcaatgacctgaatgaacaattgaaatgaaaagaaaaaagtattgttccaaattaaacgttttaaccttttaataggtttatacaataattgatatatgttttctgtatatgtctaatttgttatcatccatttagatatagacaaaaaaaatctaagaactaaaacaaatgctaatttgaaatgaagggagtatatattgggataatgtcgatgagatccctcgtaatatcaccgacatcacacgtgtccagttaatgtatcagtgatacgtgtattcacatttgttgcgcgtaggcgtacccaacaattttgatcgactatcagaaagtcaacggaagcgagtcgacctcgaggcatggagtcaaagattcaaatagaggacctaacagaactcgccgtaaagactggcgaacagttcatacagagtctcttacgactcaatgacaagaagaaaatcttcgtcaacatggtggagcacgacacgcttgtctactccaaaaatatcaaagatacagtctcagaagaccaaagggcaattgagacttttcaacaaagggtaatatccggaaacctcctcggattccattgcccagctatctgtcactttattgtgaagatagtggaaaaggaaggtggctcctacaaatgccatcattgcgataaaggaaaggccatcgttgaagatgcctctgccgacagtggtcccaaagatggacccccacccacgaggagcatcgtggaaaaagaagacgttccaaccacgtcttcaaagcaagtggattgatgtgatatctccactgacgtaagggatgacgcacaatcccactaagctgaccttcggagaagcttgcatgcctgcaggtcgactctagaggatctgcaccggacactgtctggtggcataccagacagtccggtgtgccagatcagggcacccttcggttcctttgctcctttgcttttgaaccctaactttgatcgtttattggtttgtgttgaacctttatgcacctgtggaatatataatctagaacaaactagttagtccaatcatttgtgttgggcattcaaccaccaaaattatttataggaaaaggttaaaccttatttccctttcaatctccccctttttggtgattgatgccaacacaaaccaaagaaaatatataagtgcagaattgaactagtttgcataaggtaagtgcataggttacttagaattaaatcaatttatacttttacttgatatgcatggttgctttcttttattttaacattttggaccacatttgcaccacttgttttgttttttgcaaatctttttggaaattctttttcaaagtcttttgcaaatagtcaaaggtatatgaataagattgtaagaagcattttcaagatttgaaatttctccccctgtttcaaatgcttttcctttgactaaacaaaactccccctgaataaaattctcctcttagctttcaagagggttttaaatagatatcaattggaaatatatttagatgctaattttgaaaatataccaattgaaaatcaacataccaatttgaaattaaacataccaatttaaaaaatttcaaaaagtggtggtgcggtccttttgctttgggcttaatatttctccccctttggcattaatcgccaaaaacggagactttgtgagccatttatactttctccccattggtaaatgaaatatgagtgaaagattataccaaatttggacagtgatgcggagtgacggcgaaggataaacgataccgttagagtggagtggaagccttgtcttcgccgaagactccatttccctttcaatctacgacttagcatagaaatacacttgaaaacacattagtcgtagccacgaaagagatatgatcaaaggtatacaaatgagctatgtgtgtaatgtttcaatcaaagtttcgagaatcaagaatatttagctcattcctaagtttgctaaaggttttatcatctaatggtttggtaaagatatcgactaattgttctttggtgctaacataagcaatctcgatatcacccctttgttggtgatccctcaaaaagtgataccgaatgtctatgtgcttagtgcggctgtgttcaacgggattatccgccatgcagatagcactctcattgtcacataggagagggactttgctcaatttgtagccatagtccctaaggttttgcctcatccaaagtaattgcacacaacaatgtcctgcggcaatatacttggcttcggcggtagaaagagctattgagttttgtttctttgaagtccaagacaccagggatctccctagaaactgacaagtccctgatgtgctcttcctatcaattttacaccctgcccaatcggcatctgaatatcctattaaatcaaaggtggatcccttggggtaccaaagaccaaatttaggagtgtaaactaaatatctcatgattcttttcacggccctaaggtgaacttccttaggatcggcttggaatcttgcacacatgcatatagaaagcatactatctggtcgagatgcacataaatagagtaaagatcctatcatcgaccggtataccttttggtctacggatttacctcccgtgtcgaggtcgagatgcccattagttcccatgggtgtcctgatgggcttggcatccttcattccaaacttgttgagtatgtcttgaatgtactttgtttggctgatgaaggtgccatcttggagttgcttgacttgaaatcctagaaaatatttcaacttccccatcatagacatctcgaatttcggaatcatgatcctactaaactcttcacaagtagatttgttagtagacccaaatataatatcatcaacataaatttggcatacaaacaaaacttttgaaatggttttagtaaagagagtaggatcggctttactgactctgaagccattagtgataagaaaatctcttaggcattcataccatgctgttggggcttgcttgagcccataaagcgcctttgagagtttataaacatggttagggtactcactatcttcaaagccgagaggttgctcaacatagacctattcaccccatttgatcacttttttggtccttcaggatctaatagttatgtataatttagagtctcttgtttaatggccagatatttctaattaatctaagaatttatgatattttttaattttttatcatgtctgatgagaattaacataaaggctcaattgggtcctgaattaataatagagtgaaaattaatccagaggctctattagaaccttcaattagtaataccaagatatatataagatagtagagtatagtttaaatgttggcattgttcattctttcttttgttatttaatttatgctttccacggtggttagtggttacttctgaagggtccaaataatgcatgaagagtttgaggacaagaagtctgccctaaaaatagcgatgcaaaggcatggtgtccaagccatacatatagcgcactaattttatcagcagaacaatggtatttataggtcctagtgcccaggcaacaagagacacgaataaagcatcgatcacgacaccgagactctatcagtgatagagtgtatataagactctatcagtgatagagtgaactctatcagtgatagagttatggcggcgacaatggcagtgacgacgatggtgacgaggagcaaggagagctggtcgtcattgcaggtcccggcggtggcattcccttggaagccacgaggtggcaagaccggcggcctcgagttccctcgccgggcgatgttcgccagcgtcggcctcaacgtgtgcccgggcgtcccggcggggcgcgacccgcgggagcccgatcccaaggtcgtccgggcggcctgcggcctggtccaggcacaagtcctcttccaggggtttaactgggagtcgtgcaagcagcagggaggctggtacaacaggctcaaggcccaggtcgacgacatcgccaaggccggcgtcacgcacgtctggctgcctccaccctcgcactccgtctcgccacaaggctacatgccaggccgcctatacgacctggacgcgtccaagtacggcacggcggcggagctcaagtccctgatagcggcgttccacggcaggggcgtgcagtgcgtggcggacatcgtcatcaaccaccggtgcgcggaaaagaaggacgcgcgcggcgtgtactgcatcttcgagggcgggactcccgacgaccgcctggactggggccccgggatgatctgcagcgacgacacgcagtactcggacgggacggggcaccgcgacacgggcgaggggttcgcggcggcgcccgacatcgaccacctcaacccgcgcgtgcagcgggagctctccgcctggctcaactggctcaggtccgacgccgtggggttcgacggctggcgcctcgacttcgccaagggctactcgccggccgtcgccagaatgtacgtggagagcacggggccgccgagcttcgtcgtcgcggagatatggaactcgctgagctacagcggggacggcaagccggcgcccaaccaggaccagtgccggcaggagctgctggactggacgcgggccgtcggcgggcccgccatggcgttcgacttccccaccaagggcctgctgcaggcgggcgtgcagggggagctgtggcggctgcgcgacagctccggcaacgcggccggcctgatcgggtgggcgcccgagaaggccgtcaccttcgtcgacaaccatgacaccgggtcgacgcagaagctctggccgttcccatccgacaaggtcatgcagggctacgcctacatcctcacccatccaggagtcccctgcattttctacgaccacatgttcgactggaacctgaagcaggagatatccacgctgtctgccatcagggcgcggaacggcatccgcgccgggagcaagctgcggatcctcgtggcggacgcggacgcgtacgtggccgtcgtcgacgagaaggtcatggtgaagatcgggacaaggtacggcgtgagcagcgtggtcccgtcggatttccacccggcggcgcacggcaaggactactgcgtctgggagaaagcgagcctccgcgtcccggcggggcgccacctctagcagctcagattgctcagtcttgtgctgcattgcaaacacagcagcacgacactgcataacgtcttttccttgagatctgacaaagcagcattagtccgttgatcggtggaagaccactcgtcagtgttgagttgaatgtttgatcaataaaatacggcaatgctgtaagggttgttttttatgccattgataatacactgtactgttcagttgttgaactctatttcttagccatgccaagtgcttttcttattttgaataacattacagcaaaaagttgaaagacaaaaaaaaaaacccccgaacagagtgctttgggtcccaagctactttagactgtgttcggcgttccccctaaatttctccccctatatctcactcacttgtcacatcagcgttctctttcccctatatctccacgtcgacgcggccgctctagaactagtggatcccccgggctgcaggaattcctcgagaccgtacgtgcgcgcgaatgcatccagatcttccctctagtcaaggccttaagcgcgcgttcgaacgcgcggttaagcttggtcacccggtccgggcctagaaggccgatctcccgggcacccagctttcttgtacaaagtggccgttaacggatcccggtgaagttcctattccgaagttcctattctccagaaagtataggaacttcgat

SEQ ID NO: 54 - DNA, 6755 bp, synthetic construct
  misc_feature 1..6755: note = PHP04
  source 1..6755: mol_type = other DNA
gaagttcctattccgaagttcctattctctagaaagtataggaacttcagatccaccggctagaggatccaccatggttgaacaagatggattgcacgcaggttctccggccgcttgggtggagaggctattcggctatgactgggcacaacagacaatcggctgctctgatgccgccgtgttccggctgtcagcgcaggggcgcccggttctttttgtcaagaccgacctgtccggtgccctgaatgaactgcaggacgaggcagcgcggctatcgtggctggccacgacgggcgttccttgcgcagctgtgctcgacgttgtcactgaagcgggaagggactggctgctattgggcgaagtgccggggcaggatctcctgtcatctcaccttgctcctgccgagaaagtatccatcatggctgatgcaatgcggcggctgcatacgcttgatccggctacctgcccattcgaccaccaagcgaaacatcgcatcgagcgagcacgtactcggatggaagccggtcttgtcgatcaggatgatctggacgaagagcatcaggggctcgcgccagccgaactgttcgccaggctcaaggcgcgcatgcccgacggcgatgatctcgtcgtgacccatggcgatgcctgcttgccgaatatcatggtggaaaatggccgcttttctggattcatcgactgtggccggctgggtgtggcggaccgctatcaggacatagcgttggctacccgtgatattgctgaagagcttggcggcgaatgggctgaccgcttcctcgtgctttacggtatcgccgctcccgattcgcagcgcatcgccttctatcgccttcttgacgagttcttctgaggatccaccatggttaacctagacttgtccatcttctggattggccaacttaattaatgtatgaaataaaaggatgcacacatagtgacatgctaatcactataatgtgggcatcaaagttgtgtgttatgtgtaattactagttatctgaataaaagagaaagagatcatccatatttcttatcctaaatgaatgtcacgtgtctttataattctttgatgaaccagatgcatttcattaaccaaatccatatacatataaatattaatcatatataattaatatcaattgggttagcaaaacaaatctagtctaggtgtgttttgcgaatgcggccgggtaccgagctcgaattcggcccaagtttgtacaaaaaagcaggctccggccagaatggcccggaccgaagctggccgctctagaactagtggatctcgatgtgtagtctacgagaagggttaaccgtctcttcgtgagaataaccgtggcctaaaaataagccgatgaggataaataaaatgtggtggtacagtacttcaagaggtttactcatcaagaggatgcttttccgatgagctctagtagtacatcggacctcacatacctccattgtggtgaaatattttgtgctcatttagtgatgggtaaattttgtttatgtcactctaggttttgacatttcagttttgccactcttaggttttgacaaataatttccattccgcggcaaaagcaaaacaattttattttacttttaccactcttagctttcacaatgtatcacaaatgccactctagaaattctgtttatgccacagaatgtgaaaaaaaacactcacttatttgaagccaaggtgttcatggcatggaaatgtgacataaagtaacgttcgtgtataagaaaaaattgtactcctcgtaacaagagacggaaacatcatgagacaatcgcgtttggaaggctttgcatcacctttggatgatgcgcatgaatggagtcgtctgcttgctagccttcgcctaccgcccactgagtccgggcggcaactaccatcggcgaacgacccagctgacctctaccgaccggacttgaatgcgctaccttcgtcagcgacgatggccgcgtacgctggcgacgtgcccccgcatgcatggcggcacatggcgagctcagaccgtgcgtggctggctacaaatacgtaccccgtgagtgccctagctagaaacttacacctgcaactgcgagagcgagcgtgtgagtgtagccgatagatccgcccggatcgcctcctccgagaacgtcatcaccgagttcatgcgcttcaaggtgcgcatggagggcaccgtgaacggccacgagttcgagatcgagggcgagggcgagggccgcccctacgagggccacaacaccgtgaagctgaaggtgaccaagggcggccccctgcccttcgcctgggacatcctgtccccccagttccagtacggctccaaggtgtacgtgaagcaccccgccgacatccccgactacaagaagctgtccttccccgagggcttcaagtgggagcgcgtgatgaacttcgaggacggcggcgtggcgaccgtgacccaggactcctccctgcaggacggctgcttcatctacaaggtgaagttcatcggcgtgaacttcccctccgacggccccgtgatgcagaagaagaccatgggctgggaggcctccaccgagcgcctgtacccccgcgacggcgtgctgaagggcgagacccacaaggccctgaagctgaaggacggcggccactacctggtggagttcaagtccatctacatggccaagaagcccgtgcagctgcccggctactactacgtggacgccaagctggacatcacctcccacaacgaggactacaccatcgtggagcagtacgagcgcaccgagggccgccaccacctgttcctgtagccccactgaagaaactatgtgctgtagtatagccgctgcccgctggctagctagctagttgagtcatttagcggcgatgattgagtaataatgtgtcacgcatcaccatgcatgggtggcagtgtcagtgtgagcaatgacctgaatgaacaattgaaatgaaaagaaaaaagtattgttccaaattaaacgttttaaccttttaataggtttatacaataattgatatatgttttctgtatatgtctaatttgttatcatccatttagatatagacaaaaaaaatctaagaactaaaacaaatgctaatttgaaatgaagggagtatatattgggataatgtcgatgagatccctcgtaatatcaccgacatcacacgtgtccagttaatgtatcagtgatacgtgtattcacatttgttgcgcgtaggcgtacccaacaattttgatcgactatcagaaagtcaacggaagcgagtcgacctcgagggggggccccggccgaagcttgcatgcctgcaggtcgactctagaggatctgcaccggacactgtctggtggcataccagacagtccggtgtgccagatcagggcacccttcggttcctttgctcctttgcttttgaaccctaactttgatcgtttattggtttgtgttgaacctttatgcacctgtggaatatataatctagaacaaactagttagtccaatcatttgtgttgggcattcaaccaccaaaattatttataggaaaaggttaaaccttatttccctttcaatctccccctttttggtgattgatgccaacacaaaccaaagaaaatatataagtgcagaattgaactagtttgcataaggtaagtgcataggttacttagaattaaatcaatttatacttttacttgatatgcatggttgctttcttttattttaacattttggaccacatttgcaccacttgttttgttttttgcaaatctttttggaaattctttttcaaagtcttttgcaaatagtcaaaggtatatgaataagattgtaagaagcattttcaagatttgaaatttctccccctgtttcaaatgcttttcctttgactaaacaaaactccccctgaataaaattctcctcttagctttcaagagggttttaaatagatatcaattggaaatatatttagatgctaattttgaaaatataccaattgaaaatcaacataccaatttgaaattaaacataccaatttaaaaaatttcaaaaagtggtggtgcggtccttttgctttgggcttaatatttctccccctttggcattaatcgccaaaaacggagactttgtgagccatttatactttctccccattggtaaatgaaatatgagtgaaagattataccaaatttggacagtgatgcggagtgacggcgaaggataaacgataccgttagagtggagtggaagccttgtcttcgccgaagactccatttccctttcaatctacgacttagcatagaaatacacttgaaaacacattagtcgtagccacgaaagagatatgatcaaaggtatacaaatgagctatgtgtgtaatgtttcaatcaaagtttcgagaatcaagaatatttagctcattcctaagtttgctaaaggttttatcatctaatggtttggtaaagatatcgactaattgttctttggtgctaacataagcaatctcgatatcacccctttgttggtgatccctcaaaaagtgataccgaatgtctatgtgcttagtgcggctgtgttcaacgggattatccgccatgcagatagcactctcattgtcacataggagagggactttgctcaatttgtagccatagtccctaaggttttgcctcatccaaagtaattgcacacaacaatgtcctgcggcaatatacttggcttcggcggtagaaagagctattgagttttgtttctttgaagtccaagacaccagggatctccctagaaactgacaagtccctgatgtgctcttcctatcaattttacaccctgcccaatcggcatctgaatatcctattaaatcaaaggtggatcccttggggtaccaaagaccaaatttaggagtgtaaactaaatatctcatgattcttttcacggccctaaggtgaacttccttaggatcggcttggaatcttgcacacatgcatatagaaagcatactatctggtcgagatgcacataaatagagtaaagatcctatcatcgaccggtataccttttggtctacggatttacctcccgtgtcgaggtcgagatgcccattagttcccatgggtgtcctgatgggcttggcatccttcattccaaacttgttgagtatgtcttgaatgtactttgtttggctgatgaaggtgccatcttggagttgcttgacttgaaatcctagaaaatatttcaacttccccatcatagacatctcgaatttcggaatcatgatcctactaaactcttcacaagtagatttgttagtagacccaaatataatatcatcaacataaatttggcatacaaacaaaacttttgaaatggttttagtaaagagagtaggatcggctttactgactctgaagccattagtgataagaaaatctcttaggcattcataccatgctgttggggcttgcttgagcccataaagcgcctttgagagtttataaacatggttagggtactcactatcttcaaagccgagaggttgctcaacatagacctattcaccccatttgatcacttttttggtccttcaggatctaatagttatgtataatttagagtctcttgtttaatggccagatatttctaattaatctaagaatttatgatattttttaattttttatcatgtctgatgagaattaacataaaggctcaattgggtcctgaattaataatagagtgaaaattaatccagaggctctattagaaccttcaattagtaataccaagatatatataagatagtagagtatagtttaaatgttggcattgttcattctttcttttgttatttaatttatgctttccacggtggttagtggttacttctgaagggtccaaataatgcatgaagagtttgaggacaagaagtctgccctaaaaatagcgatgcaaaggcatggtgtccaagccatacatatagcgcactaattttatcagcagaacaatggtatttataggtcctagtgcccaggcaacaagagacacgaataaagcatcgatcacgacaccagaatgatcaagatcgccacccgcaagtacctcggcaagcagaacgtgtacgacatcggcgtggagagggaccacaacttcgcgctgaagaacgggttcatcgccagcaactgcgaccaaccaagaaccatcgacatgaaagccagaggaggcaaaagactcgagagagtcccagaaacaatcatgaacgaagtcctcggaagactcagcaccatactcacatagtgctagacttgtccatcttctggattggccaacttaattaatgtatgaaataaaaggatgcacacatagtgacatgctaatcactataatgtgggcatcaaagttgtgtgttatgtgtaattactagttatctgaataaaagagaaagagatcatccatatttcttatcctaaatgaatgtcacgtgtctttataattctttgatgaaccagatgcatttcattaaccaaatccatatacatataaatattaatcatatataattaatatcaattgggttagcaaaacaaatctagggtcacccggtccgggcctagaaggccgatctcccgggcacccagctttcttgtacaaagtggccgttaacggatcccggtgaagttcctattccgaagttcctattctccagaaagtataggaacttc

SEQ ID NO: 55 - DNA, 7250 bp, synthetic construct
  misc_feature 1..7250: note = PHP05
  source 1..7250: mol_type = other DNA
gaagttcctattccgaagttcctattctctagaaagtataggaacttcagatccaccggctagaggatccaccatggttgaacaagatggattgcacgcaggttctccggccgcttgggtggagaggctattcggctatgactgggcacaacagacaatcggctgctctgatgccgccgtgttccggctgtcagcgcaggggcgcccggttctttttgtcaagaccgacctgtccggtgccctgaatgaactgcaggacgaggcagcgcggctatcgtggctggccacgacgggcgttccttgcgcagctgtgctcgacgttgtcactgaagcgggaagggactggctgctattgggcgaagtgccggggcaggatctcctgtcatctcaccttgctcctgccgagaaagtatccatcatggctgatgcaatgcggcggctgcatacgcttgatccggctacctgcccattcgaccaccaagcgaaacatcgcatcgagcgagcacgtactcggatggaagccggtcttgtcgatcaggatgatctggacgaagagcatcaggggctcgcgccagccgaactgttcgccaggctcaaggcgcgcatgcccgacggcgatgatctcgtcgtgacccatggcgatgcctgcttgccgaatatcatggtggaaaatggccgcttttctggattcatcgactgtggccggctgggtgtggcggaccgctatcaggacatagcgttggctacccgtgatattgctgaagagcttggcggcgaatgggctgaccgcttcctcgtgctttacggtatcgccgctcccgattcgcagcgcatcgccttctatcgccttcttgacgagttcttctgaggatccaccatggttaacctagacttgtccatcttctggattggccaacttaattaatgtatgaaataaaaggatgcacacatagtgacatgctaatcactataatgtgggcatcaaagttgtgtgttatgtgtaattactagttatctgaataaaagagaaagagatcatccatatttcttatcctaaatgaatgtcacgtgtctttataattctttgatgaaccagatgcatttcattaaccaaatccatatacatataaatattaatcatatataattaatatcaattgggttagcaaaacaaatctagtctaggtgtgttttgcgaatgcggccgggtaccgagctcgaattcggcccaagtttgtacaaaaaagcaggctccggccagaatggcccggaccgaagctggccgctctagaactagtggatctcgatgtgtagtctacgagaagggttaaccgtctcttcgtgagaataaccgtggcctaaaaataagccgatgaggataaataaaatgtggtggtacagtacttcaagaggtttactcatcaagaggatgcttttccgatgagctctagtagtacatcggacctcacatacctccattgtggtgaaatattttgtgctcatttagtgatgggtaaattttgtttatgtcactctaggttttgacatttcagttttgccactcttaggttttgacaaataatttccattccgcggcaaaagcaaaacaattttattttacttttaccactcttagctttcacaatgtatcacaaatgccactctagaaattctgtttatgccacagaatgtgaaaaaaaacactcacttatttgaagccaaggtgttcatggcatggaaatgtgacataaagtaacgttcgtgtataagaaaaaattgtactcctcgtaacaagagacggaaacatcatgagacaatcgcgtttggaaggctttgcatcacctttggatgatgcgcatgaatggagtcgtctgcttgctagccttcgcctaccgcccactgagtccgggcggcaactaccatcggcgaacgacccagctgacctctaccgaccggacttgaatgcgctaccttcgtcagcgacgatggccgcgtacgctggcgacgtgcccccgcatgcatggcggcacatggcgagctcagaccgtgcgtggctggctacaaatacgtaccccgtgagtgccctagctagaaacttacacctgcaactgcgagagcgagcgtgtgagtgtagccgatagatccgcccatggcccacagcaagcacggcctgaaggaggagatgaccatgaagtaccacatggagggctgcgtgaacggccacaagttcgtgatcaccggcgagggcatcggctaccccttcaagggcaagcagaccatcaacctgtgcgtgatcgagggcggccccctgcccttcagcgaggacatcctgagcgccggcttcaagtacggcgaccggatcttcaccgagtacccccaggacatcgtggactacttcaagaacagctgccccgccggctacacctggggccggagcttcctgttcgaggacggcgccgtgtgcatctgtaacgtggacatcaccgtgagcgtgaaggagaactgcatctaccacaagagcatcttcaacggcgtgaacttccccgccgacggccccgtgatgaagaagatgaccaccaactgggaggccagctgcgagaagatcatgcccgtgcctaagcagggcatcctgaagggcgacgtgagcatgtacctgctgctgaaggacggcggccggtaccggtgccagttcgacaccgtgtacaaggccaagagcgtgcccagcaagatgcccgagtggcacttcatccagcacaagctgctgcgggaggaccggagcgacgccaagaaccagaagtggcagctgaccgagcacgccatcgccttccccagcgccctggcctgaggatctcgatagggatctgttaacgatccccggcggtgtcccccactgaagaaactatgtgctgtagtatagccgctgcccgctggctagctagctagttgagtcatttagcggcgatgattgagtaataatgtgtcacgcatcaccatgcatgggtggcagtgtcagtgtgagcaatgacctgaatgaacaattgaaatgaaaagaaaaaagtattgttccaaattaaacgttttaaccttttaataggtttatacaataattgatatatgttttctgtatatgtctaatttgttatcatccatttagatatagacaaaaaaaatctaagaactaaaacaaatgctaatttgaaatgaagggagtatatattgggataatgtcgatgagatccctcgtaatatcaccgacatcacacgtgtccagttaatgtatcagtgatacgtgtattcacatttgttgcgcgtaggcgtacccaacaattttgatcgactatcagaaagtcaacggaagcgagtcgacctcgagggggggccccggccgaagcttgcatgcctgcaggtcgactctagaggatctgcaccggacactgtctggtggcataccagacagtccggtgtgccagatcagggcacccttcggttcctttgctcctttgcttttgaaccctaactttgatcgtttattggtttgtgttgaacctttatgcacctgtggaatatataatctagaacaaactagttagtccaatcatttgtgttgggcattcaaccaccaaaattatttataggaaaaggttaaaccttatttccctttcaatctccccctttttggtgattgatgccaacacaaaccaaagaaaatatataagtgcagaattgaactagtttgcataaggtaagtgcataggttacttagaattaaatcaatttatacttttacttgatatgcatggttgctttcttttattttaacattttggaccacatttgcaccacttgttttgttttttgcaaatctttttggaaattctttttcaaagtcttttgcaaatagtcaaaggtatatgaataagattgtaagaagcattttcaagatttgaaatttctccccctgtttcaaatgcttttcctttgactaaacaaaactccccctgaataaaattctcctcttagctttcaagagggttttaaatagatatcaattggaaatatatttagatgctaattttgaaaatataccaattgaaaatcaacataccaatttgaaattaaacataccaatttaaaaaatttcaaaaagtggtggtgcggtccttttgctttgggcttaatatttctccccctttggcattaatcgccaaaaacggagactttgtgagccatttatactttctccccattggtaaatgaaatatgagtgaaagattataccaaatttggacagtgatgcggagtgacggcgaaggataaacgataccgttagagtggagtggaagccttgtcttcgccgaagactccatttccctttcaatctacgacttagcatagaaatacacttgaaaacacattagtcgtagccacgaaagagatatgatcaaaggtatacaaatgagctatgtgtgtaatgtttcaatcaaagtttcgagaatcaagaatatttagctcattcctaagtttgctaaaggttttatcatctaatggtttggtaaagatatcgactaattgttctttggtgctaacataagcaatctcgatatcacccctttgttggtgatccctcaaaaagtgataccgaatgtctatgtgcttagtgcggctgtgttcaacgggattatccgccatgcagatagcactctcattgtcacataggagagggactttgctcaatttgtagccatagtccctaaggttttgcctcatccaaagtaattgcacacaacaatgtcctgcggcaatatacttggcttcggcggtagaaagagctattgagttttgtttctttgaagtccaagacaccagggatctccctagaaactgacaagtccctgatgtgctcttcctatcaattttacaccctgcccaatcggcatctgaatatcctattaaatcaaaggtggatcccttggggtaccaaagaccaaatttaggagtgtaaactaaatatctcatgattcttttcacggccctaaggtgaacttccttaggatcggcttggaatcttgcacacatgcatatagaaagcatactatctggtcgagatgcacataaatagagtaaagatcctatcatcgaccggtataccttttggtctacggatttacctcccgtgtcgaggtcgagatgcccattagttcccatgggtgtcctgatgggcttggcatccttcattccaaacttgttgagtatgtcttgaatgtactttgtttggctgatgaaggtgccatcttggagttgcttgacttgaaatcctagaaaatatttcaacttccccatcatagacatctcgaatttcggaatcatgatcctactaaactcttcacaagtagatttgttagtagacccaaatataatatcatcaacataaatttggcatacaaacaaaacttttgaaatggttttagtaaagagagtaggatcggctttactgactctgaagccattagtgataagaaaatctcttaggcattcataccatgctgttggggcttgcttgagcccataaagcgcctttgagagtttataaacatggttagggtactcactatcttcaaagccgagaggttgctcaacatagacctattcaccccatttgatcacttttttggtccttcaggatctaatagttatgtataatttagagtctcttgtttaatggccagatatttctaattaatctaagaatttatgatattttttaattttttatcatgtctgatgagaattaacataaaggctcaattgggtcctgaattaataatagagtgaaaattaatccagaggctctattagaaccttcaattagtaataccaagatatatataagatagtagagtatagtttaaatgttggcattgttcattctttcttttgttatttaatttatgctttccacggtggttagtggttacttctgaagggtccaaataatgcatgaagagtttgaggacaagaagtctgccctaaaaatagcgatgcaaaggcatggtgtccaagccatacatatagcgcactaattttatcagcagaacaatggtatttataggtcctagtgcccaggcaacaagagacacgaataaagcatcgatcacgacaccagaatgctcaagtaccagctcaagaacgagaacggctggatgcacaggagactcgtcaggaggaaaagcgacatggagagaggcgaaatctggctcgtcagcctcgatcctacagctggtcacgaacaacagggcaccagacccgtcctcatcgtcacaccagccgccttcaaccgcgtcaccagactcccagtcgtcgtcccagtcacaagcggcggcaacttcgccagaacagccggcttcgccgtcagcctcgacggagtcggaatcaggacaacaggcgtcgtcaggtgcctttctttcggaactgagatccttaccgttgagtacggaccacttcctattggtaagatcgtttctgaggaaattaactgctcagtgtactctgttgatccagaaggaagagtttacactcaggctatcgcacaatggcacgataggggtgaacaagaggttctcgagtacgagcttgaagatggatccgttattcgtgctacctctgaccatagattcttgactacagattatcagcttctcgctatcgaggaaatctttgctaggcaacttgatctccttactttggagaacatcaagcagacagaagaggctcttgacaaccacagacttccattccctttgctcgatgctggaaccatcaagtgaatgctagacttgtccatcttctggattggccaacttaattaatgtatgaaataaaaggatgcacacatagtgacatgctaatcactataatgtgggcatcaaagttgtgtgttatgtgtaattactagttatctgaataaaagagaaagagatcatccatatttcttatcctaaatgaatgtcacgtgtctttataattctttgatgaaccagatgcatttcattaaccaaatccatatacatataaatattaatcatatataattaatatcaattgggttagcaaaacaaatctagggtcacccggtccgggcctagaaggccgatctcccgggcacccagctttcttgtacaaagtggccgttaacggatcccggtgaagttcctattccgaagttcctattctccagaaagtataggaacttc

SEQ ID NO: 56 - DNA, 25 bp, synthetic construct
  misc_feature 1..25: note = RB
  source 1..25: mol_type = other DNA
gtttacccgccaatatatcctgtca

SEQ ID NO: 57 - DNA, 26 bp, synthetic construct
  misc_feature 1..26: note = LB
  source 1..26: mol_type = other DNA
gtttacaccacaatatatcctgccac

SEQ ID NO: 58 - DNA, 34 bp, synthetic construct
  misc_feature 1..34: note = LOXP
  source 1..34: mol_type = other DNA
ataacttcgtatagcatacattatacgaagttat

SEQ ID NO: 59 - DNA, 1176 bp, Escherichia coli; identical to SEQ ID NO: 24
  source 1..1176: mol_type = unassigned DNA

SEQ ID NO: 60 - protein, 391 aa, Escherichia coli; identical to SEQ ID NO: 17

SEQ ID NO: 61 - DNA, 34 bp, synthetic construct
  misc_feature 1..34: note = ALL STOPS
  source 1..34: mol_type = other DNA
taagtgactagggtcacgtgaccctagtcactta

SEQ ID NO: 62 - DNA, 980 bp, Sorghum bicolor
  source 1..980: mol_type = unassigned DNA
gccgtcaacagccagggtgattagagccccagcatgcaaaatgatcacctggtcgctcatccttgactaaagcatggctcggcggtcgctgtttacctatatccctatagtaggtactcctgtacataaagcctgaaaaaatgggttcagttgtttatcgaactctgccaaatttgcttttgcatataatgtaaaattcagctagctctgctaagctcctcgcttcagttcgacagaactgcaattgatattgatgttatggaaattgatattggaacaatcagcaatattatgcttatattcatttcttgggcgtgctctactctgtgccgatgatatcatccgatgggttttgtacttcttacttatgaagtgaacgataataggttgcctggtcccagttctcagcttgatgttatgataatcatatgtgatttcagttctttgtctggcattggtctgtttttgtgtctgtgtctgtgggctgtggctctgtgtgttgataactcgagcttgattgcatcagtgaactgcgacttacaacagcagacagagtgttagcagcagggaaggagaatagagaaattagggagtaaagagaacatagttgcctttcagaggacagcttagcaagataacaaaattatgttctctccttttaaggattacagaggcatagcctcagcgacgcgcgtgctagcggatccagttatcatcatcgtgttgggcttcctgggcctggcctgcctagcaggcctgtcgacagcttcagaaggggaactcgttggcggattgtccacagtagcacgtactatatgcagaaaaagtccttatgtctctcttatcattagcctattaatcatattaattcagtccacataggaccgaatttataacttaacaatcttttagtttcctgagcaatatcgttaaatcaaaacatattcttgtaccaaattttgctatcaacggttcaacgc

SEQ ID NO: 63 - DNA, 108 bp, Nostoc punctiforme
  source 1..108: mol_type = unassigned DNA
atgatcaagatcgccacccgcaagtacctcggcaagcagaacgtgtacgacatcggcgtggagagggaccacaacttcgcgctgaagaacgggttcatcgccagcaac

SEQ ID NO: 64 - protein, 36 aa, Nostoc punctiforme
MIKIATRKYLGKQNVYDIGVERDHNFALKNGFIASN

SEQ ID NO: 65 - DNA, 373 bp, Nostoc punctiforme
  source 1..373: mol_type = unassigned DNA
tgcctttctttcggaactgagatccttaccgttgagtacggaccacttcctattggtaagatcgtttctgaggaaattaactgctcagtgtactctgttgatccagaaggaagagtttacactcaggctatcgcacaatggcacgataggggtgaacaagaggttctcgagtacgagcttgaagatggatccgttattcgtgctacctctgaccatagattcttgactacagattatcagcttctcgctatcgaggaaatctttgctaggcaacttgatctccttactttggagaacatcaagcagacagaagaggctcttgacaaccacagacttccattccctttgctcgatgctggaaccatcaagtgaa

SEQ ID NO: 66 - protein, 123 aa, Nostoc punctiforme
CLSFGTEILTVEYGPLPIGKIVSEEINCSVYSVDPEGRVYTQAIAQWHDRGEQEVLEYELEDGSVIRATSDHRFLTTDYQLLAIEEIFARQLDLLTLENIKQTEEALDNHRLPFPLLDAGTIK

SEQ ID NO: 67 - DNA, 288 bp, Escherichia coli
  source 1..288: mol_type = unassigned DNA
atgctcaagtaccagctcaagaacgagaacggctggatgcacaggagactcgtcaggaggaaaagcgacatggagagaggcgaaatctggctcgtcagcctcgatcctacagctggtcacgaacaacagggcaccagacccgtcctcatcgtcacaccagccgccttcaaccgcgtcaccagactcccagtcgtcgtcccagtcacaagcggcggcaacttcgccagaacagccggcttcgccgtcagcctcgacggagtcggaatcaggacaacaggcgtcgtcagg

SEQ ID NO: 68 - protein, 96 aa, Escherichia coli
MLKYQLKNENGWMHRRLVRRKSDMERGEIWLVSLDPTAGHEQQGTRPVLIVTPAAFNRVTRLPVVVPVTSGGNFARTAGFAVSLDGVGIRTTGVVR

SEQ ID NO: 69 - DNA, 114 bp, Escherichia coli
  source 1..114: mol_type = unassigned DNA
tgcgaccaaccaagaaccatcgacatgaaagccagaggaggcaaaagactcgagagagtcccagaaacaatcatgaacgaagtcctcggaagactcagcaccatactcacatag

SEQ ID NO: 70 - protein, 37 aa, Escherichia coli
CDQPRTIDMKARGGKRLERVPETIMNEVLGRLSTILT

SEQ ID NO: 71 - DNA, 690 bp, Anemonia majano
  source 1..690: mol_type = unassigned DNA
atggccctgtccaacaagttcatcggcgacgacatgaagatgacgtaccacatggacgggtgcgtcaacggccactacttcaccgtcaagggcgaagggtccggtaagccatacgagggcacgcagacctccacattcaaggtcacgatggctaacggtggtccgctggccttctcattcgatatcctgagcaccgtcttcatgtacgggaacaggtgcttcacggcgtacccgacctcaatgccagactacttcaagcaggccttcccggacggcatgtcgtacgagaggaccttcacctacgaggacggtggcgtggcgactgcttcgtgggagatctccctcaagggcaactgcttcgaacacaagtcgacgttccacggcgtgaatttcccagcggacgggccagtcatggcaaagaagacgactggctgggacccgagcttcgagaagatgacggtctgcgacggcatcctcaagggcgacgttacggcttttctcatgctgcagggcggagggaattataggtgccagttccacaccagctacaagacgaagaagccggtcacgatgccgccgaaccacgtcgtcgagcacaggatagcgaggaccgaccttgacaagggcggcaactcggtgcagctcactgagcacgccgtcgcacacatcacgtcagtcgtgccgttctag

SEQ ID NO: 72 - protein, 229 aa, Anemonia majano
MALSNKFIGDDMKMTYHMDGCVNGHYFTVKGEGSGKPYEGTQTSTFKVTMANGGPLAFSFDILSTVFMYGNRCFTAYPTSMPDYFKQAFPDGMSYERTFTYEDGGVATASWEISLKGNCFEHKSTFHGVNFPADGPVMAKKTTGWDPSFEKMTVCDGILKGDVTAFLMLQGGGNYRCQFHTSYKTKKPVTMPPNHVVEHRIARTDLDKGGNSVQLTEHAVAHITSVVPF

SEQ ID NO: 73 - DNA, 2102 bp, synthetic construct
  misc_feature 1..2102: note = LTP2 PRO-AMCYAN-GZW64A TERM
  source 1..2102: mol_type = other DNA
ctctagaactagtggatctcgatgtgtagtctacgagaagggttaaccgtctcttcgtgagaataaccgtggcctaaaaataagccgatgaggataaataaaatgtggtggtacagtacttcaagaggtttactcatcaagaggatgcttttccgatgagctctagtagtacatcggacctcacatacctccattgtggtgaaatattttgtgctcatttagtgatgggtaaattttgtttatgtcactctaggttttgacatttcagttttgccactcttaggttttgacaaataatttccattccgcggcaaaagcaaaacaattttattttacttttaccactcttagctttcacaatgtatcacaaatgccactctagaaattctgtttatgccacagaatgtgaaaaaaaacactcacttatttgaagccaaggtgttcatggcatggaaatgtgacataaagtaacgttcgtgtataagaaaaaattgtactcctcgtaacaagagacggaaacatcatgagacaatcgcgtttggaaggctttgcatcacctttggatgatgcgcatgaatggagtcgtctgcttgctagccttcgcctaccgcccactgagtccgggcggcaactaccatcggcgaacgacccagctgacctctaccgaccggacttgaatgcgctaccttcgtcagcgacgatggccgcgtacgctggcgacgtgcccccgcatgcatggcggcacatggcgagctcagaccgtgcgtggctggctacaaatacgtaccccgtgagtgccctagctagaaacttacacctgcaactgcgagagcgagcgtgtgagtgtagccgagtagatcccccgggctgaaggtcgactctagaggatccaccggtcgccaccatggccctgtccaacaagttcatcggcgacgacatgaagatgacgtaccacatggacgggtgcgtcaacggccactacttcaccgtcaagggcgaagggtccggtaagccatacgagggcacgcagacctccacattcaaggtcacgatggctaacggtggtccgctggccttctcattcgatatcctgagcaccgtcttcatgtacgggaacaggtgcttcacggcgtacccgacctcaatgccagactacttcaagcaggccttcccggacggcatgtcgtacgagaggaccttcacctacgaggacggtggcgtggcgactgcttcgtgggagatctccctcaagggcaactgcttcgaacacaagtcgacgttccacggcgtgaatttcccagcggacgggccagtcatggcaaagaagacgactggctgggacccgagcttcgagaagatgacggtctgcgacggcatcctcaagggcgacgttacggcttttctcatgctgcagggcggagggaattataggtgccagttccacaccagctacaagacgaagaagccggtcacgatgccgccgaaccacgtcgtcgagcacaggatagcgaggaccgaccttgacaagggcggcaactcggtgcagctcactgagcacgccgtcgcacacatcacgtcagtcgtgccgttctagttcgaaggtaccgttaacgaagaaactatgtgctgtagtatagccgctgcccgctggctaggtagctagttgagtcatttagcggcgatgattgagtaataatgtgtcacgcatcaccatgcatgggtggcagtgtcagtgtgagcaatgacctgaatgaacaattgaaatgaaaagaaaaaagtattgttccaaattaaacgttttaaccttttaataggtttatacaataattgatatatgttttctgtatatgtctaatttgttatcatccatttagatatagacaaaaaaaatctaagaactaaaacaaatgctaatttgaaatgaagggagtatatattgggataatgtcgatgagatccctcgtaatatcaccgacatcacacgtgtccagttaatgtatcagtgatacgtgtattcacatttgttgcgcgtaggcgtacccaacaattttgatcgactatcagaaagtcaacggaagcgagtcgacctcgagggggggccc

SEQ ID NO: 74 - DNA, 3042 bp, synthetic construct
  misc_feature 1..3042: note = UBI1ZM PRO-UBI1ZM INTRON-AMCYAN-PINII TERM
  source 1..3042: mol_type = other DNA
ctgcagtgcagcgtgacccggtcgtgcccctctctagagataatgagcattgcatgtctaagttataaaaaattaccacatattttttttgtcacacttgtttgaagtgcagtttatctatctttatacatatatttaaactttactctacgaataatataatctatagtactacaataatatcagtgttttagagaatcatataaatgaacagttagacatggtctaaaggacaattgagtattttgacaacaggactctacagttttatctttttagtgtgcatgtgttctcctttttttttgcaaatagcttcacctatataatacttcatccattttattagtacatccatttagggtttagggttaatggtttttatagactaatttttttagtacatctattttattctattttagcctctaaattaagaaaactaaaactctattttagtttttttatttaataatttagatataaaatagaataaaataaagtgactaaaaattaaacaaataccctttaagaaattaaaaaaactaaggaaacatttttcttgtttcgagtagataatgccagcctgttaaacgccgtcgacgagtctaacggacaccaaccagcgaaccagcagcgtcgcgtcgggccaagcgaagcagacggcacggcatctctgtcgctgcctctggacccctctcgagagttccgctccaccgttggacttgctccgctgtcggcatccagaaattgcgtggcggagcggcagacgtgagccggcacggcaggcggcctcctcctcctctcacggcacggcagctacgggggattcctttcccaccgctccttcgctttcccttcctcgcccgccgtaataaatagacaccccctccacaccctctttccccaacctcgtgttgttcggagcgcacacacacacaaccagatctcccccaaatccacccgtcggcacctccgcttcaaggtacgccgctcgtcctccccccccccccctctctaccttctctagatcggcgttccggtccatggttagggcccggtagttctacttctgttcatgtttgtgttagatccgtgtttgtgttagatccgtgctgctagcgttcgtacacggatgcgacctgtacgtcagacacgttctgattgctaacttgccagtgtttctctttggggaatcctgggatggctctagccgttccgcagacgggatcgatttcatgattttttttgtttcgttgcatagggtttggtttgcccttttcctttatttcaatatatgccgtgcacttgtttgtcgggtcatcttttcatgcttttttttgtcttggttgtgatgatgtggtctggttgggcggtcgttctagatcggagtagaattctgtttcaaactacctggtggatttattaattttggatctgtatgtgtgtgccatacatattcatagttacgaattgaagatgatggatggaaatatcgatctaggataggtatacatgttgatgcgggttttactgatgcatatacagagatgctttttgttcgcttggttgtgatgatgtggtgtggttgggcggtcgttcattcgttctagatcggagtagaatactgtttcaaactacctggtgtatttattaattttggaactgtatgtgtgtgtcatacatcttcatagttacgagtttaagatggatggaaatatcgatctaggataggtatacatgttgatgtgggttttactgatgcatatacatgatggcatatgcagcatctattcatatgctctaaccttgagtacctatctattataataaacaagtatgttttataattattttgatcttgatatacttggatgatggcatatgcagcagctatatgtggatttttttagccctgccttcatacgctatttatttgcttggtactgtttcttttgtcgatgctcaccctgttgtttggtgttacttctgcaggtcgactctagaggatccaccggtcgccaccatggccctgtccaacaagttcatcggcgacgacatgaagatgacctaccacatggacggctgcgtgaacggccactacttcaccgtgaagggcgagggcagcggcaagccctacgagggcacccagacctccaccttcaaggtgaccatggccaacggcggccccctggccttctccttcgacatcctgtccaccgtgttcatgtacggcaaccgctgcttcaccgcctaccccaccagcatgcccgactacttcaagcaggccttccccgacggcatgtcctacgagagaaccttcacctacgaggacggcggcgtggccaccgccagctgggagatcagcctgaagggcaactgcttcgagcacaagtccaccttccacggcgtgaacttccccgccgacggccccgtgatggccaagaagaccaccggctgggacccctccttcgagaagatgaccgtgtgcgacggcatcttgaagggcgacgtgaccgccttcctgatgctgcagggcggcggcaactacagatgccagttccacacctcctacaagaccaagaagcccgtgaccatgccccccaaccacgtggtggagcaccgcatcgccagaaccgacctggacaagggcggcaacagcgtgcagctgaccgagcacgccgtggcccacatcacctccgtggtgcccttctgaagcggccgcaacctagacttgtccatcttctggattggccaacttaattaatgtatgaaataaaaggatgcacacatagtgacatgctaatcactataatgtgggcatcaaagttgtgtgttatgtgtaattactagttatctgaataaaagagaaagagatcatccatatttcttatcctaaatgaatgtcacgtgtctttataattctttgatgaaccagatgcatttcattaaccaaatccatatacatataaatattaatcatatataattaatatcaattgggttagcaaaacaaatctagtctaggtgtgttttgcgaattcg

SEQ ID NO: 75 - DNA, 2272 bp, synthetic construct
  misc_feature 1..2272: note = RAB17 PRO-MOCRE-PINII TERM
  source 1..2272: mol_type = other DNA
ctatagtattttaaaattgcattaacaaacatgtcctaattggtactcctgagatactataccctcctgttttaaaatagttggcattatcgaattatcattttactttttaatgttttctcttcttttaatatattttatgaattttaatgtattttaaaatgttatgcagttcgctctggacttttctgctgcgcctacacttgggtgtactgggcctaaattcagcctgaccgaccgcctgcattgaataatggatgagcaccggtaaaatccgcgtacccaactttcgagaagaaccgagacgtggcgggccgggccaccgacgcacggcaccagcgactgcacacgtcccgccggcgtacgtgtacgtgctgttccctcactggccgcccaatccactcatgcatgcccacgtacacccctgccgtggcgcgcccagatcctaatcctttcgccgttctgcacttctgctgcctataaatggcggcatcgaccgtcacctgcttcaccaccggcgagccacatcgagaacacgatcgagcacacaagcacgaagactcgtttaggagaaaccacaaaccaccaagccgtgcaagcaccaagcttggtcacccggtccgggcctagaaggccagcttcaagtttgtacaaaaaagcaggcttcgaaggagatagaaccgatccaccatgtccaacctgctcacggttcaccagaaccttccggctcttccagtggacgcgacgtccgatgaagtcaggaagaacctcatggacatgttccgcgacaggcaagcgttcagcgagcacacctggaagatgctgctctccgtctgccgctcctgggctgcatggtgcaagctgaacaacaggaagtggttccccgctgagcccgaggacgtgagggattaccttctgtacctgcaagcgcgaggtttgtttctgcttctacctttgatatatatataataattatcattaattagtagtaatataatatttcaaatatttttttcaaaataaaagaatgtagtatatagcaattgcttttctgtagtttataagtgtgtatattttaatttataacttttctaatatatgaccaaaacatggtgatgcctaggtctggcagtgaagaccatccagcaacaccttggacaactgaacatgcttcacaggcgctccggcctcccgcgccccagcgactcgaacgccgtgagcctcgtcatgcgccgcatcaggaaggaaaacgtcgatgccggcgaaagggcaaagcaggccctcgcgttcgagaggaccgatttcgaccaggtccgcagcctgatggagaacagcgacaggtgccaggacattaggaacctggcgttcctcggaattgcatacaacacgctcctcaggatcgcggaaattgcccgcattcgcgtgaaggacattagccgcaccgacggcggcaggatgcttatccacattggcaggaccaagacgctcgtttccaccgcaggcgtcgaaaaggccctcagcctcggagtgaccaagctcgtcgaacgctggatctccgtgtccggcgtcgcggacgacccaaacaactacctcttctgccgcgtccgcaagaacggggtggctgcccctagcgccaccagccaactcagcacgagggccttggaaggtattttcgaggccacccaccgcctgatctacggcgcgaaggatgacagcggtcaacgctacctcgcatggtccgggcactccgcccgcgttggagctgctagggacatggcccgcgccggtgtttccatccccgaaatcatgcaggcgggtggatggacgaacgtgaacattgtcatgaactacattcgcaaccttgacagcgagacgggcgcaatggttcgcctcctggaagatggtgactgagctagacccagctttcttgtacaaagtggccgttaacggatccagacttgtccatcttctggattggccaacttaattaatgtatgaaataaaaggatgcacacatagtgacatgctaatcactataatgtgggcatcaaagttgtgtgttatgtgtaattactagttatctgaataaaagagaaagagatcatccatatttcttatcctaaatgaatgtcacgtgtctttataattctttgatgaaccagatgcatttcattaaccaaatccatatacatataaatattaatcatatataattaatatcaattgggttagcaaaacaaatctagtctaggtgtgttttgcgaattgcggc

SEQ ID NO: 76 - DNA, 10435 bp, synthetic construct
  misc_feature 1..10435: note = PHP06
  source 1..10435: mol_type = other DNA
acctggcggaagttcctattccgaagttcctattctctagaaagtataggaacttcagatccaccggctagaggatccaccatggttgaacaagatggattgcacgcaggttctccggccgcttgggtggagaggctattcggctatgactgggcacaacagacaatcggctgctctgatgccgccgtgttccggctgtcagcgcaggggcgcccggttctttttgtcaagaccgacctgtccggtgccctgaatgaactgcaggacgaggcagcgcggctatcgtggctggccacgacgggcgttccttgcgcagctgtgctcgacgttgtcactgaagcgggaagggactggctgctattgggcgaagtgccggggcaggatctcctgtcatctcaccttgctcctgccgagaaagtatccatcatggctgatgcaatgcggcggctgcatacgcttgatccggctacctgcccattcgaccaccaagcgaaacatcgcatcgagcgagcacgtactcggatggaagccggtcttgtcgatcaggatgatctggacgaagagcatcaggggctcgcgccagccgaactgttcgccaggctcaaggcgcgcatgcccgacggcgatgatctcgtcgtgacccatggcgatgcctgcttgccgaatatcatggtggaaaatggccgcttttctggattcatcgactgtggccggctgggtgtggcggaccgctatcaggacatagcgttggctacccgtgatattgctgaagagcttggcggcgaatgggctgaccgcttcctcgtgctttacggtatcgccgctcccgattcgcagcgcatcgccttctatcgccttcttgacgagttcttctgaggatccaccatggttaacctagacttgtccatcttctggattggccaacttaattaatgtatgaaataaaaggatgcacacatagtgacatgctaatcactataatgtgggcatcaaagttgtgtgttatgtgtaattactagttatctgaataaaagagaaagagatcatccatatttcttatcctaaatgaatgtcacgtgtctttataattctttgatgaaccagatgcatttcattaaccaaatccatatacatataaatattaatcatatataattaatatcaattgggttagcaaaacaaatctagtctaggtgtgttttgcgaatgcggccgggtaccgagctcgaattcggcccaagtttgtacaaaaaagcaggctccggccagaatggcccggaccgaagctggccgctctagaactaggcatggagtcaaagattcaaatagaggacctaacagaactcgccgtaaagactggcgaacagttcatacagagtctcttacgactcaatgacaagaagaaaatcttcgtcaacatggtggagcacgacacgcttgtctactccaaaaatatcaaagatacagtctcagaagaccaaagggcaattgagacttttcaacaaagggtaatatccggaaacctcctcggattccattgcccagctatctgtcactttattgtgaagatagtggaaaaggaaggtggctcctacaaatgccatcattgcgataaaggaaaggccatcgttgaagatgcctctgccgacagtggtcccaaagatggacccccacccacgaggagcatcgtggaaaaagaagacgttccaaccacgtcttcaaagcaagtggattgatgtgatatctccactgacgtaagggatgacgcacaatcccactaagctgacctagtggcagtgcagcgtgacccggtcgtgcccctctctagagataatgagcattgcatgtctaagttataaaaaattaccacatattttttttgtcacacttgtttgaagtgcagtttatctatctttatacatatatttaaactttactctacgaataatataatctatagtactacaataatatcagtgttttagagaatcatataaatgaacagttagacatggtctaaaggacaattgagtattttgacaacaggactctacagttttatctttttagtgtgcatgtgttctcctttttttttgcaaatagcttcacctatataatacttcatccattttattagtacatccatttagggtttagggttaatggtttttatagactaatttttttagtacatctattttattctattttagcctctaaattaagaaaactaaaactctattttagtttttttatttaataatttagatataaaatagaataaaataaagtgactaaaaattaaacaaataccctttaagaaattaaaaaaactaaggaaacatttttcttgtttcgagtagataatgccagcctgttaaacgccgtcgacgagtctaacggacaccaaccagcgaaccagcagcgtcgcgtcgggccaagcgaagcagacggcacggcatctctgtcgctgcctctggacccctctcgagagttccgctccaccgttggacttgctccgctgtcggcatccagaaattgcgtggcggagcggcagacgtgagccggcacggcaggcggcctcctcctcctctcacggcaccggcagctacgggggattcctttcccaccgctccttcgctttcccttcctcgcccgccgtaataaatagacaccccctccacaccctctttccccaacctcgtgttgttcggagcgcacacacacacaaccagatctcccccaaatccacccgtcggcacctccgcttcaaggtacgccgctcgtcctcccccccccccctctctaccttctctagatcggcgttccggtccatggttagggcccggtagttctacttctgttcatgtttgtgttagatccgtgtttgtgttagatccgtgctgctagcgttcgtacacggatgcgacctgtacgtcagacacgttctgattgctaacttgccagtgtttctctttggggaatcctgggatggctctagccgttccgcagacgggatcgatttcatgattttttttgtttcgttgcatagggtttggtttgcccttttcctttatttcaatatatgccgtgcacttgtttgtcgggtcatcttttcatgcttttttttgtcttggttgtgatgatgtggtctggttgggcggtcgttctagatcggagtagaattctgtttcaaactacctggtggatttattaattttggatctgtatgtgtgtgccatacatattcatagttacgaattgaagatgatggatggaaatatcgatctaggataggtatacatgttgatgcgggttttactgatgcatatacagagatgctttttgttcgcttggttgtgatgatgtggtgtggttgggcggtcgttcattcgttctagatcggagtagaatactgtttcaaactacctggtgtatttattaattttggaactgtatgtgtgtgtcatacatcttcatagttacgagtttaagatggatggaaatatcgatctaggataggtatacatgttgatgtgggttttactgatgcatatacatgatggcatatgcagcatctattcatatgctctaaccttgagtacctatctattataataaacaagtatgttttataattattttgatcttgatatacttggatgatggcatatgcagcagctatatgtggatttttttagccctgccttcatacgctatttatttgcttggtactgtttcttttgtcgatgctcaccctgttgtttggtgttacttctgcaggcctcctccgagaacgtcatcaccgagttcatgcgcttcaaggtgcgcatggagggcaccgtgaacggccacgagttcgagatcgagggcgagggcgagggccgcccctacgagggccacaacaccgtgaagctgaaggtgaccaagggcggccccctgcccttcgcctgggacatcctgtccccccagttccagtacggctccaaggtgtacgtgaagcaccccgccgacatccccgactacaagaagctgtccttccccgagggcttcaagtgggagcgcgtgatgaacttcgaggacggcggcgtggcgaccgtgacccaggactcctccctgcaggacggctgcttcatctacaaggtgaagttcatcggcgtgaacttcccctccgacggccccgtgatgcagaagaagaccatgggctgggaggcctccaccgagcgcctgtacccccgcgacggcgtgctgaagggcgagacccacaaggccctgaagctgaaggacggcggccactacctggtggagttcaagtccatctacatggccaagaagcccgtgcagctgcccggctactactacgtggacgccaagctggacatcacctcccacaacgaggactacaccatcgtggagcagtacgagcgcaccgagggccgccaccacctgttcctgtagggatctcgatagggatctgttaacgatccccggcggtgtcccccactgaagaaactatgtgctgtagtatagccgctgcccgctggctagctagctagttgagtcatttagcggcgatgattgagtaataatgtgtcacgcatcaccatgcatgggtggcagtgtcagtgtgagcaatgacctgaatgaacaattgaaatgaaaagaaaaaagtattgttccaaattaaacgttttaaccttttaataggtttatacaataattgatatatgttttctgtatatgtctaatttgttatcatccatttagatatagacaaaaaaaatctaagaactaaaacaaatgctaatttgaaatgaagggagtatatattgggataatgtcgatgagatccctcgtaatatcaccgacatcacacgtgtccagttaatgtatcagtgatacgtgtattcacatttgttgcgcgtaggcgtacccaacaattttgatcgactatcagaaagtcaacggaagcgagtcgacctcgaggcatggagtcaaagattcaaatagaggacctaacagaactcgccgtaaagactggcgaacagttcatacagagtctcttacgactcaatgacaagaagaaaatcttcgtcaacatggtggagcacgacacgcttgtctactccaaaaatatcaaagatacagtctcagaagaccaaagggcaattgagacttttcaacaaagggtaatatccggaaacctcctcggattccattgcccagctatctgtcactttattgtgaagatagtggaaaaggaaggtggctcctacaaatgccatcattgcgataaaggaaaggccatcgttgaagatgcctctgccgacagtggtcccaaagatggacccccacccacgaggagcatcgtggaaaaagaagacgttccaaccacgtcttcaaagcaagtggattgatgtgatatctccactgacgtaagggatgacgcacaatcccactaagctgaccgggcccggccgaagcttgcatgcctgcaggtcgactctagaggatctgcaccggacactgtctggtggcataccagacagtccggtgtgccagatcagggcacccttcggttcctttgctcctttgcttttgaaccctaactttgatcgtttattggtttgtgttgaacctttatgcacctgtggaatatataatctagaacaaactagttagtccaatcatttgtgttgggcattcaaccaccaaaattatttataggaaaaggttaaaccttatttccctttcaatctccccctttttggtgattgatgccaacacaaaccaaagaaaatatataagtgcagaattgaactagtttgcataaggtaagtgcataggttacttagaattaaatcaatttatacttttacttgatatgcatggttgctttcttttattttaacattttggaccacatttgcaccacttgttttgttttttgcaaatctttttggaaattctttttcaaagtcttttgcaaatagtcaaaggtatatgaataagattgtaagaagcattttcaagatttgaaatttctccccctgtttcaaatgcttttcctttgactaaacaaaactccccctgaataaaattctcctcttagctttcaagagggttttaaatagatatcaattggaaatatatttagatgctaattttgaaaatataccaattgaaaatcaacataccaatttgaaattaaacataccaatttaaaaaatttcaaaaagtggtggtgcggtccttttgctttgggcttaatatttctccccctttggcattaatcgccaaaaacggagactttgtgagccatttatactttctccccattggtaaatgaaatatgagtgaaagattataccaaatttggacagtgatgcggagtgacggcgaaggataaacgataccgttagagtggagtggaagccttgtcttcgccgaagactccatttccctttcaatctacgacttagcatagaaatacacttgaaaacacattagtcgtagccacgaaagagatatgatcaaaggtatacaaatgagctatgtgtgtaatgtttcaatcaaagtttcgagaatcaagaatatttagctcattcctaagtttgctaaaggttttatcatctaatggtttggtaaagatatcgactaattgttctttggtgctaacataagcaatctcgatatcacccctttgttggtgatccctcaaaaagtgataccgaatgtctatgtgcttagtgcggctgtgttcaacgggattatccgccatgcagatagcactctcattgtcacataggagagggactttgctcaatttgtagccatagtccctaaggttttgcctcatccaaagtaattgcacacaacaatgtcctgcggcaatatacttggcttcggcggtagaaagagctattgagttttgtttctttgaagtccaagacaccagggatctccctagaaactgacaagtccctgatgtgctcttcctatcaattttacaccctgcccaatcggcatctgaatatcctattaaatcaaaggtggatcccttggggtaccaaagaccaaatttaggagtgtaaactaaatatctcatgattcttttcacggccctaaggtgaacttccttaggatcggcttggaatcttgcacacatgcatatagaaagcatactatctggtcgagatgcacataaatagagtaaagatcctatcatcgaccggtataccttttggtctacggatttacctcccgtgtcgaggtcgagatgcccattagttcccatgggtgtcctgatgggcttggcatccttcattccaaacttgttgagtatgtcttgaatgtactttgtttggctgatgaaggtgccatcttggagttgcttgacttgaaatcctagaaaatatttcaacttccccatcatagacatctcgaatttcggaatcatgatcctactaaactcttcacaagtagatttgttagtagacccaaatataatatcatcaacataaatttggcatacaaacaaaacttttgaaatggttttagtaaagagagtaggatcggctttactgactctgaagccattagtgataagaaaatctcttaggcattcataccatgctgttggggcttgcttgagcccataaagcgcctttgagagtttataaacatggttagggtactcactatcttcaaagccgagaggttgctcaacatagacctattcaccccatttgatcacttttttggtccttcaggatctaatagttatgtataatttagagtctcttgtttaatggccagatatttctaattaatctaagaatttatgatattttttaattttttatcatgtctgatgagaattaacataaaggctcaattgggtcctgaattaataatagagtgaaaattaatccagaggctctattagaaccttcaattagtaataccaagatatatataagatagtagagtatagtttaaatgttggcattgttcattctttcttttgttatttaatttatgctttccacggtggttagtggttacttctgaagggtccaaataatgcatgaagagtttgaggacaagaagtctgccctaaaaatagcgatgcaaaggcatggtgtccaagccatacatatagcgcactaattttatcagcagaacaatggtatttataggtcctagtgcccaggcaacaagagacacgaataaagcatcgatcacgacaccatggcggcgacaatggcagtgacgacgatggtgacgaggagcaaggagagctggtcgtcattgcaggtcccggcggtggcattcccttggaagccacgaggtggcaagaccggcggcctcgagttccctcgccgggcgatgttcgccagcgtcggcctcaacgtgtgcccgggcgtcccggcggggcgcgacccgcgggagcccgatcccaaggtcgtccgggcggcctgcggcctggtccaggcacaagtcctcttccaggggtttaactgggagtcgtgcaagcagcagggaggctggtacaacaggctcaaggcccaggtcgacgacatcgccaaggccggcgtcacgcacgtctggctgcctccaccctcgcactccgtctcgccacaaggctacatgccaggccgcctatacgacctggacgcgtccaagtacggcacggcggcggagctcaagtccctgatagcggcgttccacggcaggggcgtgcagtgcgtggcggacatcgtcatcaaccaccggtgcgcggaaaagaaggacgcgcgcggcgtgtactgcatcttcgagggcgggactcccgacgaccgcctggactggggccccgggatgatctgcagcgacgacacgcagtactcggacgggacggggcaccgcgacacgggcgaggggttcgcggcggcgcccgacatcgaccacctcaacccgcgcgtgcagcgggagctctccgcctggctcaactggctcaggtccgacgccgtggggttcgacggctggcgcctcgacttcgccaagggctactcgccggccgtcgccagaatgtacgtggagagcacggggccgccgagcttcgtcgtcgcggagatatggaactcgctgagctacagcggggacggcaagccggcgcccaaccaggaccagtgccggcaggagctgctggactggacgcgggccgtcggcgggcccgccatggcgttcgacttccccaccaagggcctgctgcaggcgggcgtgcagggggagctgtggcggctgcgcgacagctccggcaacgcggccggcctgatcgggtgggcgcccgagaaggccgtcaccttcgtcgacaaccatgacaccgggtcgacgcagaagctctggccgttcccatccgacaaggtcatgcagggctacgcctacatcctcacccatccaggagtcccctgcattttctacgaccacatgttcgactggaacctgaagcaggagatatccacgctgtctgccatcagggcgcggaacggcatccgcgccgggagcaagctgcggatcctcgtggcggacgcggacgcgtacgtggccgtcgtcgacgagaaggtcatggtgaagatcgggacaaggtacggcgtgagcagcgtggtcccgtcggatttccacccggcggcgcacggcaaggactactgcgtctgggagaaagcgagcctccgcgtcccggcggggcgccacctctagcagctcagattgctcagtcttgtgctgcattgcaaacacagcagcacgacactgcataacgtcttttccttgagatctgacaaagcagcattagtccgttgatcggtggaagaccactcgtcagtgttgagttgaatgtttgatcaataaaatacggcaatgctgtaagggttgttttttatgccattgataatacactgtactgttcagttgttgaactctatttcttagccatgccaagtgcttttcttattttgaataacattacagcaaaaagttgaaagacaaaaaaaaaaacccccgaacagagtgctttgggtcccaagctactttagactgtgttcggcgttccccctaaatttctccccctatatctcactcacttgtcacatcagcgttctctttcccctatatctccacgtcgacgcggccgctctagaactagtggatcccccgggctgcaggaattcctcgagaccgtacgtgcgcgcgaatgcatccagatcttccctctagtcaaggccttaagcgcgcgttcgaacgcgcggttaagcttggtcacccggtccgggcctagaaggccgatctcccgggcacccagctttcttgtacaaagtggccgttaacggatcccggtgaagttcctattccgaagttcctattctccagaaagtataggaacttcattaccgat

SEQ ID NO: 77 - DNA, 4682 bp, synthetic construct
  misc_feature 1..4682: note = PG47 PRO-ZM-BT1 TP~ZM-AA1-IN2-1 TERM
  source 1..4682: mol_type = other DNA
aagcttgcatgcctgcaggtcgactctagaggatctgcaccggacactgtctggtggcataccagacagtccggtgtgccagatcagggcacccttcggttcctttgctcctttgcttttgaaccctaactttgatcgtttattggtttgtgttgaacctttatgcacctgtggaatatataatctagaacaaactagttagtccaatcatttgtgttgggcattcaaccaccaaaattatttataggaaaaggttaaaccttatttccctttcaatctccccctttttggtgattgatgccaacacaaaccaaagaaaatatataagtgcagaattgaactagtttgcataaggtaagtgcataggttacttagaattaaatcaatttatacttttacttgatatgcatggttgctttcttttattttaacattttggaccacatttgcaccacttgttttgttttttgcaaatctttttggaaattctttttcaaagtcttttgcaaatagtcaaaggtatatgaataagattgtaagaagcattttcaagatttgaaatttctccccctgtttcaaatgcttttcctttgactaaacaaaactccccctgaataaaattctcctcttagctttcaagagggttttaaatagatatcaattggaaatatatttagatgctaattttgaaaatataccaattgaaaatcaacataccaatttgaaattaaacataccaatttaaaaaatttcaaaaagtggtggtgcggtccttttgctttgggcttaatatttctccccctttggcattaatcgccaaaaacggagactttgtgagccatttatactttctccccattggtaaatgaaatatgagtgaaagattataccaaatttggacagtgatgcggagtgacggcgaaggataaacgataccgttagagtggagtggaagccttgtcttcgccgaagactccatttccctttcaatctacgacttagcatagaaatacacttgaaaacacattagtcgtagccacgaaagagatatgatcaaaggtatacaaatgagctatgtgtgtaatgtttcaatcaaagtttcgagaatcaagaatatttagctcattcctaagtttgctaaaggttttatcatctaatggtttggtaaagatatcgactaattgttctttggtgctaacataagcaatctcgatatcacccctttgttggtgatccctcaaaaagtgataccgaatgtctatgtgcttagtgcggctgtgttcaacgggattatccgccatgcagatagcactctcattgtcacataggagagggactttgctcaatttgtagccatagtccctaaggttttgcctcatccaaagtaattgcacacaacaatgtcctgcggcaatatacttggcttcggcggtagaaagagctattgagttttgtttctttgaagtccaagacaccagggatctccctagaaactgacaagtccctgatgtgctcttcctatcaattttacaccctgcccaatcggcatctgaatatcctattaaatcaaaggtggatcccttggggtaccaaagaccaaatttaggagtgtaaactaaatatctcatgattcttttcacggccctaaggtgaacttccttaggatcggcttggaatcttgcacacatgcatatagaaagcatactatctggtcgagatgcacataaatagagtaaagatcctatcatcgaccggtataccttttggtctacggatttacctcccgtgtcgaggtcgagatgcccattagttcccatgggtgtcctgatgggcttggcatccttcattccaaacttgttgagtatgtcttgaatgtactttgtttggctgatgaaggtgccatcttggagttgcttgacttgaaatcctagaaaatatttcaacttccccatcatagacatctcgaatttcggaatcatgatcctactaaactcttcacaagtagatttgttagtagacccaaatataatatcatcaacataaatttggcatacaaacaaaacttttgaaatggttttagtaaagagagtaggatcggctttactgactctgaagccattagtgataagaaaatctcttaggcattcataccatgctgttggggcttgcttgagcccataaagcgcctttgagagtttataaacatggttagggtactcactatcttcaaagccgagaggttgctcaacatagacctattcaccccatttgatcacttttttggtccttcaggatctaatagttatgtataatttagagtctcttgtttaatggccagatatttctaattaatctaagaatttatgatattttttaattttttatcatgtctgatgagaattaacataaaggctcaattgggtcctgaattaataatagagtgaaaattaatccagaggctctattagaaccttcaattagtaataccaagatatatataagatagtagagtatagtttaaatgttggcattgttcattctttcttttgttatttaatttatgctttccacggtggttagtggttacttctgaagggtccaaataatgcatgaagagtttgaggacaagaagtctgccctaaaaatagcgatgcaaaggcatggtgtccaagccatacatatagcgcactaattttatcagcagaacaatggtatttataggtcctagtgcccaggcaacaagagacacgaataaagcatcgatcacgacaccatggcggcgacaatggcagtgacgacgatggtgacgaggagcaaggagagctggtcgtcattgcaggtcccggcggtggcattcccttggaagccacgaggtggcaagaccggcggcctcgagttccctcgccgggcgatgttcgccagcgtcggcctcaacgtgtgcccgggcgtcccggcggggcgcgacccgcgggagcccgatcccaaggtcgtccgggcggcctgcggcctggtccaggcacaagtcctcttccaggggtttaactgggagtcgtgcaagcagcagggaggctggtacaacaggctcaaggcccaggtcgacgacatcgccaaggccggcgtcacgcacgtctggctgcctccaccctcgcactccgtctcgccacaaggctacatgccaggccgcctatacgacctggacgcgtccaagtacggcacggcggcggagctcaagtccctgatagcggcgttccacggcaggggcgtgcagtgcgtggcggacatcgtcatcaaccaccggtgcgcggaaaagaaggacgcgcgcggcgtgtactgcatcttcgagggcgggactcccgacgaccgcctggactggggccccgggatgatctgcagcgacgacacgcagtactcggacgggacggggcaccgcgacacgggcgaggggttcgcggcggcgcccgacatcgaccacctcaacccgcgcgtgcagcgggagctctccgcctggctcaactggctcaggtccgacgccgtggggttcgacggctggcgcctcgacttcgccaagggctactcgccggccgtcgccagaatgtacgtggagagcacggggccgccgagcttcgtcgtcgcggagatatggaactcgctgagctacagcggggacggcaagccggcgcccaaccaggaccagtgccggcaggagctgctggactggacgcgggccgtcggcgggcccgccatggcgttcgacttccccaccaagggcctgctgcaggcgggcgtgcagggggagctgtggcggctgcgcgacagctccggcaacgcggccggcctgatcgggtgggcgcccgagaaggccgtcaccttcgtcgacaaccatgacaccgggtcgacgcagaagctctggccgttcccatccgacaaggtcatgcagggctacgcctacatcctcacccatccaggagtcccctgcattttctacgaccacatgttcgactggaacctgaagcaggagatatccacgctgtctgccatcagggcgcggaacggcatccgcgccgggagcaagctgcggatcctcgtggcggacgcggacgcgtacgtggccgtcgtcgacgagaaggtcatggtgaagatcgggacaaggtacggcgtgagcagcgtggtcccgtcggatttccacccggcggcgcacggcaaggactactgcgtctgggagaaagcgagcctccgcgtcccggcggggcgccacctctagcagctcagattgctcagtcttgtgctgcattgcaaacacagcagcacgacactgcataacgtcttttccttgagatctgacaaagcagcattagtccgttgatcggtggaagaccactcgtcagtgttgagttgaatgtttgatcaataaaatacggcaatgctgtaagggttgttttttatgccattgataatacactgtactgttcagttgttgaactctatttcttagccatgccaagtgcttttcttattttgaataacattacagcaaaaagttgaaagacaaaaaaaaaaacccccgaacagagtgctttgggtcccaagctactttagactgtgttcggcgttccccctaaatttctccccctatatctcactcacttgtcacatcagcgttctctttcccctatatctccacg

SEQ ID NO: 78 - DNA, 3602 bp, synthetic construct
  misc_feature 1..3602: note = PG47 PRO-BA-BARNASE-IN2-1 TERM
  source 1..3602: mol_type = other DNA
aagcttgcatgcctgcaggtcgactctagaggatctgcaccggacactgtctggtggcataccagacagtccggtgtgccagatcagggcacccttcggttcctttgctcctttgcttttgaaccctaactttgatcgtttattggtttgtgttgaacctttatgcacctgtggaatatataatctagaacaaactagttagtccaatcatttgtgttgggcattcaaccaccaaaattatttataggaaaaggttaaaccttatttccctttcaatctccccctttttggtgattgatgccaacacaaaccaaagaaaatatataagtgcagaattgaactagtttgcataaggtaagtgcataggttacttagaattaaatcaatttatacttttacttgatatgcatggttgctttcttttattttaacattttggaccacatttgcaccacttgttttgttttttgcaaatctttttggaaattctttttcaaagtcttttgcaaatagtcaaaggtatatgaataagattgtaagaagcattttcaagatttgaaatttctccccctgtttcaaatgcttttcctttgactaaacaaaactccccctgaataaaattctcctcttagctttcaagagggttttaaatagatatcaattggaaatatatttagatgctaattttgaaaatataccaattgaaaatcaacataccaatttgaaattaaacataccaatttaaaaaatttcaaaaagtggtggtgcggtccttttgctttgggcttaatatttctccccctttggcattaatcgccaaaaacggagactttgtgagccatttatactttctccccattggtaaatgaaatatgagtgaaagattataccaaatttggacagtgatgcggagtgacggcgaaggataaacgataccgttagagtggagtggaagccttgtcttcgccgaagactccatttccctttcaatctacgacttagcatagaaatacacttgaaaacacattagtcgtagccacgaaagagatatgatcaaaggtatacaaatgagctatgtgtgtaatgtttcaatcaaagtttcgagaatcaagaatatttagctcattcctaagtttgctaaaggttttatcatctaatggtttggtaaagatatcgactaattgttctttggtgctaacataagcaatctcgatatcacccctttgttggtgatccctcaaaaagtgataccgaatgtctatgtgcttagtgcggctgtgttcaacgggattatccgccatgcagatagcactctcattgtcacataggagagggactttgctcaatttgtagccatagtccctaaggttttgcctcatccaaagtaattgcacacaacaatgtcctgcggcaatatacttggcttcggcggtagaaagagctattgagttttgtttctttgaagtccaagacaccagggatctccctagaaactgacaagtccctgatgtgctcttcctatcaattttacaccctgcccaatcggcatctgaatatcctattaaatcaaaggtggatcccttggggtaccaaatttaaggagtgtaaactaaatatctcatgattcttttcacggccctaaggtgaacttccttaggatcggcttggaatcttgcacacatgcatatagaaagcatagctatctggtcgagatgcacataaatagagtaaagatcctatcatcgaccggtataccttttggtcgtacggatttacctcccgtgtcgaggtcgagatgcccattagttcccatgggtgtacctgatgggcttggcatccttcattccaaacttgttgagtatgtcttgaatgtactttgtttggctgatgaaggtgccatcttggagttgcttgacttgaaatcctagaaaatatttcaacttccccatcatagacatctcgaatttcggaatcatgatcctactaaactcttcacaagtagatttgttagtagacccaaatataatatcatcaacataaatttggcatacaaacaaaacttttgaaatggttttagtaaagagagtaggatcggctttactgactctgaagccattagtgataagaaaatctcttaggcattcataccatgctgttggggcttgcttgagcccataaagcgcctttgagagtttataaacatggttagggtactcactatcttcaaagccgagaggttgctcaacatagacctattcaccccatttgatcacttttttggtccttcaggatctaatagttatgtataatttagagtctcttgtttaatggccagatatttctaattaatctaagaatttatgatattttttaattttttatcatgtctgatgagaattaacataaaggctcaattgggtcctgaattaataatagagtgaaaattaatccagaggctctattagaaccttcaattagtaataccaagatatatataagatagtagagtatagtttaaatgttggcattgttcattctttcttttgttatttaatttatgctttccacggtggttagtggttacttctgaagggtccaaataatgcatgaagagtttgaggacaagaagtctgccctaaaaatagcgatgcaaaggcatggtgtccaagccatacatatagcgcactaattttatcagcagaacaatggtatttataggtcctagtgcccaggcaacaagagacacgaataaagcatcgatcacgacaccagatctcatggcacaggttatcaacacgtttgacggggttgcggattatcttcagacatatcataagctacctgataattacattacaaaatcagaagcacaagccctcggctgggtggcatcaaaagggaaccttgcagacgtcgctccggggaaaagcatcggcggagacatcttctcaaacagggaaggcaaactcccgtaagtttctgcttctacctttgatatatatataataattatcattaattagtagtaatataatatttcaaatatttttttcaaaataaaagaatgtagtatatagcaattgcttttctgtagtttataagtgtgtatattttaatttataacttttctaatatatgaccaaaacatggtgatgtgcaggggcaaaagcggacgaacatggcgtgaagcggatattaactatacatcaggcttcagaaattcagaccggattctttactcaggcgactggctgatttacaaaacaacggaccattatcagacctttacaaaaatcagataactgcagctagacttgtccatcttctggattggccaacttaattaatgtatgaaataaaaggatgcacacatagtgacatgctaatcactataatgtgggcatcaaagttgtgtgttatgtgtaattactagttatctgaataaaagagaaagagatcatccatatttcttatcctaaatgaatgtcacgtgtctttataattctttgatgaaccagatgcatttcattaaccaaatccatatacatataaatattaatcatatataattaatatcaattgggttagcaaaacaaatctag

SEQ ID NO: 79 - DNA, 1188 bp, Streptomyces griseolus
  source 1..1188: mol_type = unassigned DNA
atgaccggaaccatccccttccctcaggaccgcagttgtccctaccacccgccgacgaactaccggccgctgcgcgaatccggtccgctctcgcacgtcagcttctacaacggccgcaaggtctgggcggtgaccgggcacgccgaggcgcggacgctgctggtcgacccccgcctgtcgtccgaccggcagaatccggccttccccatcccggtcgagcggttcgaggccgtccggcgggtgcgcactcccttgatcggcgtggacgatcccgagcacaacactcagcgccgcatgctgatccccagcttcagcgtcaaacggaccgccgcgctccgaccgcagatccaacagatcgtggacggcctcctggaccggatgctggagcagggcccacccgccgagttggtctccgcgttcgcgctccccgtcccgtcgatggtgatctgctcgctgctcggcgtcccgtacgcggaccacgagttcttcgaggaccggtcgcgccgcatcctccgcggaggcacggccgaggagagcgagcaggcccgacgcgaactggagggatacctcgcggatctgatggcccgcaaggagacggatccgggtgacggactgctcgacgagctgatcgccgagcggctccgggccggcacgctccaacaccaggaactggtccggctggccatggtcctgctggtcgccgggcacgagaccaccgccaacatgatctccctcggcaccttcgccctcctcgaacaccccgaccagttggcccagttgaggtccgacgagagtctgatgccgggcgcggtcgaggagttgctgcggttcttgtccatagccgacggcatgctgcgggtcgcgaccgccgacatcgagatcgccgggcacaccatccgcaccggcgacggcgtggtgttctccacctccctgatcaaccgcgacgcgacggcctacccgtcaccggacgaactccatgtcgaccgttcggcccgccaccacgtcgcgttcggcttcggcatccaccagtgcctgggccagaatctggcccgcgccgagttggagatcgcgctacgctcgctgttccggcgagtgcccgacctgcgactcgccgtgccggctgccgaaattcccttcaagccgggggaaactctccaaggaatgatcgaactgccgctgatctggtag

SEQ ID NO: 80 - protein, 406 aa, Streptomyces griseolus
MTDTATTPQTTDAPAFPSNRSCPYQLPDGYAQLRDTPGPLHRVTLYDGRQAWVVTKHEAARKLLGDPRLSSNRTDDNFPATSPRFEAVRESPQAFIGLDPPEHGTRRRMTISEFTVKRIKGMRPEVEEVVHGFLDEMLAAGPTADLVSQFALPVPSMVICRLLGVPYADHEFFQDASKRLVQSTDAQSALTARNDLAGYLDGLITQFQTEPGAGLVGALVADQLANGEIDREELISTAMLLLIAGHETTASMTSLSVITLLDHPEQYAALRADRSLVPGAVEELLRYLAIADIAGGRVATADIEVEGHLIRAGEGVIVVNSIANRDGTVYEDPDALDIHRSARHHLAFGFGVHQCLGQNLARLELEVILNALMDRVPTLRLAVPVEQLVLRPGTTIQGVNELPVTW

SEQ ID NO: 81 - DNA, 1284 bp, Escherichia coli
  source 1..1284: mol_type = unassigned DNA
atgtcgaataacgctttacaaacaattattaacgcccggttaccaggcgaagaggggctgtggcagattcatctgcaggacggaaaaatcagcgccattgatgcgcaatccggcgtgatgcccataactgaaaacagcctggatgccgaacaaggtttagttataccgccgtttgtggagccacatattcacctggacaccacgcaaaccgccggacaaccgaactggaatcagtccggcacgctgtttgaaggcattgaacgctgggccgagcgcaaagcgttattaacccatgacgatgtgaaacaacgcgcatggcaaacgctgaaatggcagattgccaacggcattcagcatgtgcgtacccatgtcgatgtttcggatgcaacgctaactgcgctgaaagcaatgctggaagtgaagcaggaagtcgcgccgtggattgatctgcaaatcgtcgccttccctcaggaagggattttgtcgtatcccaacggtgaagcgttgctggaagaggcgttacgcttaggggcagatgtagtgggggcgattccgcattttgaatttacccgtgaatacggcgtggagtcgctgcataaaaccttcgccctggcgcaaaaatacgaccgtctcatcgacgttcactgtgatgagatcgatgacgagcagtcgcgctttgtcgaaaccgttgctgccctggcgcaccatgaaggcatgggcgcgcgagtcaccgccagccacaccacggcaatgcactcctataacggggcgtatacctcacgcctgttccgcttgctgaaaatgtccggtattaactttgtcgccaacccgctggtcaatattcatctgcaaggacgtttcgatacgtatccaaaacgtcgcggcatcacgcgcgttaaagagatgctggagtccggcattaacgtctgctttggtcacgatgatgtcttcgatccgtggtatccgctgggaacggcgaatatgctgcaagtgctgcatatggggctgcatgtttgccagttgatgggctacgggcagattaacgatggcctgaatttaatcacccaccacagcgcaaggacgttgaatttgcaggattacggcattgccgccggaaacagcgccaacctgattatcctgccggctgaaaatgggtttgatgcgctgcgccgtcaggttccggtacgttattcggtacgtggcggcaaggtgattgccagcacacaaccggcacaaaccaccgtatatctggagcagccagaagccatcgattacaaacgttga

SEQ ID NO: 82 - protein, 427 aa, Escherichia coli
MSNNALQTIINARLPGEEGLWQIHLQDGKISAIDAQSGVMPITENSLDAEQGLVIPPFVEPHIHLDTTQTAGQPNWNQSGTLFEGIERWAERKALLTHDDVKQRAWQTLKWQIANGIQHVRTHVDVSDATLTALKAMLEVKQEVAPWIDLQIVAFPQEGILSYPNGEALLEEALRLGADVVGAIPHFEFTREYGVESLHKTFALAQKYDRLIDVHCDEIDDEQSRFVETVAALAHHEGMGARVTASHTTAMHSYNGAYTSRLFRLLKMSGINFVANPLVNIHLQGRFDTYPKRRGITRVKEMLESGINVCFGHDDVFDPWYPLGTANMLQVLHMGLHVCQLMGYGQINDGLNLITHHSARTLNLQDYGIAAGNSANLIILPAENGFDALRRQVPVRYSVRGGKVIASTQPAQTTVYLEQPEAIDYKR

SEQ ID NO: 83 - DNA, 1645 bp, synthetic construct
  misc_feature 1..1645: note = ZM-U6 POLIII CHR8 PRO-GT1 GUIDE RNA-ZM-U6 POLIII CHR8 TERM
  source 1..1645: mol_type = other DNA
tgagagtacaatgatgaacctagattaatcaatgccaaagtctgaaaaatgcaccctcagtctatgatccagaaaatcaagattgcttgaggccctgttcggttgttccggattagagccccggattaattcctagccggattacttctctaatttatatagattttgatgagctggaatgaatcctggcttattccggtacaaccgaacaggccctgaaggataccagtaatcgctgagctaaattggcatgctgtcagagtgtcagtattgcagcaaggtagtgagataaccggcatcatggtgccagtttgatggcaccattagggttagagatggtggccatgggcgcatgtcctggccaactttgtatgatatatggcagggtgaataggaaagtaaaattgtattgtaaaaagggatttcttctgtttgttagcgcatgtacaaggaatgcaagttttgagcgagggggcatcaaagatctggctgtgtttccagctgtttttgttagccccatcgaatccttgacataatgatcccgcttaaataagcaacctcgcttgtatagttccttgtgctctaacacacgatgatgataagtcgtaaaatagtggtgtccaaagaatttccaggcccagttgtaaaagctaaaatgctattcgaatttctactagcagtaagtcgtgtttagaaattatttttttatataccttttttccttctatgtacagtaggacacagtgtcagcgccgcgttgacggagaatatttgcaaaaaagtaaaagagaaagtcatagcggcgtatgtgccaaaaacttcgtcacagagagggccataagaaacatggcccacggcccaatacgaagcaccgcgacgaagcccaaacagcagtccgtaggtggagcaaagcgctgggtaatacgcaaacgttttgtcccaccttgactaatcacaagagtggagcgtaccttataaaccgagccgcaagcaccgaattggcgcgccgttcactgccgtataggcaggtgcatcatggactcatggttttagagctagaaatagcaagttaaaataaggctagtccgttatcaacttgaaaaagtggcaccgagtcggtgctgttcactgccgtataggcagcgctgtacggcgtggtagacgttttagagctagaaatagcaagttaaaataaggctagtccgttatcaacttgaaaaagtggcaccgagtcggtgctgttcactgccgtataggcagccagcaacgtccagcgcgcgttttagagctagaaatagcaagttaaaataaggctagtccgttatcaacttgaaaaagtggcaccgagtcggtgctgttcactgccgtataggcaggggtgcccgtgcgttgcaagttttagagctagaaatagcaagttaaaataaggctagtccgttatcaacttgaaaaagtggcaccgagtcggtgctgttcactgccgtataggcaggcatttcgcgagtcaaatttgttttagagctagaaatagcaagttaaaataaggctagtccgttatcaacttgaaaaagtggcaccgagtcggtgctgttcactgccgtataggcaggttcactgccgtataggcaggcgatcgctttttttt

SEQ ID NO: 84 - DNA, 4452 bp, synthetic construct
  misc_feature 1..4452: note = moDCAS9 EXON1-STLS1 INTRON-moCAS9 EXON2
  source 1..4452: mol_type = other DNA
atggcaccgaagaagaagcgcaaggtgctggatcttcagcttagactgggcggtggcggtggatccgacaagaagtacagcatcggcctcgccatcggcaccaactcggtgggctgggccgtcatcacggacgaatataaggtcccgtcgaagaagttcaaggtcctcggcaatacagaccgccacagcatcaagaaaaacttgatcggcgccctcctgttcgatagcggcgagaccgcggaggcgaccaggctcaagaggaccgccaggagacggtacactaggcgcaagaacaggatctgctacctgcaggagatcttcagcaacgagatggcgaaggtggacgactccttcttccaccgcctggaggaatcattcctggtggaggaggacaagaagcatgagcggcacccaatcttcggcaacatcgtcgacgaggtaagtttctgcttctacctttgatatatatataataattatcattaattagtagtaatataatatttcaaatatttttttcaaaataaaagaatgtagtatatagcaattgcttttctgtagtttataagtgtgtatattttaatttataacttttctaatatatgaccaaaacatggtgatgtgcaggtggcctaccacgagaagtacccgacaatctaccacctccggaagaaactggtggacagcacagacaaggcggacctccggctcatctaccttgccctcgcgcatatgatcaagttccgcggccacttcctcatcgagggcgacctgaacccggacaactccgacgtggacaagctgttcatccagctcgtgcagacgtacaatcaactgttcgaggagaaccccataaacgctagcggcgtggacgccaaggccatcctctcggccaggctctcgaaatcaagaaggctggagaaccttatcgcgcagttgccaggcgaaaagaagaacggcctcttcggcaaccttattgcgctcagcctcggcctgacgccgaacttcaaatcaaacttcgacctcgcggaggacgccaagctccagctctcaaaggacacctacgacgacgacctcgacaacctcctggcccagataggagaccagtacgcggacctcttcctcgccgccaagaacctctccgacgctatcctgctcagcgacatccttcgggtcaacaccgaaattaccaaggcaccgctgtccgccagcatgattaaacgctacgacgagcaccatcaggacctcacgctgctcaaggcactcgtccgccagcagctccccgagaagtacaaggagatcttcttcgaccaatcaaaaaacggctacgcgggatatatcgacggcggtgccagccaggaagagttctacaagttcatcaaaccaatcctggagaagatggacggcaccgaggagttgctggtcaagctcaacagggaggacctcctcaggaagcagaggaccttcgacaacggctccatcccgcatcagatccacctgggcgaactgcatgccatcctgcggcgccaggaggacttctacccgttcctgaaggataaccgggagaagatcgagaagatcttgacgttccgcatcccatactacgtgggcccgctggctcgcggcaactcccggttcgcctggatgacccggaagtcggaggagaccatcacaccctggaactttgaggaggtggtcgataagggcgctagcgctcagagcttcatcgagcgcatgaccaacttcgataaaaacctgcccaatgaaaaagtcctccccaagcactcgctgctctacgagtacttcaccgtgtacaacgagctcaccaaggtcaaatacgtcaccgagggcatgcggaagccggcgttcctgagcggcgagcagaagaaggcgatagtggacctcctcttcaagaccaacaggaaggtgaccgtgaagcaattaaaagaggactacttcaagaaaatagagtgcttcgactccgtggagatctcgggcgtggaggatcggttcaacgcctcactcggcacgtatcacgacctcctcaagatcattaaagacaaggacttcctcgacaacgaggagaacgaggacatcctcgaggacatcgtcctcaccctgaccctgttcgaggaccgcgaaatgatcgaggagaggctgaagacctacgcgcacctgttcgacgacaaggtcatgaaacagctcaagaggcgccgctacactggttggggaaggctgtcccgcaagctcattaatggcatcagggacaagcagagcggcaagaccatcctggacttcctcaagtccgacgggttcgccaaccgcaacttcatgcagctcattcacgacgactcgctcacgttcaaggaagacatccagaaggcacaggtgagcgggcagggtgactccctccacgaacacatcgccaacctggccggctcgccggccattaaaaagggcatcctgcagacggtcaaggtcgtcgacgagctcgtgaaggtgatgggccggcacaagcccgaaaatatcgtcatagagatggccagggagaaccagaccacccaaaaagggcagaagaactcgcgcgagcggatgaaacggatcgaggagggcattaaagagctcgggtcccagatcctgaaggagcaccccgtggaaaatacccagctccagaatgaaaagctctacctctactacctgcagaacggccgcgacatgtacgtggaccaggagctggacattaatcggctatcggactacgacgtcgacgccatcgtgccgcagtcgttcctcaaggacgatagcatcgacaacaaggtgctcacccggtcggataaaaatcggggcaagagcgacaacgtgcccagcgaggaggtcgtgaagaagatgaaaaactactggcgccagctcctcaacgcgaaactgatcacccagcgcaagttcgacaacctgacgaaggcggaacgcggtggcttgagcgaactcgataaggcgggcttcataaaaaggcagctggtcgagacgcgccagatcacgaagcatgtcgcccagatcctggacagccgcatgaatactaagtacgatgaaaacgacaagctgatccgggaggtgaaggtgatcacgctgaagtccaagctcgtgtcggacttccgcaaggacttccagttctacaaggtccgcgagatcaacaactaccaccacgcccacgacgcctacctgaatgcggtggtcgggaccgccctgatcaagaagtacccgaagctggagtcggagttcgtgtacggcgactacaaggtctacgacgtgcgcaaaatgatcgccaagtccgagcaggagatcggcaaggccacggcaaaatacttcttctactcgaacatcatgaacttcttcaagaccgagatcaccctcgcgaacggcgagatccgcaagcgcccgctcatcgaaaccaacggcgagacgggcgagatcgtctgggataagggccgggatttcgcgacggtccgcaaggtgctctccatgccgcaagtcaatatcgtgaaaaagacggaggtccagacgggcgggttcagcaaggagtccatcctcccgaagcgcaactccgacaagctcatcgcgaggaagaaggattgggacccgaaaaaatatggcggcttcgacagcccgaccgtcgcatacagcgtcctcgtcgtggcgaaggtggagaagggcaagtcaaagaagctcaagtccgtgaaggagctgctcgggatcacgattatggagcggtcctccttcgagaagaacccgatcgacttcctagaggccaagggatataaggaggtcaagaaggacctgattattaaactgccgaagtactcgctcttcgagctggaaaacggccgcaagaggatgctcgcctccgcaggcgagttgcagaagggcaacgagctcgccctcccgagcaaatacgtcaatttcctgtacctcgctagccactatgaaaagctcaagggcagcccggaggacaacgagcagaagcagctcttcgtggagcagcacaagcattacctggacgagatcatcgagcagatcagcgagttctcgaagcgggtgatcctcgccgacgcgaacctggacaaggtgctgtcggcatataacaagcaccgcgacaaaccaatacgcgagcaggccgaaaatatcatccacctcttcaccctcaccaacctcggcgctccggcagccttcaagtacttcgacaccacgattgaccggaagcggtacacgagcacgaaggaggtgctcgatgcgacgctgatccaccagagcatcacagggctctatgaaacacgcatcgacctgagccagctgggcggagacggtggcggtggatccctggatcttcagcttagactgggcaagagaccacgggaccgccacgatggcgagctgggaggccgcaagcgggcaaggtag

SEQ ID NO: 85 - protein, 1368 aa, synthetic construct [sequence omitted]

SEQ ID NO: 86 - DNA, 1000 bp, synthetic construct
  misc_feature 1..1000: note = ZM-U6 POLIII CHR8 PRO
  source 1..1000: mol_type = other DNA
tgagagtacaatgatgaacctagattaatcaatgccaaagtctgaaaaatgcaccctcagtctatgatccagaaaatcaagattgcttgaggccctgttcggttgttccggattagagccccggattaattcctagccggattacttctctaatttatatagattttgatgagctggaatgaatcctggcttattccggtacaaccgaacaggccctgaaggataccagtaatcgctgagctaaattggcatgctgtcagagtgtcagtattgcagcaaggtagtgagataaccggcatcatggtgccagtttgatggcaccattagggttagagatggtggccatgggcgcatgtcctggccaactttgtatgatatatggcagggtgaataggaaagtaaaattgtattgtaaaaagggatttcttctgtttgttagcgcatgtacaaggaatgcaagttttgagcgagggggcatcaaagatctggctgtgtttccagctgtttttgttagccccatcgaatccttgacataatgatcccgcttaaataagcaacctcgcttgtatagttccttgtgctctaacacacgatgatgataagtcgtaaaatagtggtgtccaaagaatttccaggcccagttgtaaaagctaaaatgctattcgaatttctactagcagtaagtcgtgtttagaaattatttttttatataccttttttccttctatgtacagtaggacacagtgtcagcgccgcgttgacggagaatatttgcaaaaaagtaaaagagaaagtcatagcggcgtatgtgccaaaaacttcgtcacagagagggccataagaaacatggcccacggcccaatacgaagcaccgcgacgaagcccaaacagcagtccgtaggtggagcaaagcgctgggtaatacgcaaacgttttgtcccaccttgactaatcacaagagtggagcgtaccttataaaccgagccgcaagcaccgaatt

SEQ ID NO: 87 - DNA, 4452 bp, synthetic construct; identical to SEQ ID NO: 84
  misc_feature 1..4452: note = DCAS9-RP
  source 1..4452: mol_type = other DNA

SEQ ID NO: 88 - protein, 1420 aa, synthetic construct
  REGION 1..1420: note = DCAS9-RP
MAPKKKRKVLDLQLRLGGGGGSDKKYSIGLAIGTNSVGWAVITDEYKVPSKKFKVLGNTDRHSIKKNLIGALLFDSGETAEATRLKRTARRRYTRRKNRICYLQEIFSNEMAKVDDSFFHRLEESFLVEEDKKHERHPIFGNIVDEVAYHEKYPTIYHLRKKLVDSTDKADLRLIYLALAHMIKFRGHFLIEGDLNPDNSDVDKLFIQLVQTYNQLFEENPINASGVDAKAILSARLSKSRRLENLIAQLPGEKKNGLFGNLIALSLGLTPNFKSNFDLAEDAKLQLSKDTYDDDLDNLLAQIGDQYADLFLAAKNLSDAILLSDILRVNTEITKAPLSASMIKRYDEHHQDLTLLKALVRQQLPEKYKEIFFDQSKNGYAGYIDGGASQEEFYKFIKPILEKMDGTEELLVKLNREDLLRKQRTFDNGSIPHQIHLGELHAILRRQEDFYPFLKDNREKIEKILTFRIPYYVGPLARGNSRFAWMTRKSEETITPWNFEEVVDKGASAQSFIERMTNFDKNLPNEKVLPKHSLLYEYFTVYNELTKVKYVTEGMRKPAFLSGEQKKAIVDLLFKTNRKVTVKQLKEDYFKKIECFDSVEISGVEDRFNASLGTYHDLLKIIKDKDFLDNEENEDILEDIVLTLTLFEDREMIEERLKTYAHLFDDKVMKQLKRRRYTGWGRLSRKLINGIRDKQSGKTILDFLKSDGFANRNFMQLIHDDSLTFKEDIQKAQVSGQGDSLHEHIANLAGSPAIKKGILQTVKVVDELVKVMGRHKPENIVIEMARENQTTQKGQKNSRERMKRIEEGIKELGSQILKEHPVENTQLQNEKLYLYYLQNGRDMYVDQELDINRLSDYDVDAIVPQSFLKDDSIDNKVLTRSDKNRGKSDNVPSEEVVKKMKNYWRQLLNAKLITQRKFDNLTKAERGGLSELDKAGFIKRQLVETRQITKHVAQILDSRMNTKYDENDKLIREVKVITLKSKLVSDFRKDFQFYKVREINNYHHAHDAYLNAVVGTALIKKYPKLESEFVYGDYKVYDVRKMIAKSEQEIGKATAKYFFYSNIMNFFKTEITLANGEIRKRPLIETNGETGEIVWDKGRDFATVRKVLSMPQVNIVKKTEVQTGGFSKESILPKRNSDKLIARKKDWDPKKYGGFDSPTVAYSVLVVAKVEKGKSKKLKSVKELLGITIMERSSFEKNPIDFLEAKGYKEVKKDLIIKLPKYSLFELENGRKRMLASAGELQKGNELALPSKYVNFLYLASHYEKLKGSPEDNEQKQLFVEQHKHYLDEIIEQISEFSKRVILADANLDKVLSAYNKHRDKPIREQAENIIHLFTLTNLGAPAAFKYFDTTIDRKRYTSTKEVLDATLIHQSITGLYETRIDLSQLGGDGGGGSLDLQLRLGKRPRDRHDGELGGRKRAR

SEQ ID NO: 89 - DNA, 3938 bp, synthetic construct
  misc_feature 1..3938: note = RB-LOXP-OSACTIN PRO,INTRON-FRT1-MOPAT-35STERM-FRT87-LB
  source 1..3938: mol_type = other DNA
gtttacccgccaatatatcctgtcaaacactgatagtttaaactgaaggcgggaaacgacaatctgatcatgagcggagaattaagggagtcacgttatgacccccgccgatgacgcgggacaagccgttttacgtttggaactgacagaaccgcaacgttgaaggagccactcagcaagctggtacgattgtaatacgactcactatagggcgaattgagcgctgtttaaacgctcttcaactggaagagcggttactaccggctggatggcggggccttgatcgtgcaccgccggcgtccggactaactaactagtcgagctagttaccctatgaggtgacatgaagcgctcacggttactatgacggttagcttcacgactgttggtggcagtagcgtacgacttagctatagttccggacttacccttaagataacttcgtatagcatacattatacgaagttatacctggtggcgccgctaggaccgaattatcgaattcctgcagcccatccctcagccgcctttcactatcttttttgcccgagtcattgtcatgtgaaccttggcatgtataatcggtgaattgcgtcgattttcctcttataggtgggccaatgaatccgtgtgatcgcgtctgattggctagagatatgtttcttccttgttggatgtattttcatacataatcatatgcatacaaatatttcattacactttatagaaatggtcagtaataaaccctatcactatgtctggtgtttcattttatttgcttttaaacgaaaattgacttcctgattcaatatttaaggatcgtcaacggtgtgcagttactaaattctggtttgtaggaactatagtaaactattcaagtcttcacttattgtgcactcacctctcgccacatcaccacagatgttattcacgtcttaaatttgaactacacatcatattgacacaatattttttttaaataagcgattaaaacctagcctctatgtcaacaatggtgtacataaccagcgaagtttagggagtaaaaaacatcgccttacacaaagttcgctttaaaaaataaagagtaaattttactttggaccacccttcaaccaatgtttcactttagaacgagtaattttattattgtcactttggaccaccctcaaatcttttttccatctacatccaatttatcatgtcaaagaaatggtctacatacagctaaggagatttatcgacgaatagtagctagcatactcgaggtcattcatatgcttgagaagagagtcgggatagtccaaaataaaacaaaggtaagattacctggtcaaaagtgaaaacatcagttaaaaggtggtataaagtaaaatatcggtaataaaaggtggcccaaagtgaaatttactcttttctactattataaaaattgaggatgtttttgtcggtactttgatacgtcatttttgtatgaattggtttttaagtttattcgcttttggaaatgcatatctgtatttgagtcgggttttaagttcgtttgcttttgtaaatacagagggatttgtataagaaatatctttaaaaaaacccatatgctaatttgacataatttttgagaaaaatatatattcaggcgaattctcacaatgaacaataataagattaaaatagctttcccccgttgcagcgcatgggtattttttctagtaaaaataaaagataaacttagactcaaaacatttacaaaaacaacccctaaagttcctaaagcccaaagtgctatccacgatccatagcaagcccagcccaacccaacccaacccaacccaccccagtccagccaactggacaatagtctccacacccccccactatcaccgtgagttgtccgcacgcaccgcacgtctcgcagccaaaaaaaaaaaaagaaagaaaaaaaagaaaaagaaaaaacagcaggtgggtccgggtcgtgggggccggaaacgcgaggaggatcgcgagccagcgacgaggccggccctccctccgcttccaaagaaacgccccccatcgccactatatacatacccccccctctcctcccatccccccaaccctaccaccaccaccaccaccacctccacctcctcccccctcgctgccggacgacgagctcctcccccctccccctccgccgccgccgcgccggtaaccaccccgcccctctcctctttctttctccgttttttttttccgtctcggtctcgatctttggccttggtagtttgggtgggcgagaggcggcttcgtgcgcgcccagatcggtgcgcgggaggggcgggatctcgcggctggggctctcgccggcgtggatcaggcccggatctcgcggggaatggggctctcggatgtagatctgcgatccgccgttgttgggggagatgatggggggtttaaaatttccgccatgctaaacaagatcaggaagaggggaaaagggcactatggtttatatttttatatatttctgctgcttcgtcaggcttagatgtgctagatctttctttcttctttttgtgggtagaatttgaatccctcagcattgttcatcggtagtttttcttttcatgatttgtgacaaatgcagcctcgtgcggagcttttttgtaggtagaaggatctcgactctagaggatcaattcgctagcgaagttcctattccgaagttcctattctctagaaagtataggaacttcagatccaccgggatccacacgacaccatgtcccccgagcgccgccccgtcgagatccgcccggccaccgccgccgacatggccgccgtgtgcgacatcgtgaaccactacatcgagacctccaccgtgaacttccgcaccgagccgcagaccccgcaggagtggatcgacgacctggagcgcctccaggaccgctacccgtggctcgtggccgaggtggagggcgtggtggccggcatcgcctacgccggcccgtggaaggcccgcaacgcctacgactggaccgtggagtccaccgtgtacgtgtcccaccgccaccagcgcctcggcctcggctccaccctctacacccacctcctcaagagcatggaggcccagggcttcaagtccgtggtggccgtgatcggcctcccgaacgacccgtccgtgcgcctccacgaggccctcggctacaccgcccgcggcaccctccgcgccgccggctacaagcacggcggctggcacgacgtcggcttctggcagcgcgacttcgagctgccggccccgccgcgcccggtgcgcccggtgacgcagatctgagtcgacctgcaggcatgccgctgaaatcaccagtctctctctacaaatctatctctctctataataatgtgtgagtagttcccagataagggaattagggttcttatagggtttcgctcatgtgttgagcatataagaaacccttagtatgtatttgtatttgtaaaatacttctatcaataaaatttctaattcctaaaaccaaaatccagtggcgagctcgagcccgggtggatcctctagagtcgacctgcagaagcttcggtcctagcgtatacgaagttcctattccgaagttcctattctccagaaagtataggaacttctgtacacctgagctgattccgatgacttcgtaggttcctagctcaagccgctcgtgtccaagcgtcacttacgattagctaatgattacggcatctaggaccgactagctaactaactagtacgtagaattaattcattccgattaatcgtggcctcttgctcttcaggatgaagagctatgtttaaacgtgcaagcgctactagacaattcagtacattaaaaacgtccgcaatgtgttattaagttgtctaagcgtcaatttgtttacaccacaatatatcctgccac

SEQ ID NO: 90 - DNA, 4682 bp, synthetic construct; identical to SEQ ID NO: 77
  misc_feature 1..4682: note = PG47 PRO-ZMAA1-IN2-1 TERM
  source 1..4682: mol_type = other DNA

SEQ ID NO: 91 - DNA, 3042 bp, synthetic construct
  misc_feature 1..3042: note = LTP2 PRO-AMCYAN1-PINII TERM
  source 1..3042: mol_type = other DNA
gtgcagcgtgacccggtcgtgcccctctctagagataatgagcattgcatgtctaagttataaaaaattaccacatattttttttgtcacacttgtttgaagtgcagtttatctatctttatacatatatttaaactttactctacgaataatataatctatagtactacaataatatcagtgttttagagaatcatataaatgaacagttagacatggtctaaaggacaattgagtattttgacaacaggactctacagttttatctttttagtgtgcatgtgttctcctttttttttgcaaatagcttcacctatataatacttcatccattttattagtacatccatttagggtttagggttaatggtttttatagactaatttttttagtacatctattttattctattttagcctctaaattaagaaaactaaaactctattttagtttttttatttaataatttagatataaaatagaataaaataaagtgactaaaaattaaacaaataccctttaagaaattaaaaaaactaaggaaacatttttcttgtttcgagtagataatgccagcctgttaaacgccgtcgacgagtctaacggacaccaaccagcgaaccagcagcgtcgcgtcgggccaagcgaagcagacggcacggcatctctgtcgctgcctctggacccctctcgagagttccgctccaccgttggacttgctccgctgtcggcatccagaaattgcgtggcggagcggcagacgtgagccggcacggcaggcggcctcctcctcctctcacggcaccggcagctacgggggattcctttcccaccgctccttcgctttcccttcctcgcccgccgtaataaatagacaccccctccacaccctctttccccaacctcgtgttgttcggagcgcacacacacacaaccagatctcccccaaatccacccgtcggcacctccgcttcaaggtacgccgctcgtcctcccccccccccctctctaccttctctagatcggcgttccggtccatgcatggttagggcccggtagttctacttctgttcatgtttgtgttagatccgtgtttgtgttagatccgtgctgctagcgttcgtacacggatgcgacctgtacgtcagacacgttctgattgctaacttgccagtgtttctctttggggaatcctgggatggctctagccgttccgcagacgggatcgatttcatgattttttttgtttcgttgcatagggtttggtttgcccttttcctttatttcaatatatgccgtgcacttgtttgtcgggtcatcttttcatgcttttttttgtcttggttgtgatgatgtggtctggttgggcggtcgttctagatcggagtagaattctgtttcaaactacctggtggatttattaattttggatctgtatgtgtgtgccatacatattcatagttacgaattgaagatgatggatggaaatatcgatctaggataggtatacatgttgatgcgggttttactgatgcatatacagagatgctttttgttcgcttggttgtgatgatgtggtgtggttgggcggtcgttcattcgttctagatcggagtagaatactgtttcaaactacctggtgtatttattaattttggaactgtatgtgtgtgtcatacatcttcatagttacgagtttaagatggatggaaatatcgatctaggataggtatacatgttgatgtgggttttactgatgcatatacatgatggcatatgcagcatctattcatatgctctaaccttgagtacctatctattataataaacaagtatgttttataattattttgatcttgatatacttggatgatggcatatgcagcagctatatgtggatttttttagccctgccttcatacgctatttatttgcttggtactgtttcttttgtcgatgctcaccctgttgtttggtgttacttctgcaggtcgactctagaggatccaccggtcgccaccatggccctgtccaacaagttcatcggcgacgacatgaagatgacctaccacatggacggctgcgtgaacggccactacttcaccgtgaagggcgagggcagcggcaagccctacgagggcacccagacctccaccttcaaggtgaccatggccaacggcggccccctggccttctccttcgacatcctgtccaccgtgttcatgtacggcaaccgctgcttcaccgcctaccccaccagcatgcccgactacttcaagcaggccttccccgacggcatgtcctacgagagaaccttcacctacgaggacggcggcgtggccaccgccagctgggagatcagcctgaagggcaactgcttcgagcacaagtccaccttccacggcgtgaacttccccgccgacggccccgtgatggccaagaagaccaccggctgggacccctccttcgagaagatgaccgtgtgcgacggcatcttgaagggcgacgtgaccgccttcctgatgctgcagggcggcggcaactacagatgccagttccacacctcctacaagaccaagaagcccgtgaccatgccccccaaccacgtggtggagcaccgcatcgccagaaccgacctggacaagggcggcaacagcgtgcagctgaccgagcacgccgtggcccacatcacctccgtggtgcccttctgaagcggccgcaacctagacttgtccatcttctggattggccaacttaattaatgtatgaaataaaaggatgcacacatagtgacatgctaatcactataatgtgggcatcaaagttgtgtgttatgtgtaattactagttatctgaataaaagagaaagagatcatccatatttcttatcctaaatgaatgtcacgtgtctttataattctttgatgaaccagatgcatttcattaaccaaatccatatacatataaatattaatcatatataattaatatcaattgggttagcaaaacaaatctagtctaggtgtgttttgcgaatgcgg

SEQ ID NO: 92 - DNA, 3118 bp, synthetic construct
  misc_feature 1..3118: note = UBI1ZM PRO and INTRON-NPTII-PINII TERM
  source 1..3118: mol_type = other DNA
gtgcagcgtgacccggtcgtgcccctctctagagataatgagcattgcatgtctaagttataaaaaattaccacatattttttttgtcacacttgtttgaagtgcagtttatctatctttatacatatatttaaactttactctacgaataatataatctatagtactacaataatatcagtgttttagagaatcatataaatgaacagttagacatggtctaaaggacaattgagtattttgacaacaggactctacagttttatctttttagtgtgcatgtgttctcctttttttttgcaaatagcttcacctatataatacttcatccattttattagtacatccatttagggtttagggttaatggtttttatagactaatttttttagtacatctattttattctattttagcctctaaattaagaaaactaaaactctattttagtttttttatttaataatttagatataaaatagaataaaataaagtgactaaaaattaaacaaataccctttaagaaattaaaaaaactaaggaaacatttttcttgtttcgagtagataatgccagcctgttaaacgccgtcgacgagtctaacggacaccaaccagcgaaccagcagcgtcgcgtcgggccaagcgaagcagacggcacggcatctctgtcgctgcctctggacccctctcgagagttccgctccaccgttggacttgctccgctgtcggcatccagaaattgcgtggcggagcggcagacgtgagccggcacggcaggcggcctcctcctcctctcacggcaccggcagctacgggggattcctttcccaccgctccttcgctttcccttcctcgcccgccgtaataaatagacaccccctccacaccctctttccccaacctcgtgttgttcggagcgcacacacacacaaccagatctcccccaaatccacccgtcggcacctccgcttcaaggtacgccgctcgtcctcccccccccccctctctaccttctctagatcggcgttccggtccatgcatggttagggcccggtagttctacttctgttcatgtttgtgttagatccgtgtttgtgttagatccgtgctgctagcgttcgtacacggatgcgacctgtacgtcagacacgttctgattgctaacttgccagtgtttctctttggggaatcctgggatggctctagccgttccgcagacgggatcgatttcatgattttttttgtttcgttgcatagggtttggtttgcccttttcctttatttcaatatatgccgtgcacttgtttgtcgggtcatcttttcatgcttttttttgtcttggttgtgatgatgtggtctggttgggcggtcgttctagatcggagtagaattctgtttcaaactacctggtggatttattaattttggatctgtatgtgtgtgccatacatattcatagttacgaattgaagatgatggatggaaatatcgatctaggataggtatacatgttgatgcgggttttactgatgcatatacagagatgctttttgttcgcttggttgtgatgatgtggtgtggttgggcggtcgttcattcgttctagatcggagtagaatactgtttcaaactacctggtgtatttattaattttggaactgtatgtgtgtgtcatacatcttcatagttacgagtttaagatggatggaaatatcgatctaggataggtatacatgttgatgtgggttttactgatgcatatacatgatggcatatgcagcatctattcatatgctctaaccttgagtacctatctattataataaacaagtatgttttataattattttgatcttgatatacttggatgatggcatatgcagcagctatatgtggatttttttagccctgccttcatacgctatttatttgcttggtactgtttcttttgtcgatgctcaccctgttgtttggtgttacttctgcagttagatggttgaacaagatggattgcacgcaggttctccggccgcttgggtggagaggctattcggctatgactgggcacaacagacaatcggctgctctgatgccgccgtgttccggctgtcagcgcaggggcgcccggttctttttgtcaagaccgacctgtccggtgccctgaatgaactgcaggacgaggcagcgcggctatcgtggctggccacgacgggcgttccttgcgcagctgtgctcgacgttgtcactgaagcgggaagggactggctgctattgggcgaagtgccggggcaggatctcctgtcatctcaccttgctcctgccgagaaagtatccatcatggctgatgcaatgcggcggctgcatacgcttgatccggctacctgcccattcgaccaccaagcgaaacatcgcatcgagcgagcacgtactcggatggaagccggtcttgtcgatcaggatgatctggacgaagagcatcaggggctcgcgccagccgaactgttcgccaggctcaaggcgcgcatgcccgacggcgatgatctcgtcgtgacccatggcgatgcctgcttgccgaatatcatggtggaaaatggccgcttttctggattcatcgactgtggccggctgggtgtggcggaccgctatcaggacatagcgttggctacccgtgatattgctgaagagcttggcggcgaatgggctgaccgcttcctcgtgctttacggtatcgccgctcccgattcgcagcgcatcgccttctatcgccttcttgacgagttcttctgaggatccaccatggttaacctagacttgtccatcttctggattggccaacttaattaatgtatgaaataaaaggatgcacacatagtgacatgctaatcactataatgtgggcatcaaagttgtgtgttatgtgtaattactagttatctgaataaaagagaaagagatcatccatatttcttatcctaaatgaatgtcacgtgtctttataattctttgatgaaccagatgcatttcattaaccaaatccatatacatataaatattaatcatatataattaatatcaattgggttagcaaaacaaatctagtctaggtgtgttttgc

SEQ ID NO: 93 - DNA, 690 bp, synthetic construct
  misc_feature 1..690: note = AMCYAN1 DNA
  source 1..690: mol_type = other DNA
atggccctgtccaacaagttcatcggcgacgacatgaagatgacctaccacatggacggctgcgtgaacggccactacttcaccgtgaagggcgagggcagcggcaagccctacgagggcacccagacctccaccttcaaggtgaccatggccaacggcggccccctggccttctccttcgacatcctgtccaccgtgttcatgtacggcaaccgctgcttcaccgcctaccccaccagcatgcccgactacttcaagcaggccttccccgacggcatgtcctacgagagaaccttcacctacgaggacggcggcgtggccaccgccagctgggagatcagcctgaagggcaactgcttcgagcacaagtccaccttccacggcgtgaacttccccgccgacggccccgtgatggccaagaagaccaccggctgggacccctccttcgagaagatgaccgtgtgcgacggcatcttgaagggcgacgtgaccgccttcctgatgctgcagggcggcggcaactacagatgccagttccacacctcctacaagaccaagaagcccgtgaccatgccccccaaccacgtggtggagcaccgcatcgccagaaccgacctggacaagggcggcaacagcgtgcagctgaccgagcacgccgtggcccacatcacctccgtggtgcccttctga

SEQ ID NO: 94 - protein, 229 aa, synthetic construct; identical to SEQ ID NO: 72
  REGION 1..229: note = AMCYAN1 PRT

SEQ ID NO: 95 - DNA, 2939 bp, synthetic construct
  misc_feature 1..2939: note = OSACTIN PRO and INTRON-MOPAT-35S TERM
  source 1..2939: mol_type = other DNA
atccctcagccgcctttcactatcttttttgcccgagtcattgtcatgtgaaccttggcatgtataatcggtgaattgcgtcgattttcctcttataggtgggccaatgaatccgtgtgatcgcgtctgattggctagagatatgtttcttccttgttggatgtattttcatacataatcatatgcatacaaatatttcattacactttatagaaatggtcagtaataaaccctatcactatgtctggtgtttcattttatttgcttttaaacgaaaattgacttcctgattcaatatttaaggatcgtcaacggtgtgcagttactaaattctggtttgtaggaactatagtaaactattcaagtcttcacttattgtgcactcacctctcgccacatcaccacagatgttattcacgtcttaaatttgaactacacatcatattgacacaatattttttttaaataagcgattaaaacctagcctctatgtcaacaatggtgtacataaccagcgaagtttagggagtaaaaaacatcgccttacacaaagttcgctttaaaaaataaagagtaaattttactttggaccacccttcaaccaatgtttcactttagaacgagtaattttattattgtcactttggaccaccctcaaatcttttttccatctacatccaatttatcatgtcaaagaaatggtctacatacagctaaggagatttatcgacgaatagtagctagcatactcgaggtcattcatatgcttgagaagagagtcgggatagtccaaaataaaacaaaggtaagattacctggtcaaaagtgaaaacatcagttaaaaggtggtataaagtaaaatatcggtaataaaaggtggcccaaagtgaaatttactcttttctactattataaaaattgaggatgtttttgtcggtactttgatacgtcatttttgtatgaattggtttttaagtttattcgcttttggaaatgcatatctgtatttgagtcgggttttaagttcgtttgcttttgtaaatacagagggatttgtataagaaatatctttaaaaaaacccatatgctaatttgacataatttttgagaaaaatatatattcaggcgaattctcacaatgaacaataataagattaaaatagctttcccccgttgcagcgcatgggtattttttctagtaaaaataaaagataaacttagactcaaaacatttacaaaaacaacccctaaagttcctaaagcccaaagtgctatccacgatccatagcaagcccagcccaacccaacccaacccaacccaccccagtccagccaactggacaatagtctccacacccccccactatcaccgtgagttgtccgcacgcaccgcacgtctcgcagccaaaaaaaaaaaaagaaagaaaaaaaagaaaaagaaaaaacagcaggtgggtccgggtcgtgggggccggaaacgcgaggaggatcgcgagccagcgacgaggccggccctccctccgcttccaaagaaacgccccccatcgccactatatacatacccccccctctcctcccatccccccaaccctaccaccaccaccaccaccacctccacctcctcccccctcgctgccggacgacgagctcctcccccctccccctccgccgccgccgcgccggtaaccaccccgcccctctcctctttctttctccgttttttttttccgtctcggtctcgatctttggccttggtagtttgggtgggcgagaggcggcttcgtgcgcgcccagatcggtgcgcgggaggggcgggatctcgcggctggggctctcgccggcgtggatcaggcccggatctcgcggggaatggggctctcggatgtagatctgcgatccgccgttgttgggggagatgatggggggtttaaaatttccgccatgctaaacaagatcaggaagaggggaaaagggcactatggtttatatttttatatatttctgctgcttcgtcaggcttagatgtgctagatctttctttcttctttttgtgggtagaatttgaatccctcagcattgttcatcggtagtttttcttttcatgatttgtgacaaatgcagcctcgtgcggagcttttttgtaggtagaaggatccacacgacaccatgtcccccgagcgccgccccgtcgagatccgcccggccaccgccgccgacatggccgccgtgtgcgacatcgtgaaccactacatcgagacctccaccgtgaacttccgcaccgagccgcagaccccgcaggagtggatcgacgacctggagcgcctccaggaccgctacccgtggctcgtggccgaggtggagggcgtggtggccggcatcgcctacgccggcccgtggaaggcccgcaacgcctacgactggaccgtggagtccaccgtgtacgtgtcccaccgccaccagcgcctcggcctcggctccaccctctacacccacctcctcaagagcatggaggcccagggcttcaagtccgtggtggccgtgatcggcctcccgaacgacccgtccgtgcgcctccacgaggccctcggctacaccgcccgcggcaccctgcgcgccgccggctacaagcacggcggctggcacgacgtcggcttctggcagcgcgacttcgagctgccggccccgccgcgcccggtgcgcccggtgacgcagatctgagtcgacctgcaggcatgccgctgaaatcaccagtctctctctacaaatctatctctctctataataatgtgtgagtagttcccagataagggaattagggttcttatagggtttcgctcatgtgttgagcatataagaaacccttagtatgtatttgtatttgtaaaatacttctatcaataaaatttctaattcctaaaaccaaaatccagtggcgagct

SEQ ID NO: 96 - DNA, 4452 bp, synthetic construct; identical to SEQ ID NO: 84
  misc_feature 1..4452: note = NLS-EAR MOTIF-G4S LINKER-----LInker R-EAR MOTIF-VIRD2 NLS
  source 1..4452: mol_type = other DNA

SEQ ID NO: 97 - DNA, 606 bp, synthetic construct
  misc_feature 1..606: note = moLEXA DNA
  source 1..606: mol_type = other DNA
atgaaagcgctcaccgcccgccaacaggaggtcttcgacctgatcagggatcacatctcccagacaggcatgccaccaacaagggcggaaatcgcacagaggctcgggtttcgctcgccaaacgctgccgaggagcaccttaaggcgctcgcgcgcaaaggcgttatcgagattgtgagcggagccagccgcggaatcaggctcttacaggaggaggaagagggacttccacttgtgggcagagtggccgctgacgaaccactccttgcccagcagcacatcgaaggacactaccaggtcgacccatccctgttcaagccaaacgccgatttcctcctccgcgtgtccgggatggcgatgaaagacatcggcatcatggacggcgacctgctggccgtccataaaactcaggacgtgcgcaacggccaggtggtggtggcccgcatcgacgatgaggtcacggtgaaacgcctcaagaagcagggcaataaagtggagctcctccccgaaaatagcgagttcaaaccaatcgtggtcgaccttcggcaacagtctttcacgattgagggcctggcggtgggcgttatcaggaacggcgattggctt

SEQ ID NO: 98 - protein, 202 aa, synthetic construct
  REGION 1..202: note = moLEXA PRT
MKALTARQQEVFDLIRDHISQTGMPPTRAEIAQRLGFRSPNAAEEHLKALARKGVIEIVSGASRGIRLLQEEEEGLPLVGRVAADEPLLAQQHIEGHYQVDPSLFKPNADFLLRVSGMAMKDIGIMDGDLLAVHKTQDVRNGQVVVARIDDEVTVKRLKKQGNKVELLPENSEFKPIVVDLRQQSFTIEGLAVGVIRNGDWL

SEQ ID NO: 99 - DNA, 17 bp, Escherichia coli
  source 1..17: mol_type = unassigned DNA
cggaagactctcctccg

SEQ ID NO: 100 - DNA, 297 bp, synthetic construct
  misc_feature 1..297: note = moCBF1A
  source 1..297: mol_type = other DNA
acctgcgccaaggacatccagaaagcggctgcagaagctgctctggcgttccaagacgaaacctgcgacaccacgacgacgaaccacgggctcgatatggaggagactatggtggaggcgatctacacgccagaacagtctgagggcgccttctacatggacgaggagaccatgttcggcatgccaacactgctggacaacatggccgagggcatgcttcttccgccaccatctgtgcagtggaaccacaactacgatggcgagggcgatggcgacgttagcctgtggagctactag

SEQ ID NO: 101 - protein, 98 aa, synthetic construct
  REGION 1..98: note = moCBF1A Maize-opt. gene for Arath CBF1 activation domain
TCAKDIQKAAAEAALAFQDETCDTTTTNHGLDMEETMVEAIYTPEQSEGAFYMDEETMFGMPTLLDNMAEGMLLPPPSVQWNHNYDGEGDGDVSLWSY

SEQ ID NO: 102 - DNA, 11596 bp, synthetic construct
  misc_feature 1..11596: note = PG47-moLEXA-CBF1-IN2 PG47-MOCODA-PINII UBI-NPTII-PINII
  source 1..11596: mol_type = other DNA
aagcttgcatgcctgcaggtcgactctagaggatctgcaccggacactgtctggtggcataccagacagtccggtgtgccagatcagggcacccttcggttcctttgctcctttgcttttgaaccctaactttgatcgtttattggtttgtgttgaacctttatgcacctgtggaatatataatctagaacaaactagttagtccaatcatttgtgttgggcattcaaccaccaaaattatttataggaaaaggttaaaccttatttccctttcaatctccccctttttggtgattgatgccaacacaaaccaaagaaaatatataagtgcagaattgaactagtttgcataaggtaagtgcataggttacttagaattaaatcaatttatacttttacttgatatgcatggttgctttcttttattttaacattttggaccacatttgcaccacttgttttgttttttgcaaatctttttggaaattctttttcaaagtcttttgcaaatagtcaaaggtatatgaataagattgtaagaagcattttcaagatttgaaatttctccccctgtttcaaatgcttttcctttgactaaacaaaactccccctgaataaaattctcctcttagctttcaagagggttttaaatagatatcaattggaaatatatttagatgctaattttgaaaatataccaattgaaaatcaacataccaatttgaaattaaacataccaatttaaaaaatttcaaaaagtggtggtgcggtccttttgctttgggcttaatatttctccccctttggcattaatcgccaaaaacggagactttgtgagccatttatactttctccccattggtaaatgaaatatgagtgaaagattataccaaatttggacagtgatgcggagtgacggcgaaggataaacgataccgttagagtggagtggaagccttgtcttcgccgaagactccatttccctttcaatctacgacttagcatagaaatacacttgaaaacacattagtcgtagccacgaaagagatatgatcaaaggtatacaaatgagctatgtgtgtaatgtttcaatcaaagtttcgagaatcaagaatatttagctcattcctaagtttgctaaaggttttatcatctaatggtttggtaaagatatcgactaattgttctttggtgctaacataagcaatctcgatatcacccctttgttggtgatccctcaaaaagtgataccgaatgtctatgtgcttagtgcggctgtgttcaacgggattatccgccatgcagatagcactctcattgtcacataggagagggactttgctcaatttgtagccatagtccctaaggttttgcctcatccaaagtaattgcacacaacaatgtcctgcggcaatatacttggcttcggcggtagaaagagctattgagttttgtttctttgaagtccaagacaccagggatctccctagaaactgacaagtccctgatgtgctcttcctatcaattttacaccctgcccaatcggcatctgaatatcctattaaatcaaaggtggatcccttggggtaccaaagaccaaatttaggagtgtaaactaaatatctcatgattcttttcacggccctaaggtgaacttccttaggatcggcttggaatcttgcacacatgcatatagaaagcatactatctggtcgagatgcacataaatagagtaaagatcctatcatcgaccggtataccttttggtctacggatttacctcccgtgtcgaggtcgagatgcccattagttcccatgggtgtcctgatgggcttggcatccttcattccaaacttgttgagtatgtcttgaatgtactttgtttggctgatgaaggtgccatcttggagttgcttgacttgaaatcctagaaaatatttcaacttccccatcatagacatctcgaatttcggaatcatgatcctactaaactcttcacaagtagatttgttagtagacccaaatataatatcatcaacataaatttggcatacaaacaaaacttttgaaatggttttagtaaagagagtaggatcggctttactgactctgaagccattagtgataagaaaatctcttaggcattcataccatgctgttggggcttgcttgagcccataaagcgcctttgagagtttataaacatggttagggtactcactatcttcaaagccgagaggttgctcaacatagacctattcaccccatttgatcacttttttggtccttcaggatctaatagttatgtataatttagagtctcttgtttaatggccagatatttctaattaatctaagaatttatgatattttttaattttttatcatgtctgatgagaattaacataaaggctcaattgggtcctgaattaataatagagtgaaaattaatccagaggctctattagaaccttcaattagtaataccaagatatatataagatagtagagtatagtttaaatgttggcattgttcattctttcttttgttatttaatttatgctttccacggtggttagtggttacttctgaagggtccaaataatgcatgaagagtttgaggacaagaagtctgccctaaaaatagcgatgcaaaggcatggtgtccaagccatacatatagcgcactaattttatcagcagaacaatggtatttataggtcctagtgcccaggcaacaagagacacgaataaagcatcgatcacgacaccatgaaagcgctcaccgcccgccaacaggaggtcttcgacctgatcagggatcacatctcccagacaggcatgccaccaacaagggcggaaatcgcacagaggctcgggtttcgctcgccaaacgctgccgaggagcaccttaaggcgctcgcgcgcaaaggcgttatcgagattgtgagcggagccagccgcggaatcaggctcttacaggaggaggaagagggacttccacttgtgggcagagtggccgctgacgaaccactccttgcccagcagcacatcgaaggacactaccaggtcgacccatccctgttcaagccaaacgccgatttcctcctccgcgtgtccgggatggcgatgaaagacatcggcatcatggacggcgacctgctggccgtccataaaactcaggacgtgcgcaacggccaggtggtggtggcccgcatcgacgatgaggtcacggtgaaacgcctcaagaagcagggcaataaagtggagctcctccccgaaaatagcgagttcaaaccaatcgtggtcgaccttcggcaacagtctttcacgattgagggcctggcggtgggcgttatcaggaacggcgattggcttacctgcgccaaggacatccagaaagcggctgcagaagctgctctggcgttccaagacgaaacctgcgacaccacgacgacgaaccacgggctcgatatggaggagactatggtggaggcgatctacacgccagaacagtctgagggcgccttctacatggacgaggagaccatgttcggcatgccaacactgctggacaacatggccgagggcatgcttcttccgccaccatctgtgcagtggaaccacaactacgatggcgagggcgatggcgacgttagcctgtggagctactagcgacgcggccgatctgacaaagcagcattagtccgttgatcggtggaagaccactcgtcagtgttgagttgaatgtttgatcaataaaatacggcaatgctgtaagggttgttttttatgccattgataatacactgtactgttcagttgttgaactctatttcttagccatgccaagtgcttttcttattttgaataacattacagcaaaaagttgaaagacaaaaaaaaaaacccccgaacagagtgctttgggtcccaagctactttagactgtgttcggcgttccccctaaatttctccccctatatctcactcacttgtcacatcagcgttctctttcccctatatctccacgtcgacgcggaagctaagcttgcatgcctgcaggtcgactctagaggatctgcaccggacactgtctggtggcataccagacagtccggtgtgccagatcagggcacccttcggttcctttgctcctttgcttttgaaccctaactttgatcgtttattggtttgtgttgaacctttatgcacctgtggaatatataatctagaacaaactagttagtccaatcatttgtgttgggcattcaaccaccaaaattatttataggaaaaggttaaaccttatttccctttcaatctccccctttttggtgattgatgccaacacaaaccaaagaaaatatataagtgcagaattgaactagtttgcataaggtaagtgcataggttacttagaattaaatcaatttatacttttacttgatatgcatggttgctttcttttattttaacattttggaccacatttgcaccacttgttttgttttttgcaaatctttttggaaattctttttcaaagtcttttgcaaatagtcaaaggtatatgaataagattgtaagaagcattttcaagatttgaaatttctccccctgtttcaaatgcttttcctttgactaaacaaaactccccctgaataaaattctcctcttagctttcaagagggttttaaatagatatcaattggaaatatatttagatgctaattttgaaaatataccaattgaaaatcaacataccaatttgaaattaaacataccaatttaaaaaatttcaaaaagtggtggtgcggtccttttgctttgggcttaatatttctccccctttggcattaatcgccaaaaacggagactttgtgagccatttatactttctccccattggtaaatgaaatatgagtgaaagattataccaaatttggacagtgatgcggagtgacggcgaaggataaacgataccgttagagtggagtggaagccttgtcttcgccgaagactccatttccctttcaatctacgacttagcatagaaatacacttgaaaacacattagtcgtagccacgaaagagatatgatcaaaggtatacaaatgagctatgtgtgtaatgtttcaatcaaagtttcgagaatcaagaatatttagctcattcctaagtttgctaaaggttttatcatctaatggtttggtaaagatatcgactaattgttctttggtgctaacataagcaatctcgatatcacccctttgttggtgatccctcaaaaagtgataccgaatgtctatgtgcttagtgcggctgtgttcaacgggattatccgccatgcagatagcactctcattgtcacataggagagggactttgctcaatttgtagccatagtccctaaggttttgcctcatccaaagtaattgcacacaacaatgtcctgcggcaatatacttggcttcggcggtagaaagagctattgagttttgtttctttgaagtccaagacaccagggatctccctagaaactgacaagtccctgatgtgctcttcctatcaattttacaccctgcccaatcggcatctgaatatcctattaaatcaaaggtggatcccttggggtaccaaagaccaaatttaggagtgtaaactaaatatctcatgattcttttcacggccctaaggtgaacttccttaggatcggcttggaatcttgcacacatgcatatagaaagcatactatctggtcgagatgcacataaatagagtaaagatcctatcatcgaccggtataccttttggtctacggatttacctcccgtgtcgaggtcgagatgcccattagttcccatgggtgtcctgatgggcttggcatccttcattccaaacttgttgagtatgtcttgaatgtactttgtttggctgatgaaggtgccatcttggagttgcttgacttgaaatcctagaaaatatttcaacttccccatcatagacatctcgaatttcggaatcatgatcctactaaactcttcacaagtagatttgttagtagacccaaatataatatcatcaacataaatttggcatacaaacaaaacttttgaaatggttttagtaaagagagtaggatcggctttactgactctgaagccattagtgataagaaaatctcttaggcattcataccatgctgttggggcttgcttgagcccataaagcgcctttgagagtttataaacatggttagggtactcactatcttcaaagccgagaggttgctcaacatagacctattcaccccatttgatcacttttttggtccttcaggatctaatagttatgtataatttagagtctcttgtttaatggccagatatttctaattaatctaagaatttatgatattttttaattttttatcatgtctgatgagaattaacataaaggctcaattgggtcctgaattaataatagagtgaaaattaatccagaggctctattagaaccttcaattagtaataccaagatatatataagatagtagagtatagtttaaatgttggcattgttcattctttcttttgttatttaatttatgctttccacggtggttagtggttacttctgaagggtccaaataatgcatgaagagtttgaggacaagaagtctgccctaaaaatagcgatgcaaaggcatggtgtccaagccatacatatagcgcactaattttatcagcagaacaatggtatttataggtcctagtgcccaggcaacaagagacacgaataaagcatcgatcacgacaccatgagcaacaacgccctccagaccataataaacgcgaggctgccggggaaagagggcctctggcagatccacctccaagacggcaagatcagcgctatagacgcccaatcgggcgtgatgccaatcaccgagaactccctcgacgccgaacaaggtctcgtgatccctccattcgtcgaaccccacatccacctcgacacgacccaaacagcaggtcaacccaactggaaccaatccggcacactcttcgaaggcatcgagcgctgggcagaaaggaaggcgttgctcacacacgacgatgtgaagcagcgcgcatggcaaacgctcaagtggcagatagccaacggcatccagcacgtcagaacgcacgtcgacgtgtccgacgccacgcttacagctctgaaggctatgctcgaggtcaagcaggaggtcgcaccctggatagacctgcagatcgtcgcattcccacaggagggaatcctctcataccccaatggggaagccctcctcgaggaagctctgaggttgggtgctgacgttgtcggcgctatcccacacttcgagttcaccagggagtacggagtcgagtcgttgcataaaaccttcgcactggctcaaaaatacgacagactcatcgacgtccactgcgacgaaatcgacgacgagcagagcagattcgtcgagaccgtggctgcactggcccatagggaaggaatgggtgctagggttacggcgtcacataccaccgcaatgcacagctacaacggggcatacacctcccggctctttaggctcctcaaaatgtccggaatcaacttcgtcgccaaccccctggtcaatatacacctccagggacggttcgacacatacccgaaacgccgcgggataaccagggtgaaggagatgctggagagcggcatcaacgtctgctttggccacgacgacgtcttcgatccatggtacccactcggcaccgctaacatgctccaagtgctgcacatgggtctgcacgtctgccagctcatgggctatggacagatcaacgacggcctcaacctcatcacccaccactctgctcggacactcaacctccaggactacggcatagccgccgggaactcggctaatctcatcatcctcccggcggagaatggattcgatgcacttaggcgccaggtgccagtcaggtattcagtgcgcggaggaaaggtgatagcctccacccaaccagcacagaccaccgtctacctcgaacagccggaagcgatcgactacaagcgctagcactagacttgtccatcttctggattggccaacttaattaatgtatgaaataaaaggatgcacacatagtgacatgctaatcactataatgtgggcatcaaagttgtgtgttatgtgtaattactagttatctgaataaaagagaaagagatcatccatatttcttatcctaaatgaatgtcacgtgtctttataattctttgatgaaccagatgcatttcattaaccaaatccatatacatataaatattaatcatatataattaatatcaattgggttagcaaaacaaatctagtctaggtgtgttttgcggatcagctgcagtgcagcgtgacccggtcgtgcccctctctagagataatgagcattgcatgtctaagttataaaaaattaccacatattttttttgtcacacttgtttgaagtgcagtttatctatctttatacatatatttaaactttactctacgaataatataatctatagtactacaataatatcagtgttttagagaatcatataaatgaacagttagacatggtctaaaggacaattgagtattttgacaacaggactctacagttttatctttttagtgtgcatgtgttctcctttttttttgcaaatagcttcacctatataatacttcatccattttattagtacatccatttagggtttagggttaatggtttttatagactaatttttttagtacatctattttattctattttagcctctaaattaagaaaactaaaactctattttagtttttttatttaataatttagatataaaatagaataaaataaagtgactaaaaattaaacaaataccctttaagaaattaaaaaaactaaggaaacatttttcttgtttcgagtagataatgccagcctgttaaacgccgtcgacgagtctaacggacaccaaccagcgaaccagcagcgtcgcgtcgggccaagcgaagcagacggcacggcatctctgtcgctgcctctggacccctctcgagagttccgctccaccgttggacttgctccgctgtcggcatccagaaattgcgtggcggagcggcagacgtgagccggcacggcaggcggcctcctcctcctctcacggcacggcagctacgggggattcctttcccaccgctccttcgctttcccttcctcgcccgccgtaataaatagacaccccctccacaccctctttccccaacctcgtgttgttcggagcgcacacacacacaaccagatctcccccaaatccacccgtcggcacctccgcttcaaggtacgccgctcgtcctccccccccccccctctctaccttctctagatcggcgttccggtccatggttagggcccggtagttctacttctgttcatgtttgtgttagatccgtgtttgtgttagatccgtgctgctagcgttcgtacacggatgcgacctgtacgtcagacacgttctgattgctaacttgccagtgtttctctttggggaatcctgggatggctctagccgttccgcagacgggatcgatttcatgattttttttgtttcgttgcatagggtttggtttgcccttttcctttatttcaatatatgccgtgcacttgtttgtcgggtcatcttttcatgcttttttttgtcttggttgtgatgatgtggtctggttgggcggtcgttctagatcggagtagaattctgtttcaaactacctggtggatttattaattttggatctgtatgtgtgtgccatacatattcatagttacgaattgaagatgatggatggaaatatcgatctaggataggtatacatgttgatgcgggttttactgatgcatatacagagatgctttttgttcgcttggttgtgatgatgtggtgtggttgggcggtcgttcattcgttctagatcggagtagaatactgtttcaaactacctggtgtatttattaattttggaactgtatgtgtgtgtcatacatcttcatagttacgagtttaagatggatggaaatatcgatctaggataggtatacatgttgatgtgggttttactgatgcatatacatgatggcatatgcagcatctattcatatgctctaaccttgagtacctatctattataataaacaagtatgttttataattattttgatcttgatatacttggatgatggcatatgcagcagctatatgtggatttttttagccctgccttcatacgctatttatttgcttggtactgtttcttttgtcgatgctcaccctgttgtttggtgttacttctgcagatggttgaacaagatggattgcacgcaggttctccggccgcttgggtggagaggctattcggctatgactgggcacaacagacaatcggctgctctgatgccgccgtgttccggctgtcagcgcaggggcgcccggttctttttgtcaagaccgacctgtccggtgccctgaatgaactgcaggacgaggcagcgcggctatcgtggctggccacgacgggcgttccttgcgcagctgtgctcgacgttgtcactgaagcgggaagggactggctgctattgggcgaagtgccggggcaggatctcctgtcatctcaccttgctcctgccgagaaagtatccatcatggctgatgcaatgcggcggctgcatacgcttgatccggctacctgcccattcgaccaccaagcgaaacatcgcatcgagcgagcacgtactcggatggaagccggtcttgtcgatcaggatgatctggacgaagagcatcaggggctcgcgccagccgaactgttcgccaggctcaaggcgcgcatgcccgacggcgatgatctcgtcgtgacccatggcgatgcctgcttgccgaatatcatggtggaaaatggccgcttttctggattcatcgactgtggccggctgggtgtggcggaccgctatcaggacatagcgttggctacccgtgatattgctgaagagcttggcggcgaatgggctgaccgcttcctcgtgctttacggtatcgccgctcccgattcgcagcgcatcgccttctatcgccttcttgacgagttcttctgagagcttactgaaaaaattaacatctcttgctaagatccatggatattcgaacgcgtaggtaccacatggttaacctagacttgtccatcttctggattggccaacttaattaatgtatgaaataaaaggatgcacacatagtgacatgctaatcactataatgtgggcatcaaagttgtgtgttatgtgtaattactagttatctgaataaaagagaaagagatcatccatatttcttatcctaaatgaatgtcacgtgtctttataattctttgatgaaccagatgcatttcattaaccaaatccatatacatataaatattaatcatatataattaatatcaattgggttagcaaaacaaatctagtctaggtgtgttttgcg

SEQ ID NO: 103 - DNA, 10091 bp, synthetic construct
  misc_feature 1..10091: note = 5xUAS-45 35s PRO-ZMAA1-IN2-1 TERM-----INTRON-PMI-PINII
  source 1..10091: mol_type = other DNA
ctgtatatactcacagtcgactctatcagtgatagagtctgtatatactcacagactctatcagtgatagagtctgtatatactcacagactctatcagtgatagagtactgtatatactcacagactctatcagtgatagagtgcactgtatatactcacagactctatcagtgatagagtcgcgacgagacccttcctctatataaggaagttcatttcatttggagaggaccggatggcggcgacaatggcagtgacgacgatggtgacgaggagcaaggagagctggtcgtcattgcaggtcccggcggtggcattcccttggaagccacgaggtggcaagaccggcggcctcgagttccctcgccgggcgatgttcgccagcgtcggcctcaacgtgtgcccgggcgtcccggcggggcgcgacccgcgggagcccgatcccaaggtcgtccgggcggcctgcggcctggtccaggcacaagtcctcttccaggggtttaactgggagtcgtgcaagcagcagggaggctggtacaacaggctcaaggcccaggtcgacgacatcgccaaggccggcgtcacgcacgtctggctgcctccaccctcgcactccgtctcgccacaaggctacatgccaggccgcctatacgacctggacgcgtccaagtacggcacggcggcggagctcaagtccctgatagcggcgttccacggcaggggcgtgcagtgcgtggcggacatcgtcatcaaccaccggtgcgcggaaaagaaggacgcgcgcggcgtgtactgcatcttcgagggcgggactcccgacgaccgcctggactggggccccgggatgatctgcagcgacgacacgcagtactcggacgggacggggcaccgcgacacgggcgaggggttcgcggcggcgcccgacatcgaccacctcaacccgcgcgtgcagcgggagctctccgcctggctcaactggctcaggtccgacgccgtggggttcgacggctggcgcctcgacttcgccaagggctactcgccggccgtcgccagaatgtacgtggagagcacggggccgccgagcttcgtcgtcgcggagatatggaactcgctgagctacagcggggacggcaagccggcgcccaaccaggaccagtgccggcaggagctgctggactggacgcgggccgtcggcgggcccgccatggcgttcgacttccccaccaagggcctgctgcaggcgggcgtgcagggggagctgtggcggctgcgcgacagctccggcaacgcggccggcctgatcgggtgggcgcccgagaaggccgtcaccttcgtcgacaaccatgacaccgggtcgacgcagaagctctggccgttcccatccgacaaggtcatgcagggctacgcctacatcctcacccatccaggagtcccctgcattttctacgaccacatgttcgactggaacctgaagcaggagatatccacgctgtctgccatcagggcgcggaacggcatccgcgccgggagcaagctgcggatcctcgtggcggacgcggacgcgtacgtggccgtcgtcgacgagaaggtcatggtgaagatcgggacaaggtacggcgtgagcagcgtggtcccgtcggatttccacccggcggcgcacggcaaggactactgcgtctgggagaaagcgagcctccgcgtcccggcggggcgccacctctagcagctcagattgctcagtcttgtgctgcattgcaaacacagcagcacgacactgcataacgtcttttccttgaccgatctgacaaagcagcattagtccgttgatcggtggaagaccactcgtcagtgttgagttgaatgtttgatcaataaaatacggcaatgctgtaagggttgttttttatgccattgataatacactgtactgttcagttgttgaactctatttcttagccatgccaagtgcttttcttattttgaataacattacagcaaaaagttgaaagacaaaaaaaaaaacccccgaacagagtgctttgggtcccaagctactttagactgtgttcggcgttccccctaaatttctccccctatatctcactcacttgtcacatcagcgttctctttcccctatatctccacgtcgacgcggaagctaagcttgcatgcctgcaggtcgactctagaggatctgcaccggacactgtctggtggcataccagacagtccggtgtgccagatcagggcacccttcggttcctttgctcctttgcttttgaaccctaactttgatcgtttattggtttgtgttgaacctttatgcacctgtggaatatataatctagaacaaactagttagtccaatcatttgtgttgggcattcaaccaccaaaattatttataggaaaaggttaaaccttatttccctttcaatctccccctttttggtgattgatgccaacacaaaccaaagaaaatatataagtgcagaattgaactagtttgcataaggtaagtgcataggttacttagaattaaatcaatttatacttttacttgatatgcatggttgctttcttttattttaacattttggaccacatttgcaccacttgttttgttttttgcaaatctttttggaaattctttttcaaagtcttttgcaaatagtcaaaggtatatgaataagattgtaagaagcattttcaagatttgaaatttctccccctgtttcaaatgcttttcctttgactaaacaaaactccccctgaataaaattctcctcttagctttcaagagggttttaaatagatatcaattggaaatatatttagatgctaattttgaaaatataccaattgaaaatcaacataccaatttgaaattaaacataccaatttaaaaaatttcaaaaagtggtggtgcggtccttttgctttgggcttaatatttctccccctttggcattaatcgccaaaaacggagactttgtgagccatttatactttctccccattggtaaatgaaatatgagtgaaagattataccaaatttggacagtgatgcggagtgacggcgaaggataaacgataccgttagagtggagtggaagccttgtcttcgccgaagactccatttccctttcaatctacgacttagcatagaaatacacttgaaaacacattagtcgtagccacgaaagagatatgatcaaaggtatacaaatgagctatgtgtgtaatgtttcaatcaaagtttcgagaatcaagaatatttagctcattcctaagtttgctaaaggttttatcatctaatggtttggtaaagatatcgactaattgttctttggtgctaacataagcaatctcgatatcacccctttgttggtgatccctcaaaaagtgataccgaatgtctatgtgcttagtgcggctgtgttcaacgggattatccgccatgcagatagcactctcattgtcacataggagagggactttgctcaatttgtagccatagtccctaaggttttgcctcatccaaagtaattgcacacaacaatgtcctgcggcaatatacttggcttcggcggtagaaagagctattgagttttgtttctttgaagtccaagacaccagggatctccctagaaactgacaagtccctgatgtgctcttcctatcaattttacaccctgcccaatcggcatctgaatatcctattaaatcaaaggtggatcccttggggtaccaaagaccaaatttaggagtgtaaactaaatatctcatgattcttttcacggccctaaggtgaacttccttaggatcggcttggaatcttgcacacatgcatatagaaagcatactatctggtcgagatgcacataaatagagtaaagatcctatcatcgaccggtataccttttggtctacggatttacctcccgtgtcgaggtcgagatgcccattagttcccatgggtgtcctgatgggcttggcatccttcattccaaacttgttgagtatgtcttgaatgtactttgtttggctgatgaaggtgccatcttggagttgcttgacttgaaatcctagaaaatatttcaacttccccatcatagacatctcgaatttcggaatcatgatcctactaaactcttcacaagtagatttgttagtagacccaaatataatatcatcaacataaatttggcatacaaacaaaacttttgaaatggttttagtaaagagagtaggatcggctttactgactctgaagccattagtgataagaaaatctcttaggcattcataccatgctgttggggcttgcttgagcccataaagcgcctttgagagtttataaacatggttagggtactcactatcttcaaagccgagaggttgctcaacatagacctattcaccccatttgatcacttttttggtccttcaggatctaatagttatgtataatttagagtctcttgtttaatggccagatatttctaattaatctaagaatttatgatattttttaattttttatcatgtctgatgagaattaacataaaggctcaattgggtcctgaattaataatagagtgaaaattaatccagaggctctattagaaccttcaattagtaataccaagatatatataagatagtagagtatagtttaaatgttggcattgttcattctttcttttgttatttaatttatgctttccacggtggttagtggttacttctgaagggtccaaataatgcatgaagagtttgaggacaagaagtctgccctaaaaatagcgatgcaaaggcatggtgtccaagccatacatatagcgcactaattttatcagcagaacaatggtatttataggtcctagtgcccaggcaacaagagacacgaataaagcatcgatcacgacaccatgagcaacaacgccctccagaccataataaacgcgaggctgccggggaaagagggcctctggcagatccacctccaagacggcaagatcagcgctatagacgcccaatcgggcgtgatgccaatcaccgagaactccctcgacgccgaacaaggtctcgtgatccctccattcgtcgaaccccacatccacctcgacacgacccaaacagcaggtcaacccaactggaaccaatccggcacactcttcgaaggcatcgagcgctgggcagaaaggaaggcgttgctcacacacgacgatgtgaagcagcgcgcatggcaaacgctcaagtggcagatagccaacggcatccagcacgtcagaacgcacgtcgacgtgtccgacgccacgcttacagctctgaaggctatgctcgaggtcaagcaggaggtcgcaccctggatagacctgcagatcgtcgcattcccacaggagggaatcctctcataccccaatggggaagccctcctcgaggaagctctgaggttgggtgctgacgttgtcggcgctatcccacacttcgagttcaccagggagtacggagtcgagtcgttgcataaaaccttcgcactggctcaaaaatacgacagactcatcgacgtccactgcgacgaaatcgacgacgagcagagcagattcgtcgagaccgtggctgcactggcccatagggaaggaatgggtgctagggttacggcgtcacataccaccgcaatgcacagctacaacggggcatacacctcccggctctttaggctcctcaaaatgtccggaatcaacttcgtcgccaaccccctggtcaatatacacctccagggacggttcgacacatacccgaaacgccgcgggataaccagggtgaaggagatgctggagagcggcatcaacgtctgctttggccacgacgacgtcttcgatccatggtacccactcggcaccgctaacatgctccaagtgctgcacatgggtctgcacgtctgccagctcatgggctatggacagatcaacgacggcctcaacctcatcacccaccactctgctcggacactcaacctccaggactacggcatagccgccgggaactcggctaatctcatcatcctcccggcggagaatggattcgatgcacttaggcgccaggtgccagtcaggtattcagtgcgcggaggaaaggtgatagcctccacccaaccagcacagaccaccgtctacctcgaacagccggaagcgatcgactacaagcgctagcactagacttgtccatcttctggattggccaacttaattaatgtatgaaataaaaggatgcacacatagtgacatgctaatcactataatgtgggcatcaaagttgtgtgttatgtgtaattactagttatctgaataaaagagaaagagatcatccatatttcttatcctaaatgaatgtcacgtgtctttataattctttgatgaaccagatgcatttcattaaccaaatccatatacatataaatattaatcatatataattaatatcaattgggttagcaaaacaaatctagtctaggtgtgttttgcggatcagctgcagtgcagcgtgacccggtcgtgcccctctctagagataatgagcattgcatgtctaagttataaaaaattaccacatattttttttgtcacacttgtttgaagtgcagtttatctatctttatacatatatttaaactttactctacgaataatataatctatagtactacaataatatcagtgttttagagaatcatataaatgaacagttagacatggtctaaaggacaattgagtattttgacaacaggactctacagttttatctttttagtgtgcatgtgttctcctttttttttgcaaatagcttcacctatataatacttcatccattttattagtacatccatttagggtttagggttaatggtttttatagactaatttttttagtacatctattttattctattttagcctctaaattaagaaaactaaaactctattttagtttttttatttaataatttagatataaaatagaataaaataaagtgactaaaaattaaacaaataccctttaagaaattaaaaaaactaaggaaacatttttcttgtttcgagtagataatgccagcctgttaaacgccgtcgacgagtctaacggacaccaaccagcgaaccagcagcgtcgcgtcgggccaagcgaagcagacggcacggcatctctgtcgctgcctctggacccctctcgagagttccgctccaccgttggacttgctccgctgtcggcatccagaaattgcgtggcggagcggcagacgtgagccggcacggcaggcggcctcctcctcctctcacggcacggcagctacgggggattcctttcccaccgctccttcgctttcccttcctcgcccgccgtaataaatagacaccccctccacaccctctttccccaacctcgtgttgttcggagcgcacacacacacaaccagatctcccccaaatccacccgtcggcacctccgcttcaaggtacgccgctcgtcctccccccccccccctctctaccttctctagatcggcgttccggtccatggttagggcccggtagttctacttctgttcatgtttgtgttagatccgtgtttgtgttagatccgtgctgctagcgttcgtacacggatgcgacctgtacgtcagacacgttctgattgctaacttgccagtgtttctctttggggaatcctgggatggctctagccgttccgcagacgggatcgatttcatgattttttttgtttcgttgcatagggtttggtttgcccttttcctttatttcaatatatgccgtgcacttgtttgtcgggtcatcttttcatgcttttttttgtcttggttgtgatgatgtggtctggttgggcggtcgttctagatcggagtagaattctgtttcaaactacctggtggatttattaattttggatctgtatgtgtgtgccatacatattcatagttacgaattgaagatgatggatggaaatatcgatctaggataggtatacatgttgatgcgggttttactgatgcatatacagagatgctttttgttcgcttggttgtgatgatgtggtgtggttgggcggtcgttcattcgttctagatcggagtagaatactgtttcaaactacctggtgtatttattaattttggaactgtatgtgtgtgtcatacatcttcatagttacgagtttaagatggatggaaatatcgatctaggataggtatacatgttgatgtgggttttactgatgcatatacatgatggcatatgcagcatctattcatatgctctaaccttgagtacctatctattataataaacaagtatgttttataattattttgatcttgatatacttggatgatggcatatgcagcagctatatgtggatttttttagccctgccttcatacgctatttatttgcttggtactgtttcttttgtcgatgctcaccctgttgtttggtgttacttctgcagatgcaaaaactcattaactcagtgcaaaactatgcctggggcagcaaaacggcgttgactgaactttatggtatggaaaatccgtccagccagccgatggccgagctgtggatgggcgcacatccgaaaagcagttcacgagtgcagaatgccgccggagatatcgtttcactgcgtgatgtgattgagagtgataaatcgactctgctcggagaggccgttgccaaacgctttggcgaactgcctttcctgttcaaagtattatgcgcagcacagccactctccattcaggttcatccaaacaaacacaattctgaaatcggttttgccaaagaaaatgccgcaggtatcccgatggatgccgccgagcgtaactataaagatcctaaccacaagccggagctggtttttgcgctgacgcctttccttgcgatgaacgcgtttcgtgaattttccgagattgtctccctactccagccggtcgcaggtgcacatccggcgattgctcactttttacaacagcctgatgccgaacgtttaagcgaactgttcgccagcctgttgaatatgcagggtgaagaaaaatcccgcgcgctggcgattttaaaatcggccctcgatagccagcagggtgaaccgtggcaaacgattcgtttaatttctgaattttacccggaagacagcggtctgttctccccgctattgctgaatgtggtgaaattgaaccctggcgaagcgatgttcctgttcgctgaaacaccgcacgcttacctgcaaggcgtggcgctggaagtgatggcaaactccgataacgtgctgcgtgcgggtctgacgcctaaatacattgatattccggaactggttgccaatgtgaaattcgaagccaaaccggctaaccagttgttgacccagccggtgaaacaaggtgcagaactggacttcccgattccagtggatgattttgccttctcgctgcatgaccttagtgataaagaaaccaccattagccagcagagtgccgccattttgttctgcgtcgaaggcgatgcaacgttgtggaaaggttctcagcagttacagcttaaaccgggtgaatcagcgtttattgccgccaacgaatcaccggtgactgtcaaaggccacggccgtttagcgcgtgtttacaacaagctgtaagagcttactgaaaaaattaacatctcttgctaagatccatggatattcgaacgcgtaggtaccacatggttaacctagacttgtccatcttctggattggccaacttaattaatgtatgaaataaaaggatgcacacatagtgacatgctaatcactataatgtgggcatcaaagttgtgtgttatgtgtaattactagttatctgaataaaagagaaagagatcatccatatttcttatcctaaatgaatgtcacgtgtctttataattctttgatgaaccagatgcatttcattaaccaaatccatatacatataaatattaatcatatataattaatatcaattgggttagcaaaacaaatctagtctaggtgtgttttgcg

SEQ ID NO: 104 - DNA, 189 bp, Solanum tuberosum
  source 1..189: mol_type = unassigned DNA
gtaagtttctgcttctacctttgatatatatataataattatcattaattagtagtaatataatatttcaaatatttttttcaaaataaaagaatgtagtatatagcaattgcttttctgtagtttataagtgtgtatattttaatttataacttttctaatatatgaccaaaacatggtgatgtgcag

SEQ ID NO: 105 - DNA, 20 bp, synthetic construct
  misc_feature 1..20: note = CYS4 RECOGNITION SITE
  source 1..20: mol_type = other DNA
gttcactgccgtataggcag

SEQ ID NO: 106 - DNA, 564 bp, synthetic construct
  misc_feature 1..564: note = CYS4 (MO) DNA
  source 1..564: mol_type = other DNA
atggatcactatctcgacattaggctgaggccagatcctgagtttccacctgctcagcttatgagcgttttgttcggtaagctccaccaggccctggtggcacagggcggagacagaattggtgttagcttcccagatcttgacgaaagccgtagcaggttgggcgagagactccgtattcacgctagcgccgatgacctgagggcacttttggctagaccttggctcgaaggactgcgtgatcaccttcagtttggtgagccagccgtggttcctcacccaaccccttacaggcaggtgagcagagttcaggcaaagagcaatccagaacgtttgaggagaaggctcatgcgtaggcacgacctgagcgaggaagaggctagaaagcgtattcctgataccgtggccagggcacttgacttgccattcgttaccctcagaagccagagcaccggccagcacttccgtctgtttattaggcacggacctcttcaggtgaccgctgaagagggtggcttcacctgctatggattgagcaagggtggcttcgttccatggttttga

SEQ ID NO: 107 - protein, 187 aa, synthetic construct
  REGION 1..187: note = CYS4 (MO) PRT
MDHYLDIRLRPDPEFPPAQLMSVLFGKLHQALVAQGGDRIGVSFPDLDESRSRLGERLRIHASADDLRALLARPWLEGLRDHLQFGEPAVVPHPTPYRQVSRVQAKSNPERLRRRLMRRHDLSEEEARKRIPDTVARALDLPFVTLRSQSTGQHFRLFIRHGPLQVTAEEGGFTCYGLSKGGFVPWF

SEQ ID NO: 108 - DNA, 77 bp, synthetic construct
  misc_feature 1..77: note = DNA version of GUIDE RNA
  source 1..77: mol_type = other DNA
gttttagagctagaaatagcaagttaaaataaggctagtccgttatcaacttgaaaaagtggcaccgagtcggtgct

SEQ ID NO: 109 - DNA, 3697 bp, synthetic construct
  misc_feature 1..3697: note = PG46 PRO-CYS4(MO)-IN2-1 TERM
  source 1..3697: mol_type = other DNA
aagcttgcatgcctgcaggtcgactctagaggatctgcaccggacactgtctggtggcataccagacagtccggtgtgccagatcagggcacccttcggttcctttgctcctttgcttttgaaccctaactttgatcgtttattggtttgtgttgaacctttatgcacctgtggaatatataatctagaacaaactagttagtccaatcatttgtgttgggcattcaaccaccaaaattatttataggaaaaggttaaaccttatttccctttcaatctccccctttttggtgattgatgccaacacaaaccaaagaaaatatataagtgcagaattgaactagtttgcataaggtaagtgcataggttacttagaattaaatcaatttatacttttacttgatatgcatggttgctttcttttattttaacattttggaccacatttgcaccacttgttttgttttttgcaaatctttttggaaattctttttcaaagtcttttgcaaatagtcaaaggtatatgaataagattgtaagaagcattttcaagatttgaaatttctccccctgtttcaaatgcttttcctttgactaaacaaaactccccctgaataaaattctcctcttagctttcaagagggttttaaatagatatcaattggaaatatatttagatgctaattttgaaaatataccaattgaaaatcaacataccaatttgaaattaaacataccaatttaaaaaatttcaaaaagtggtggtgcggtccttttgctttgggcttaatatttctccccctttggcattaatcgccaaaaacggagactttgtgagccatttatactttctccccattggtaaatgaaatatgagtgaaagattataccaaatttggacagtgatgcggagtgacggcgaaggataaacgataccgttagagtggagtggaagccttgtcttcgccgaagactccatttccctttcaatctacgacttagcatagaaatacacttgaaaacacattagtcgtagccacgaaagagatatgatcaaaggtatacaaatgagctatgtgtgtaatgtttcaatcaaagtttcgagaatcaagaatatttagctcattcctaagtttgctaaaggttttatcatctaatggtttggtaaagatatcgactaattgttctttggtgctaacataagcaatctcgatatcacccctttgttggtgatccctcaaaaagtgataccgaatgtctatgtgcttagtgcggctgtgttcaacgggattatccgccatgcagatagcactctcattgtcacataggagagggactttgctcaatttgtagccatagtccctaaggttttgcctcatccaaagtaattgcacacaacaatgtcctgcggcaatatacttggcttcggcggtagaaagagctattgagttttgtttctttgaagtccaagacaccagggatctccctagaaactgacaagtccctgatgtgctcttcctatcaattttacaccctgcccaatcggcatctgaatatcctattaaatcaaaggtggatcccttggggtaccaaagaccaaatttaggagtgtaaactaaatatctcatgattcttttcacggccctaaggtgaacttccttaggatcggcttggaatcttgcacacatgcatatagaaagcatactatctggtcgagatgcacataaatagagtaaagatcctatcatcgaccggtataccttttggtctacggatttacctcccgtgtcgaggtcgagatgcccattagttcccatgggtgtcctgatgggcttggcatccttcattccaaacttgttgagtatgtcttgaatgtactttgtttggctgatgaaggtgccatcttggagttgcttgacttgaaatcctagaaaatatttcaacttccccatcatagacatctcgaatttcggaatcatgatcctactaaactcttcacaagtagatttgttagtagacccaaatataatatcatcaacataaatttggcatacaaacaaaacttttgaaatggttttagtaaagagagtaggatcggctttactgactctgaagccattagtgataagaaaatctcttaggcattcataccatgctgttggggcttgcttgagcccataaagcgcctttgagagtttataaacatggttagggtactcactatcttcaaagccgagaggttgctcaacatagacctattcaccccatttgatcacttttttggtccttcaggatctaatagttatgtataatttagagtctcttgtttaatggccagatatttctaattaatctaagaatttatgatattttttaattttttatcatgtctgatgagaattaacataaaggctcaattgggtcctgaattaataatagagtgaaaattaatccagaggctctattagaaccttcaattagtaataccaagatatatataagatagtagagtatagtttaaatgttggcattgttcattctttcttttgttatttaatttatgctttccacggtggttagtggttacttctgaagggtccaaataatgcatgaagagtttgaggacaagaagtctgccctaaaaatagcgatgcaaaggcatggtgtccaagccatacatatagcgcactaattttatcagcagaacaatggtatttataggtcctagtgcccaggcaacaagagacacgaataaagcatcgatcacgacaccggatccatggatcactatctcgacattaggctgaggccagatcctgagtttccacctgctcagcttatgagcgttttgttcggtaagctccaccaggccctggtggcacagggcggagacagaattggtgttagcttcccagatcttgacgaaagccgtagcaggttgggcgagagactccgtattcacgctagcgccgatgacctgagggcacttttggctagaccttggctcgaaggactgcgtgatcaccttcagtttggtgagccagccgtggttcctcacccaaccccttacaggcaggtgagcagagttcaggcaaagagcaatccagaacgtttgaggagaaggctcatgcgtaggcacgacctgagcgaggaagaggctagaaagcgtattcctgataccgtggccagggcacttgacttgccattcgttaccctcagaagccagagcaccggccagcacttccgtctgtttattaggcacggacctcttcaggtgaccgctgaagagggtggcttcacctgctatggattgagcaagggtggcttcgttccatggttttgaggtaccgatctgacaaagcagcattagtccgttgatcggtggaagaccactcgtcagtgttgagttgaatgtttgatcaataaaatacggcaatgctgtaagggttgttttttatgccattgataatacactgtactgttcagttgttgaactctatttcttagccatgccaagtgcttttcttattttgaataacattacagcaaaaagttgaaagacaaaaaaaaaaacccccgaacagagtgctttgggtcccaagctactttagactgtgttcggcgttccccctaaatttctccccctatatctcactcacttgtcacatcagcgttctctttcccctatatctccacg

SEQ ID NO: 110 - DNA, 18 bp, synthetic construct
  misc_feature 1..18: note = GT1 PRO TARGET1
  source 1..18: mol_type = other DNA
gtgcatcatggactcatg

SEQ ID NO: 111 - DNA, 20 bp, synthetic construct
  misc_feature 1..20: note = GT1 PRO TARGET2
  source 1..20: mol_type = other DNA
cgctgtacggcgtggtagac

SEQ ID NO: 112 - DNA, 19 bp, synthetic construct
  misc_feature 1..19: note = GT1 PRO TARGET3
  source 1..19: mol_type = other DNA
ccagcaacgtccagcgcgc

SEQ ID NO: 113 - DNA, 19 bp, synthetic construct
  misc_feature 1..19: note = GT1 PRO TARGET4
  source 1..19: mol_type = other DNA
gggtgcccgtgcgttgcaa

SEQ ID NO: 114 - DNA, 20 bp, synthetic construct
  misc_feature 1..20: note = GT1 PRO TARGET5
  source 1..20: mol_type = other DNA
gcatttcgcgagtcaaattt

SEQ ID NO: 115 - DNA, 1000 bp, synthetic construct; identical to SEQ ID NO: 86
  misc_feature 1..1000: note = ZM-U6 POLIII CHR8 PRO
  source 1..1000: mol_type = other DNA

SEQ ID NO: 116 - DNA, 12792 bp, synthetic construct
  misc_feature 1..12792: note = UBI-PMI-PINII TERM ----PRO-ZMAA1-IN2-1 TERM
  source 1..12792: mol_type = other DNA
gtgcagcgtgacccggtcgtgcccctctctagagataatgagcattgcatgtctaagttataaaaaattaccacatattttttttgtcacacttgtttgaagtgcagtttatctatctttatacatatatttaaactttactctacgaataatataatctatagtactacaataatatcagtgttttagagaatcatataaatgaacagttagacatggtctaaaggacaattgagtattttgacaacaggactctacagttttatctttttagtgtgcatgtgttctcctttttttttgcaaatagcttcacctatataatacttcatccattttattagtacatccatttagggtttagggttaatggtttttatagactaatttttttagtacatctattttattctattttagcctctaaattaagaaaactaaaactctattttagtttttttatttaataatttagatataaaatagaataaaataaagtgactaaaaattaaacaaataccctttaagaaattaaaaaaactaaggaaacatttttcttgtttcgagtagataatgccagcctgttaaacgccgtcgacgagtctaacggacaccaaccagcgaaccagcagcgtcgcgtcgggccaagcgaagcagacggcacggcatctctgtcgctgcctctggacccctctcgagagttccgctccaccgttggacttgctccgctgtcggcatccagaaattgcgtggcggagcggcagacgtgagccggcacggcaggcggcctcctcctcctctcacggcaccggcagctacgggggattcctttcccaccgctccttcgctttcccttcctcgcccgccgtaataaatagacaccccctccacaccctctttccccaacctcgtgttgttcggagcgcacacacacacaaccagatctcccccaaatccacccgtcggcacctccgcttcaaggtacgccgctcgtcctcccccccccccctctctaccttctctagatcggcgttccggtccatgcatggttagggcccggtagttctacttctgttcatgtttgtgttagatccgtgtttgtgttagatccgtgctgctagcgttcgtacacggatgcgacctgtacgtcagacacgttctgattgctaacttgccagtgtttctctttggggaatcctgggatggctctagccgttccgcagacgggatcgatttcatgattttttttgtttcgttgcatagggtttggtttgcccttttcctttatttcaatatatgccgtgcacttgtttgtcgggtcatcttttcatgcttttttttgtcttggttgtgatgatgtggtctggttgggcggtcgttctagatcggagtagaattctgtttcaaactacctggtggatttattaattttggatctgtatgtgtgtgccatacatattcatagttacgaattgaagatgatggatggaaatatcgatctaggataggtatacatgttgatgcgggttttactgatgcatatacagagatgctttttgttcgcttggttgtgatgatgtggtgtggttgggcggtcgttcattcgttctagatcggagtagaatactgtttcaaactacctggtgtatttattaattttggaactgtatgtgtgtgtcatacatcttcatagttacgagtttaagatggatggaaatatcgatctaggataggtatacatgttgatgtgggttttactgatgcatatacatgatggcatatgcagcatctattcatatgctctaaccttgagtacctatctattataataaacaagtatgttttataattattttgatcttgatatacttggatgatggcatatgcagcagctatatgtggatttttttagccctgccttcatacgctatttatttgcttggtactgtttcttttgtcgatgctcaccctgttgtttggtgttacttctgcaggtcgactttaacttagcctagcgaagttcctattccgaagttcctattctctagaaagtataggaacttcagatccaccgggatccccgatcatgcaaaaactcattaactcagtgcaaaactatgcctggggcagcaaaacggcgttgactgaactttatggtatggaaaatccgtccagccagccgatggccgagctgtggatgggcgcacatccgaaaagcagttcacgagtgcagaatgccgccggagatatcgtttcactgcgtgatgtgattgagagtgataaatcgactctgctcggagaggccgttgccaaacgctttggcgaactgcctttcctgttcaaagtattatgcgcagcacagccactctccattcaggttcatccaaacaaacacaattctgaaatcggttttgccaaagaaaatgccgcaggtatcccgatggatgccgccgagcgtaactataaagatcctaaccacaagccggagctggtttttgcgctgacgcctttccttgcgatgaacgcgtttcgtgaattttccgagattgtctccctactccagccggtcgcaggtgcacatccggcgattgctcactttttacaacagcctgatgccgaacgtttaagcgaactgttcgccagcctgttgaatatgcagggtgaagaaaaatcccgcgcgctggcgattttaaaatcggccctcgatagccagcagggtgaaccgtggcaaacgattcgtttaatttctgaattttacccggaagacagcggtctgttctccccgctattgctgaatgtggtgaaattgaaccctggcgaagcgatgttcctgttcgctgaaacaccgcacgcttacctgcaaggcgtggcgctggaagtgatggcaaactccgataacgtgctgcgtgcgggtctgacgcctaaatacattgatattccggaactggttgccaatgtgaaattcgaagccaaaccggctaaccagttgttgacccagccggtgaaacaaggtgcagaactggacttcccgattccagtggatgattttgccttctcgctgcatgaccttagtgataaagaaaccaccattagccagcagagtgccgccattttgttctgcgtcgaaggcgatgcaacgttgtggaaaggttctcagcagttacagcttaaaccgggtgaatcagcgtttattgccgccaacgaatcaccggtgactgtcaaaggccacggccgtttagcgcgtgtttacaacaagctgtaagagcttactgaaaaaattaacatctcttgctaagctgggggtggaacctagacttgtccatcttctggattggccaacttaattaatgtatgaaataaaaggatgcacacatagtgacatgctaatcactataatgtgggcatcaaagttgtgtgttatgtgtaattactagttatctgaataaaagagaaagagatcatccatatttcttatcctaaatgaatgtcacgtgtctttataattctttgatgaaccagatgcatttcattaaccaaatccatatacatataaatattaatcatatataattaatatcaattgggttagcaaaacaaatctagtctaggtgtgttttgcgaatgcgaccttcttatgtgcttctagtctccaaatgtggttgatagttattttgctctaagatcaacagtaatgaagtataaatcatcgttgtggtgtgctactcggttaattgagcattaacacacacaaacatgacgaggatggtataatctccaaaaatgtgtactttgttaggtgggaccctatagccttgattaatgtgctatgttaggcatgcctggaaacgtgtgacgcatatgttttgtgaacctgttgatattatatgtgcttttatattaccatattttattaaaatactaatatttattactagtaagatataacattctatctagcttaaaaactaaccataaatattccataataactagatttaccaaactaatatactaaatatacataataaatacaaaattaacaagacaataatcaatatttatgagcttaatatatttagacattatggttggtcgacgataatcatgctaacttttcgtaattgcttgattgaaatatgcttagaataatgcctctttgttctacatggcaaatagggaccattatggtgtaacaccctgggaaccacaaacaccccgaaatgctactaaactacacaactaaccttcatatataaaatttcgacagcatctcctttgaaaatttgcatagacgtggaagcaacagagtataaacagatatcatgataagaaaacatactagacattaataatctgctagaaatgggaagaatcgctgcacctgtgcagcgtgacccggtcgtgcccctctctagagataatgagcattgcatgtctaagttataaaaaattaccacatattttttttgtcacacttgtttgaagtgcagtttatctatctttatacatatatttaaactttactctacgaataatataatctatagtactacaataatatcagtgttttagagaatcatataaatgaacagttagacatggtctaaaggacaattgagtattttgacaacaggactctacagttttatctttttagtgtgcatgtgttctcctttttttttgcaaatagcttcacctatataatacttcatccattttattagtacatccatttagggtttagggttaatggtttttatagactaatttttttagtacatctattttattctattttagcctctaaattaagaaaactaaaactctattttagtttttttatttaataatttagatataaaatagaataaaataaagtgactaaaaattaaacaaataccctttaagaaattaaaaaaactaaggaaacatttttcttgtttcgagtagataatgccagcctgttaaacgccgtcgacgagtctaacggacaccaaccagcgaaccagcagcgtcgcgtcgggccaagcgaagcagacggcacggcatctctgtcgctgcctctggacccctctcgagagttccgctccaccgttggacttgctccgctgtcggcatccagaaattgcgtggcggagcggcagacgtgagccggcacggcaggcggcctcctcctcctctcacggcaccggcagctacgggggattcctttcccaccgctccttcgctttcccttcctcgcccgccgtaataaatagacaccccctccacaccctctttccccaacctcgtgttgttcggagcgcacacacacacaaccagatctcccccaaatccacccgtcggcacctccgcttcaaggtacgccgctcgtcctcccccccccccctctctaccttctctagatcggcgttccggtccatgcatggttagggcccggtagttctacttctgttcatgtttgtgttagatccgtgtttgtgttagatccgtgctgctagcgttcgtacacggatgcgacctgtacgtcagacacgttctgattgctaacttgccagtgtttctctttggggaatcctgggatggctctagccgttccgcagacgggatcgatttcatgattttttttgtttcgttgcatagggtttggtttgcccttttcctttatttcaatatatgccgtgcacttgtttgtcgggtcatcttttcatgcttttttttgtcttggttgtgatgatgtggtctggttgggcggtcgttctagatcggagtagaattctgtttcaaactacctggtggatttattaattttggatctgtatgtgtgtgccatacatattcatagttacgaattgaagatgatggatggaaatatcgatctaggataggtatacatgttgatgcgggttttactgatgcatatacagagatgctttttgttcgcttggttgtgatgatgtggtgtggttgggcggtcgttcattcgttctagatcggagtagaatactgtttcaaactacctggtgtatttattaattttggaactgtatgtgtgtgtcatacatcttcatagttacgagtttaagatggatggaaatatcgatctaggataggtatacatgttgatgtgggttttactgatgcatatacatgatggcatatgcagcatctattcatatgctctaaccttgagtacctatctattataataaacaagtatgttttataattattttgatcttgatatacttggatgatggcatatgcagcagctatatgtggatttttttagccctgccttcatacgctatttatttgcttggtactgtttcttttgtcgatgctcaccctgttgtttggtgttacttctgcagatggcccacagcaagcacggcctgaaggaggagatgaccatgaagtaccacatggagggctgcgtgaacggccacaagttcgtgatcaccggcgagggcatcggctaccccttcaagggcaagcagaccatcaacctgtgcgtgatcgagggcggccccctgcccttcagcgaggacatcctgagcgccggcttcaagtacggcgaccggatcttcaccgagtacccccaggacatcgtggactacttcaagaacagctgccccgccggctacacctggggccggagcttcctgttcgaggacggcgccgtgtgcatctgtaacgtggacatcaccgtgagcgtgaaggagaactgcatctaccacaagagcatcttcaacggcgtgaacttccccgccgacggccccgtgatgaagaagatgaccaccaactgggaggccagctgcgagaagatcatgcccgtgcctaagcagggcatcctgaagggcgacgtgagcatgtacctgctgctgaaggacggcggccggtaccggtgccagttcgacaccgtgtacaaggccaagagcgtgcccagcaagatgcccgagtggcacttcatccagcacaagctgctgcgggaggaccggagcgacgccaagaaccagaagtggcagctgaccgagcacgccatcgccttccccagcgccctggcctgaggatctcgatagggatctgttaacgatccccggcggtgtcccccactgaagaaactatgtgctgtagtatagccgctgcccgctggctagctagctagttgagtcatttagcggcgatgattgagtaataatgtgtcacgcatcaccatgcatgggtggcagtgtcagtgtgagcaatgacctgaatgaacaattgaaatgaaaagaaaaaagtattgttccaaattaaacgttttaaccttttaataggtttatacaataattgatatatgttttctgtatatgtctaatttgttatcatccatttagatatagacaaaaaaaatctaagaactaaaacaaatgctaatttgaaatgaagggagtatatattgggataatgtcgatgagatccctcgtaatatcaccgacatcacacgtgtccagttaatgtatcagtgatacgtgtattcacatttgttgcgcgtaggcgtacccaacaattttgatcgactatcagaaagtcaacggaagcgagtcgacctcgagggggggcccctgggctcgaaggcatggagtcaaagattcaaatagaggacctaacagaactcgccgtaaagactggcgaacagttcatacagagtctcttacgactcaatgacaagaagaaaatcttcgtcaacatggtggagcacgacacgcttgtctactccaaaaatatcaaagatacagtctcagaagaccaaagggcaattgagacttttcaacaaagggtaatatccggaaacctcctcggattccattgcccagctatctgtcactttattgtgaagatagtggaaaaggaaggtggctcctacaaatgccatcattgcgataaaggaaaggccatcgttgaagatgcctctgccgacagtggtcccaaagatggacccccacccacgaggagcatcgtggaaaaagaagacgttccaaccacgtcttcaaagcaagtggattgatgtgatatctccactgacgtaagggatgacgcacaatcccactaagctgaccgggcccggccgaagcttgcatgcctgcaggtcgactctagaggatctgcaccggacactgtctggtggcataccagacagtccggtgtgccagatcagggcacccttcggttcctttgctcctttgcttttgaaccctaactttgatcgtttattggtttgtgttgaacctttatgcacctgtggaatatataatctagaacaaactagttagtccaatcatttgtgttgggcattcaaccaccaaaattatttataggaaaaggttaaaccttatttccctttcaatctccccctttttggtgattgatgccaacacaaaccaaagaaaatatataagtgcagaattgaactagtttgcataaggtaagtgcataggttacttagaattaaatcaatttatacttttacttgatatgcatggttgctttcttttattttaacattttggaccacatttgcaccacttgttttgttttttgcaaatctttttggaaattctttttcaaagtcttttgcaaatagtcaaaggtatatgaataagattgtaagaagcattttcaagatttgaaatttctccccctgtttcaaatgcttttcctttgactaaacaaaactccccctgaataaaattctcctcttagctttcaagagggttttaaatagatatcaattggaaatatatttagatgctaattttgaaaatataccaattgaaaatcaacataccaatttgaaattaaacataccaatttaaaaaatttcaaaaagtggtggtgcggtccttttgctttgggcttaatatttctccccctttggcattaatcgccaaaaacggagactttgtgagccatttatactttctccccattggtaaatgaaatatgagtgaaagattataccaaatttggacagtgatgcggagtgacggcgaaggataaacgataccgttagagtggagtggaagccttgtcttcgccgaagactccatttccctttcaatctacgacttagcatagaaatacacttgaaaacacattagtcgtagccacgaaagagatatgatcaaaggtatacaaatgagctatgtgtgtaatgtttcaatcaaagtttcgagaatcaagaatatttagctcattcctaagtttgctaaaggttttatcatctaatggtttggtaaagatatcgactaattgttctttggtgctaacataagcaatctcgatatcacccctttgttggtgatccctcaaaaagtgataccgaatgtctatgtgcttagtgcggctgtgttcaacgggattatccgccatgcagatagcactctcattgtcacataggagagggactttgctcaatttgtagccatagtccctaaggttttgcctcatccaaagtaattgcacacaacaatgtcctgcggcaatatacttggcttcggcggtagaaagagctattgagttttgtttctttgaagtccaagacaccagggatctccctagaaactgacaagtccctgatgtgctcttcctatcaattttacaccctgcccaatcggcatctgaatatcctattaaatcaaaggtggatcccttggggtaccaaagaccaaatttaggagtgtaaactaaatatctcatgattcttttcacggccctaaggtgaacttccttaggatcggcttggaatcttgcacacatgcatatagaaagcatactatctggtcgagatgcacataaatagagtaaagatcctatcatcgaccggtataccttttggtctacggatttacctcccgtgtcgaggtcgagatgcccattagttcccatgggtgtcctgatgggcttggcatccttcattccaaacttgttgagtatgtcttgaatgtactttgtttggctgatgaaggtgccatcttggagttgcttgacttgaaatcctagaaaatatttcaacttccccatcatagacatctcgaatttcggaatcatgatcctactaaactcttcacaagtagatttgttagtagacccaaatataatatcatcaacataaatttggcatacaaacaaaacttttgaaatggttttagtaaagagagtaggatcggctttactgactctgaagccattagtgataagaaaatctcttaggcattcataccatgctgttggggcttgcttgagcccataaagcgcctttgagagtttataaacatggttagggtactcactatcttcaaagccgagaggttgctcaacatagacctattcaccccatttgatcacttttttggtccttcaggatctaatagttatgtataatttagagtctcttgtttaatggccagatatttctaattaatctaagaatttatgatattttttaattttttatcatgtctgatgagaattaacataaaggctcaattgggtcctgaattaataatagagtgaaaattaatccagaggctctattagaaccttcaattagtaataccaagatatatataagatagtagagtatagtttaaatgttggcattgttcattctttcttttgttatttaatttatgctttccacggtggttagtggttacttctgaagggtccaaataatgcatgaagagtttgaggacaagaagtctgccctaaaaatagcgatgcaaaggcatggtgtccaagccatacatatagcgcactaattttatcagcagaacaatggtatttataggtcctagtgcccaggcaacaagagacacgaataaagcatcgatcacgacaccatggcggcgacaatggcagtgacgacgatggtgacgaggagcaaggagagctggtcgtcattgcaggtcccggcggtggcattcccttggaagccacgaggtggcaagaccggcggcctcgagttccctcgccgggcgatgttcgccagcgtcggcctcaacgtgtgcccgggcgtcccggcggggcgcgacccgcgggagcccgatcccaaggtcgtccgggcggcctgcggcctggtccaggcacaagtcctcttccaggggtttaactgggagtcgtgcaagcagcagggaggctggtacaacaggctcaaggcccaggtcgacgacatcgccaaggccggcgtcacgcacgtctggctgcctccaccctcgcactccgtctcgccacaaggctacatgccaggccgcctatacgacctggacgcgtccaagtacggcacggcggcggagctcaagtccctgatagcggcgttccacggcaggggcgtgcagtgcgtggcggacatcgtcatcaaccaccggtgcgcggaaaagaaggacgcgcgcggcgtgtactgcatcttcgagggcgggactcccgacgaccgcctggactggggccccgggatgatctgcagcgacgacacgcagtactcggacgggacggggcaccgcgacacgggcgaggggttcgcggcggcgcccgacatcgaccacctcaacccgcgcgtgcagcgggagctctccgcctggctcaactggctcaggtccgacgccgtggggttcgacggctggcgcctcgacttcgccaagggctactcgccggccgtcgccagaatgtacgtggagagcacggggccgccgagcttcgtcgtcgcggagatatggaactcgctgagctacagcggggacggcaagccggcgcccaaccaggaccagtgccggcaggagctgctggactggacgcgggccgtcggcgggcccgccatggcgttcgacttccccaccaagggcctgctgcaggcgggcgtgcagggggagctgtggcggctgcgcgacagctccggcaacgcggccggcctgatcgggtgggcgcccgagaaggccgtcaccttcgtcgacaaccatgacaccgggtcgacgcagaagctctggccgttcccatccgacaaggtcatgcagggctacgcctacatcctcacccatccaggagtcccctgcattttctacgaccacatgttcgactggaacctgaagcaggagatatccacgctgtctgccatcagggcgcggaacggcatccgcgccgggagcaagctgcggatcctcgtggcggacgcggacgcgtacgtggccgtcgtcgacgagaaggtcatggtgaagatcgggacaaggtacggcgtgagcagcgtggtcccgtcggatttccacccggcggcgcacggcaaggactactgcgtctgggagaaagcgagcctccgcgtcccggcggggcgccacctctagcagctcagattgctcagtcttgtgctgcattgcaaacacagcagcacgacactgcataacgtcttttccttgagatctgacaaagcagcattagtccgttgatcggtggaagaccactcgtcagtgttgagttgaatgtttgatcaataaaatacggcaatgctgtaagggttgttttttatgccattgataatacactgtactgttcagttgttgaactctatttcttagccatgccaagtgcttttcttattttgaataacattacagcaaaaagttgaaagacaaaaaaaaaaacccccgaacagagtgctttgggtcccaagctactttagactgtgttcggcgttccccctaaatttctccccctatatctcactcacttgtcacatcagcgttctctttcccctatatctccacg

SEQ ID NO: 117 - DNA, 11637 bp, synthetic construct
  misc_feature 1..11637: note = UBI-FLP-PINII TERM OSACTIN-PINII UBI-ODP2-PINII
  source 1..11637: mol_type = other DNA
ctgcagtgcagcgtgacccggtcgtgcccctctctagagataatgagcattgcatgtctaagttataaaaaattaccacatattttttttgtcacacttgtttgaagtgcagtttatctatctttatacatatatttaaactttactctacgaataatataatctatagtactacaataatatcagtgttttagagaatcatataaatgaacagttagacatggtctaaaggacaattgagtattttgacaacaggactctacagttttatctttttagtgtgcatgtgttctcctttttttttgcaaatagcttcacctatataatacttcatccattttattagtacatccatttagggtttagggttaatggtttttatagactaatttttttagtacatctattttattctattttagcctctaaattaagaaaactaaaactctattttagtttttttatttaataatttagatataaaatagaataaaataaagtgactaaaaattaaacaaataccctttaagaaattaaaaaaactaaggaaacatttttcttgtttcgagtagataatgccagcctgttaaacgccgtcgacgagtctaacggacaccaaccagcgaaccagcagcgtcgcgtcgggccaagcgaagcagacggcacggcatctctgtcgctgcctctggacccctctcgagagttccgctccaccgttggacttgctccgctgtcggcatccagaaattgcgtggcggagcggcagacgtgagccggcacggcaggcggcctcctcctcctctcacggcacggcagctacgggggattcctttcccaccgctccttcgctttcccttcctcgcccgccgtaataaatagacaccccctccacaccctctttccccaacctcgtgttgttcggagcgcacacacacacaaccagatctcccccaaatccacccgtcggcacctccgcttcaaggtacgccgctcgtcctccccccccccccctctctaccttctctagatcggcgttccggtccatggttagggcccggtagttctacttctgttcatgtttgtgttagatccgtgtttgtgttagatccgtgctgctagcgttcgtacacggatgcgacctgtacgtcagacacgttctgattgctaacttgccagtgtttctctttggggaatcctgggatggctctagccgttccgcagacgggatcgatttcatgattttttttgtttcgttgcatagggtttggtttgcccttttcctttatttcaatatatgccgtgcacttgtttgtcgggtcatcttttcatgcttttttttgtcttggttgtgatgatgtggtctggttgggcggtcgttctagatcggagtagaattctgtttcaaactacctggtggatttattaattttggatctgtatgtgtgtgccatacatattcatagttacgaattgaagatgatggatggaaatatcgatctaggataggtatacatgttgatgcgggttttactgatgcatatacagagatgctttttgttcgcttggttgtgatgatgtggtgtggttgggcggtcgttcattcgttctagatcggagtagaatactgtttcaaactacctggtgtatttattaattttggaactgtatgtgtgtgtcatacatcttcatagttacgagtttaagatggatggaaatatcgatctaggataggtatacatgttgatgtgggttttactgatgcatatacatgatggcatatgcagcatctattcatatgctctaaccttgagtacctatctattataataaacaagtatgttttataattattttgatcttgatatacttggatgatggcatatgcagcagctatatgtggatttttttagccctgccttcatacgctatttatttgcttggtactgtttcttttgtcgatgctcaccctgttgtttggtgttacttctgcaggtcgactctagaggatccaacaatgccccagttcgacatcctctgcaagaccccccccaaggtgctcgtgaggcagttcgtggagaggttcgagaggccctccggcgagaagatcgccctctgcgccgccgagctcacctacctctgctggatgatcacccacaacggcaccgccattaagagggccaccttcatgtcatacaacaccatcatctccaactccctctccttcgacatcgtgaacaagtccctccagttcaaatacaagacccagaaggccaccatcctcgaggcctccctcaagaagctcatccccgcctgggagttcaccatcatcccctactacggccagaagcaccagtccgacatcaccgacatcgtgtcatccctccagcttcagttcgagtcctccgaggaggctgacaagggcaactcccactccaagaagatgctgaaggccctcctctccgagggcgagtccatctgggagatcaccgagaagatcctcaactccttcgagtacacctccaggttcactaagaccaagaccctctaccagttcctcttcctcgccaccttcatcaactgcggcaggttctcagacatcaagaacgtggaccccaagtccttcaagctcgtgcagaacaagtacctcggcgtgatcatccagtgcctcgtgaccgagaccaagacctccgtgtccaggcacatctacttcttctccgctcgcggcaggatcgaccccctcgtgtacctcgacgagttcctcaggaactcagagcccgtgctcaagagggtgaacaggaccggcaactcctcctccaacaagcaggagtaccagctcctcaaggacaacctcgtgaggtcctacaacaaggccctcaagaagaacgccccctactccatcttcgccatcaagaacggccccaagtcccacatcggtaggcacctcatgacctccttcctctcaatgaagggcctcaccgagctcaccaacgtggtgggcaactggtccgacaagagggcctccgccgtggccaggaccacctacacccaccagatcaccgccatccccgaccactacttcgccctcgtgtcaaggtactacgcctacgaccccatctccaaggagatgatcgccctcaaggacgagactaaccccatcgaggagtggcagcacatcgagcagctcaagggctccgccgagggctccatcaggtaccccgcctggaacggcatcatctcccaggaggtgctcgactacctctcctcctacatcaacaggaggatctgagttaacctagacttgtccatcttctggattggccaacttaattaatgtatgaaataaaaggatgcacacatagtgacatgctaatcactataatgtgggcatcaaagttgtgtgttatgtgtaattactagttatctgaataaaagagaaagagatcatccatatttcttatcctaaatgaatgtcacgtgtctttataattctttgatgaaccagatgcatttcattaaccaaatccatatacatataaatattaatcatatataattaatatcaattgggttagcaaaacaaatctagtctaggtgtgttttgcccgggatccctcagccgcctttcactatcttttttgcccgagtcattgtcatgtgaaccttggcatgtataatcggtgaattgcgtcgattttcctcttataggtgggccaatgaatccgtgtgatcgcgtctgattggctagagatatgtttcttccttgttggatgtattttcatacataatcatatgcatacaaatatttcattacactttatagaaatggtcagtaataaaccctatcactatgtctggtgtttcattttatttgcttttaaacgaaaattgacttcctgattcaatatttaaggatcgtcaacggtgtgcagttactaaattctggtttgtaggaactatagtaaactattcaagtcttcacttattgtgcactcacctctcgccacatcaccacagatgttattcacgtcttaaatttgaactacacatcatattgacacaatattttttttaaataagcgattaaaacctagcctctatgtcaacaatggtgtacataaccagcgaagtttagggagtaaaaaacatcgccttacacaaagttcgctttaaaaaataaagagtaaattttactttggaccacccttcaaccaatgtttcactttagaacgagtaattttattattgtcactttggaccaccctcaaatcttttttccatctacatccaatttatcatgtcaaagaaatggtctacatacagctaaggagatttatcgacgaatagtagctagcatactcgaggtcattcatatgcttgagaagagagtcgggatagtccaaaataaaacaaaggtaagattacctggtcaaaagtgaaaacatcagttaaaaggtggtataaagtaaaatatcggtaataaaaggtggcccaaagtgaaatttactcttttctactattataaaaattgaggatgtttttgtcggtactttgatacgtcatttttgtatgaattggtttttaagtttattcgcttttggaaatgcatatctgtatttgagtcgggttttaagttcgtttgcttttgtaaatacagagggatttgtataagaaatatctttaaaaaaacccatatgctaatttgacataatttttgagaaaaatatatattcaggcgaattctcacaatgaacaataataagattaaaatagctttcccccgttgcagcgcatgggtattttttctagtaaaaataaaagataaacttagactcaaaacatttacaaaaacaacccctaaagttcctaaagcccaaagtgctatccacgatccatagcaagcccagcccaacccaacccaacccaacccaccccagtccagccaactggacaatagtctccacacccccccactatcaccgtgagttgtccgcacgcaccgcacgtctcgcagccaaaaaaaaaaaaagaaagaaaaaaaagaaaaagaaaaaacagcaggtgggtccgggtcgtgggggccggaaacgcgaggaggatcgcgagccagcgacgaggccggccctccctccgcttccaaagaaacgccccccatcgccactatatacatacccccccctctcctcccatccccccaaccctaccaccaccaccaccaccacctccacctcctcccccctcgctgccggacgacgagctcctcccccctccccctccgccgccgccgcgccggtaaccaccccgcccctctcctctttctttctccgttttttttttccgtctcggtctcgatctttggccttggtagtttgggtgggcgagaggcggcttcgtgcgcgcccagatcggtgcgcgggaggggcgggatctcgcggctggggctctcgccggcgtggatcaggcccggatctcgcggggaatggggctctcggatgtagatctgcgatccgccgttgttgggggagatgatggggggtttaaaatttccgccatgctaaacaagatcaggaagaggggaaaagggcactatggtttatatttttatatatttctgctgcttcgtcaggcttagatgtgctagatctttctttcttctttttgtgggtagaatttgaatccctcagcattgttcatcggtagtttttcttttcatgatttgtgacaaatgcagcctcgtgcggagcttttttgtaggtagaagctgcatggcggccaatgcgggcggcggtggagcgggaggaggcagcggcagcggcagcgtggctgcgccggcggtgtgccgccccagcggctcgcggtggacgccgacgccggagcagatcaggatgctgaaggagctctactacggctgcggcatccggtcgcccagctcggagcagatccagcgcatcaccgccatgctgcggcagcacggcaagatcgagggcaagaacgtcttctactggttccagaaccacaaggcccgcgagcgccagaagcgccgcctcaccagcctcgacgtcaacgtgcccgccgccggcgcggccgacgccaccaccagccaactcggcgtcctctcgctgtcgtcgccgccgccttcaggcgcggcgcctccctcgcccaccctcggcttctacgccgccggcaatggcggcggatcggctgtgctgctggacacgagttccgactggggcagcagcggcgctgctatggccaccgagacatgcttcctgcaggactacatgggcgtgacggacacgggcagctcgtcgcagtggccacgcttctcgtcgtcggacacgataatggcggcggccgcggcgcgggcggcgacgacgcgggcgcccgagacgctccctctcttcccgacctgcggcgacgacggcggcagcggtagcagcagctacttgccgttctggggtgccgcgtccacaactgccggcgccacttcttccgttgcgatccaacagcaacaccagctgcaggagcagtacagcttttacagcaacagcaacagcacccagctggccggcaccggcaaccaagacgtatcggcaacagcagcagcagccgccgccctggagctgagcctcagctcatggtgctccccttaccctgctgcagggagtatgtgagagcaacgcgagctgccactgctcttcactgatgtctctggaatggaaggaggaggaagtgagcatagcgttggtgcgttgctgtcaagggcgaattgtaccacatggttaacctagacttgtccatcttctggattggccaacttaattaatgtatgaaataaaaggatgcacacatagtgacatgctaatcactataatgtgggcatcaaagttgtgtgttatgtgtaattactagttatctgaataaaagagaaagagatcatccatatttcttatcctaaatgaatgtcacgtgtctttataattctttgatgaaccagatgcatttcattaaccaaatccatatacatataaatattaatcatatataattaatatcaattgggttagcaaaacaaatctagtctaggtgtgttttgcgaggaattcctcgtgcagcgtgacccggtcgtgcccctctctagagataatgagcattgcatgtctaagttataaaaaattaccacatattttttttgtcacacttgtttgaagtgcagtttatctatctttatacatatatttaaactttactctacgaataatataatctatagtactacaataatatcagtgttttagagaatcatataaatgaacagttagacatggtctaaaggacaattgagtattttgacaacaggactctacagttttatctttttagtgtgcatgtgttctcctttttttttgcaaatagcttcacctatataatacttcatccattttattagtacatccatttagggtttagggttaatggtttttatagactaatttttttagtacatctattttattctattttagcctctaaattaagaaaactaaaactctattttagtttttttatttaataatttagatataaaatagaataaaataaagtgactaaaaattaaacaaataccctttaagaaattaaaaaaactaaggaaacatttttcttgtttcgagtagataatgccagcctgttaaacgccgtcgacgagtctaacggacaccaaccagcgaaccagcagcgtcgcgtcgggccaagcgaagcagacggcacggcatctctgtcgctgcctctggacccctctcgagagttccgctccaccgttggacttgctccgctgtcggcatccagaaattgcgtggcggagcggcagacgtgagccggcacggcaggcggcctcctcctcctctcacggcaccggcagctacgggggattcctttcccaccgctccttcgctttcccttcctcgcccgccgtaataaatagacaccccctccacaccctctttccccaacctcgtgttgttcggagcgcacacacacacaaccagatctcccccaaatccacccgtcggcacctccgcttcaaggtacgccgctcgtcctcccccccccccctctctaccttctctagatcggcgttccggtccatgcatggttagggcccggtagttctacttctgttcatgtttgtgttagatccgtgtttgtgttagatccgtgctgctagcgttcgtacacggatgcgacctgtacgtcagacacgttctgattgctaacttgccagtgtttctctttggggaatcctgggatggctctagccgttccgcagacgggatcgatttcatgattttttttgtttcgttgcatagggtttggtttgcccttttcctttatttcaatatatgccgtgcacttgtttgtcgggtcatcttttcatgcttttttttgtcttggttgtgatgatgtggtctggttgggcggtcgttctagatcggagtagaattctgtttcaaactacctggtggatttattaattttggatctgtatgtgtgtgccatacatattcatagttacgaattgaagatgatggatggaaatatcgatctaggataggtatacatgttgatgcgggttttactgatgcatatacagagatgctttttgttcgcttggttgtgatgatgtggtgtggttgggcggtcgttcattcgttctagatcggagtagaatactgtttcaaactacctggtgtatttattaattttggaactgtatgtgtgtgtcatacatcttcatagttacgagtttaagatggatggaaatatcgatctaggataggtatacatgttgatgtgggttttactgatgcatatacatgatggcatatgcagcatctattcatatgctctaaccttgagtacctatctattataataaacaagtatgttttataattattttgatcttgatatacttggatgatggcatatgcagcagctatatgtggatttttttagccctgccttcatacgctatttatttgcttggtactgtttcttttgtcgatgctcaccctgttgtttggtgttacttctgcaggtcgactctagaggatccatggccactgtgaacaactggctcgctttctccctctccccgcaggagctgccgccctcccagacgacggactccacactcatctcggccgccaccgccgaccatgtctccggcgatgtctgcttcaacatcccccaagattggagcatgaggggatcagagctttcggcgctcgtcgcggagccgaagctggaggacttcctcggcggcatctccttctccgagcagcatcacaaggccaactgcaacatgatacccagcactagcagcacagtttgctacgcgagctcaggtgctagcaccggctaccatcaccagctgtaccaccagcccaccagctcagcgctccacttcgcggactccgtaatggtggcctcctcggccggtgtccacgacggcggtgccatgctcagcgcggccgccgctaacggtgtcgctggcgctgccagtgccaacggcggcggcatcgggctgtccatgattaagaactggctgcggagccaaccggcgcccatgcagccgagggtggcggcggctgagggcgcgcaggggctctctttgtccatgaacatggcggggacgacccaaggcgctgctggcatgccacttctcgctggagagcgcgcacgggcgcccgagagtgtatcgacgtcagcacagggtggagccgtcgtcgtcacggcgccgaaggaggatagcggtggcagcggtgttgccggcgctctagtagccgtgagcacggacacgggtggcagcggcggcgcgtcggctgacaacacggcaaggaagacggtggacacgttcgggcagcgcacgtcgatttaccgtggcgtgacaaggcatagatggactgggagatatgaggcacatctttgggataacagttgcagaagggaagggcaaactcgtaagggtcgtcaagtctatttaggtggctatgataaagaggagaaagctgctagggcttatgatcttgctgctctgaagtactggggtgccacaacaacaacaaattttccagtgagtaactacgaaaaggagctcgaggacatgaagcacatgacaaggcaggagtttgtagcgtctctgagaaggaagagcagtggtttctccagaggtgcatccatttacaggggagtgactaggcatcaccaacatggaagatggcaagcacggattggacgagttgcagggaacaaggatctttacttgggcaccttcagcacccaggaggaggcagcggaggcgtacgacatcgcggcgatcaagttccgcggcctcaacgccgtcaccaacttcgacatgagccgctacgacgtgaagagcatcctggacagcagcgccctccccatcggcagcgccgccaagcgcctcaaggaggccgaggccgcagcgtccgcgcagcaccaccacgccggcgtggtgagctacgacgtcggccgcatcgcctcgcagctcggcgacggcggagccctggcggcggcgtacggcgcgcactaccacggcgccgcctggccgaccatcgcgttccagccgggcgccgccagcacaggcctgtaccacccgtacgcgcagcagccaatgcgcggcggcgggtggtgcaagcaggagcaggaccacgcggtgatcgcggccgcgcacagcctgcaggacctccaccacctgaacctgggcgcggccggcgcgcacgactttttctcggcagggcagcaggccgccgccgctgcgatgcacggcctgggtagcatcgacagtgcgtcgctcgagcacagcaccggctccaactccgtcgtctacaacggcggggtcggcgacagcaacggcgccagcgccgtcggcggcagtggcggtggctacatgatgccgatgagcgctgccggagcaaccactacatcggcaatggtgagccacgagcaggtgcatgcacgggcctacgacgaagccaagcaggctgctcagatggggtacgagagctacctggtgaacgcggagaacaatggtggcggaaggatgtctgcatgggggactgtcgtgtctgcagccgcggcggcagcagcaagcagcaacgacaacatggccgccgacgtcggccatggcggcgcgcagctcttcagtgtctggaacgacacttaagcgtacgtgccggcctggctctccgaaagggcgaattccagcacactggcggccgttactagacccaacctagacttgtccatcttctggattggccaacttaattaatgtatgaaataaaaggatgcacacatagtgacatgctaatcactataatgtgggcatcaaagttgtgtgttatgtgtaattactagttatctgaataaaagagaaagagatcatccatatttcttatcctaaatgaatgtcacgtgtctttataattctttgatgaaccagatgcatttcattaaccaaatccatatacatataaatattaatcatatataattaatatcaattgggttagcaaaacaaatctagtctaggtgtgttttgcgaatgcggcc

SEQ ID NO: 118 - DNA, 1272 bp, synthetic construct
  misc_feature 1..1272: note = FLPm DNA
  source 1..1272: mol_type = other DNA
atgccccagttcgacatcctctgcaagaccccccccaaggtgctcgtgaggcagttcgtggagaggttcgagaggccctccggcgagaagatcgccctctgcgccgccgagctcacctacctctgctggatgatcacccacaacggcaccgccattaagagggccaccttcatgtcatacaacaccatcatctccaactccctctccttcgacatcgtgaacaagtccctccagttcaaatacaagacccagaaggccaccatcctcgaggcctccctcaagaagctcatccccgcctgggagttcaccatcatcccctactacggccagaagcaccagtccgacatcaccgacatcgtgtcatccctccagcttcagttcgagtcctccgaggaggctgacaagggcaactcccactccaagaagatgctgaaggccctcctctccgagggcgagtccatctgggagatcaccgagaagatcctcaactccttcgagtacacctccaggttcactaagaccaagaccctctaccagttcctcttcctcgccaccttcatcaactgcggcaggttctcagacatcaagaacgtggaccccaagtccttcaagctcgtgcagaacaagtacctcggcgtgatcatccagtgcctcgtgaccgagaccaagacctccgtgtccaggcacatctacttcttctccgctcgcggcaggatcgaccccctcgtgtacctcgacgagttcctcaggaactcagagcccgtgctcaagagggtgaacaggaccggcaactcctcctccaacaagcaggagtaccagctcctcaaggacaacctcgtgaggtcctacaacaaggccctcaagaagaacgccccctactccatcttcgccatcaagaacggccccaagtcccacatcggtaggcacctcatgacctccttcctctcaatgaagggcctcaccgagctcaccaacgtggtgggcaactggtccgacaagagggcctccgccgtggccaggaccacctacacccaccagatcaccgccatccccgaccactacttcgccctcgtgtcaaggtactacgcctacgaccccatctccaaggagatgatcgccctcaaggacgagactaaccccatcgaggagtggcagcacatcgagcagctcaagggctccgccgagggctccatcaggtaccccgcctggaacggcatcatctcccaggaggtgctcgactacctctcctcctacatcaacaggaggatctga

SEQ ID NO: 119 - protein, 423 aa, synthetic construct
  REGION 1..423: note = FLPm PRT
MPQFDILCKTPPKVLVRQFVERFERPSGEKIALCAAELTYLCWMITHNGTAIKRATFMSYNTIISNSLSFDIVNKSLQFKYKTQKATILEASLKKLIPAWEFTIIPYYGQKHQSDITDIVSSLQLQFESSEEADKGNSHSKKMLKALLSEGESIWEITEKILNSFEYTSRFTKTKTLYQFLFLATFINCGRFSDIKNVDPKSFKLVQNKYLGVIIQCLVTETKTSVSRHIYFFSARGRIDPLVYLDEFLRNSEPVLKRVNRTGNSSSNKQEYQLLKDNLVRSYNKALKKNAPYSIFAIKNGPKSHIGRHLMTSFLSMKGLTELTNVVGNWSDKRASAVARTTYTHQITAIPDHYFALVSRYYAYDPISKEMIALKDETNPIEEWQHIEQLKGSAEGSIRYPAWNGIISQEVLDYLSSYINRRI

SEQ ID NO: 120 - DNA, 30 bp, synthetic construct
  misc_feature 1..30: note = minimal FRT5 mutant recombination site
  source 1..30: mol_type = other DNA
agttcctattcttcaaaaggtataggaact

SEQ ID NO: 121 - DNA, 30 bp, synthetic construct
  misc_feature 1..30: note = minimal FRT6 mutant recombination site
  source 1..30: mol_type = other DNA
agttcctattcttcaaaaagtataggaact

SEQ ID NO: 122 - DNA, 30 bp, synthetic construct
  misc_feature 1..30: note = minimal FRT12 mutant recombination site
  source 1..30: mol_type = other DNA
agttcctattctacatagagtataggaact